European Patent Specification EP 3 243 835 B1, published April 10, 2024. Title: Albumin variants and conjugates. Applicant: Albumedix A/S. The sequence listing filed with the application follows.

SEQUENCE LISTING (108 sequences)

SEQ ID NO: 1 - protein, 585 aa, Homo sapiens [sequence omitted]

SEQ ID NO: 2 - DNA, 1758 bp, Artificial Sequence
  Polynucleotide coding sequence (not codon optimised) for human serum albumin
gatgcacacaagagtgaggttgctcatcggtttaaagatttgggagaagaaaatttcaaagccttggtgttgattgcctttgctcagtatcttcagcagtgtccatttgaagatcatgtaaaattagtgaatgaagtaactgaatttgcaaaaacatgtgttgctgatgagtcagctgaaaattgtgacaaatcacttcataccctttttggagacaaattatgcacagttgcaactcttcgtgaaacctatggtgaaatggctgactgctgtgcaaaacaagaacctgagagaaatgaatgcttcttgcaacacaaagatgacaacccaaacctcccccgattggtgagaccagaggttgatgtgatgtgcactgcttttcatgacaatgaagagacatttttgaaaaaatacttatatgaaattgccagaagacatccttacttttatgccccggaactccttttctttgctaaaaggtataaagctgcttttacagaatgttgccaagctgctgataaagctgcctgcctgttgccaaagctcgatgaacttcgggatgaagggaaggcttcgtctgccaaacagagactcaagtgtgccagtctccaaaaatttggagaaagagctttcaaagcatgggcagtagctcgcctgagccagagatttcccaaagctgagtttgcagaagtttccaagttagtgacagatcttaccaaagtccacacggaatgctgccatggagatctgcttgaatgtgctgatgacagggcggaccttgccaagtatatctgtgaaaatcaagattcgatctccagtaaactgaaggaatgctgtgaaaaacctctgttggaaaaatcccactgcattgccgaagtggaaaatgatgagatgcctgctgacttgccttcattagctgctgattttgttgaaagtaaggatgtttgcaaaaactatgctgaggcaaaggatgtcttcctgggcatgtttttgtatgaatatgcaagaaggcatcctgattactctgtcgtgctgctgctgagacttgccaagacatatgaaaccactctagagaagtgctgtgccgctgcagatcctcatgaatgctatgccaaagtgttcgatgaatttaaacctcttgtggaagagcctcagaatttaatcaaacaaaattgtgagctttttgagcagcttggagagtacaaattccagaatgcgctattagttcgttacaccaagaaagtaccccaagtgtcaactccaactcttgtagaggtctcaagaaacctaggaaaagtgggcagcaaatgttgtaaacatcctgaagcaaaaagaatgccctgtgcagaagactatctatccgtggtcctgaaccagttatgtgtgttgcatgagaaaacgccagtaagtgacagagtcaccaaatgctgcacagaatccttggtgaacaggcgaccatgcttttcagctctggaagtcgatgaaacatacgttcccaaagagtttaatgctgaaacattcaccttccatgcagatatatgcacactttctgagaaggagagacaaatcaagaaacaaactgcacttgttgagctcgtgaaacacaagcccaaggcaacaaaagagcaactgaaagctgttatggatgatttcgcagcttttgtagagaagtgctgcaaggctgacgataaggagacctgctttgccgaggagggtaaaaaacttgttgctgcaagtcaagctgccttaggcttataa

SEQ ID NO: 3 - DNA, 1758 bp, Artificial Sequence
  Polynucleotide coding sequence (codon optimised for expression in yeast) for human serum albumin
gacgctcacaagtccgaagtcgctcacagattcaaggacttgggtgaagaaaacttcaaggctttggtcttgatcgctttcgctcaatacttgcaacaatgtccattcgaagatcacgtcaagttggtcaacgaagttaccgaattcgctaagacttgtgttgctgacgaatctgctgaaaactgtgacaagtccttgcacaccttgttcggtgataagttgtgtactgttgctaccttgagagaaacctacggtgaaatggctgactgttgtgctaagcaagaaccagaaagaaacgaatgtttcttgcaacacaaggacgacaacccaaacttgccaagattggttagaccagaagttgacgtcatgtgtactgctttccacgacaacgaagaaaccttcttgaagaagtacttgtacgaaattgctagaagacacccatacttctacgctccagaattgttgttcttcgctaagagatacaaggctgctttcaccgaatgttgtcaagctgctgataaggctgcttgtttgttgccaaagttggatgaattgagagacgaaggtaaggcttcttccgctaagcaaagattgaagtgtgcttccttgcaaaagttcggtgaaagagctttcaaggcttgggctgtcgctagattgtctcaaagattcccaaaggctgaattcgctgaagtttctaagttggttactgacttgactaaggttcacactgaatgttgtcacggtgacttgttggaatgtgctgatgacagagctgacttggctaagtacatctgtgaaaaccaagactctatctcttccaagttgaaggaatgttgtgaaaagccattgttggaaaagtctcactgtattgctgaagttgaaaacgatgaaatgccagctgacttgccatctttggctgctgacttcgttgaatctaaggacgtttgtaagaactacgctgaagctaaggacgtcttcttgggtatgttcttgtacgaatacgctagaagacacccagactactccgttgtcttgttgttgagattggctaagacctacgaaactaccttggaaaagtgttgtgctgctgctgacccacacgaatgttacgctaaggttttcgatgaattcaagccattggtcgaagaaccacaaaacttgatcaagcaaaactgtgaattgttcgaacaattgggtgaatacaagttccaaaacgctttgttggttagatacactaagaaggtcccacaagtctccaccccaactttggttgaagtctctagaaacttgggtaaggtcggttctaagtgttgtaagcacccagaagctaagagaatgccatgtgctgaagattacttgtccgtcgttttgaaccaattgtgtgttttgcacgaaaagaccccagtctctgatagagtcaccaagtgttgtactgaatctttggttaacagaagaccatgtttctctgctttggaagtcgacgaaacttacgttccaaaggaattcaacgctgaaactttcaccttccacgctgatatctgtaccttgtccgaaaaggaaagacaaattaagaagcaaactgctttggttgaattggtcaagcacaagccaaaggctactaaggaacaattgaaggctgtcatggatgatttcgctgctttcgttgaaaagtgttgtaaggctgatgataaggaaacttgtttcgctgaagaaggtaagaagttggtcgctgcttcccaagctgctttgggtttgtaa

SEQ ID NO: 4 - DNA, 1758 bp, Artificial Sequence
  HA mutated to introduce restriction enzyme sites
gatgcacacaagagtgaggttgctcatcggtttaaagatttgggagaagaaaatttcaaagccttggtgttgattgcctttgctcagtatcttcagcagtgtccatttgaagatcatgtaaaattagtgaatgaagtaactgaatttgcaaaaacatgtgttgctgatgagtccgcggaaaattgtgacaaatcacttcataccctttttggagacaaattatgcacagttgcaactcttcgtgaaacctatggtgaaatggctgactgctgtgcaaaacaagaacctgagagaaatgaatgcttcttgcaacacaaagatgacaacccaaacctcccccgattggtgagaccagaggttgatgtgatgtgcactgcttttcatgacaatgaagagacatttttgaaaaaatacttatatgaaattgccagaagacatccttacttttatgccccggaactccttttctttgctaaaaggtataaagctgcttttacagaatgttgccaagctgctgataaagctgcctgcctgttgccaaagctcgatgaacttcgggatgaagggaaggctagctctgccaaacagagactcaagtgtgccagtctccaaaaatttggagaaagagctttcaaagcatgggcagtagctcgcctgagccagagatttcccaaagctgagtttgcagaagtttccaagttagtgacagatcttaccaaagtccacacggaatgctgccatggagatctgctcgagtgtgctgatgacagggcggaccttgccaagtatatctgtgaaaatcaagattcgatctccagtaaactgaaggaatgctgtgaaaaacctctgttggaaaaatcccactgcattgccgaagtggaaaatgatgagatgcctgctgacttgccttcattagctgctgattttgttgaaagtaaggatgtttgcaaaaactatgctgaggcaaaggatgtcttcctgggcatgtttttgtatgaatatgcaagaaggcatcctgattactctgtcgtgctgctgctgagacttgccaagacatatgaaaccactctagagaagtgctgtgccgctgctgatcctcatgaatgctatgccaaagtgttcgatgaatttaaacctcttgtggaagagcctcagaatttaatcaaacaaaattgtgagctttttgagcagcttggagagtacaaattccagaatgcgctattagttcgttacaccaagaaagtaccccaagtgtcaactccaactcttgtagaggtctcaagaaacctaggaaaagtgggatccaaatgttgtaaacatcctgaagcaaaaagaatgccctgtgcagaagactatctatccgtggtcctgaaccagttatgtgtgttgcatgagaaaacgccagtaagtgacagagtcaccaaatgctgcacagaatccttggtgaacaggcgaccatgcttttcagctctggaagtcgacgaaacatacgttcccaaagagtttaatgctgaaacattcaccttccatgcagatatatgcacactttctgagaaggagagacaaatcaagaaacaaactgcacttgttgagctcgtgaaacacaagcccaaggcaacaaaagagcaactgaaagctgttatggatgatttcgcagcttttgtagagaagtgctgcaaggctgacgataaggagacctgctttgccgaggagggtaaaaaacttgttgctgcaagtcaagctgccttaggcttataa

SEQ ID NO: 5 - DNA, 1758 bp, Artificial sequence
  TA1: HA with A2C
gattgtcacaagagtgaggttgctcatcggtttaaagatttgggagaagaaaatttcaaagccttggtgttgattgcctttgctcagtatcttcagcagtgtccatttgaagatcatgtaaaattagtgaatgaagtaactgaatttgcaaaaacatgtgttgctgatgagtccgcggaaaattgtgacaaatcacttcataccctttttggagacaaattatgcacagttgcaactcttcgtgaaacctatggtgaaatggctgactgctgtgcaaaacaagaacctgagagaaatgaatgcttcttgcaacacaaagatgacaacccaaacctcccccgattggtgagaccagaggttgatgtgatgtgcactgcttttcatgacaatgaagagacatttttgaaaaaatacttatatgaaattgccagaagacatccttacttttatgccccggaactccttttctttgctaaaaggtataaagctgcttttacagaatgttgccaagctgctgataaagctgcctgcctgttgccaaagctcgatgaacttcgggatgaagggaaggctagctctgccaaacagagactcaagtgtgccagtctccaaaaatttggagaaagagctttcaaagcatgggcagtagctcgcctgagccagagatttcccaaagctgagtttgcagaagtttccaagttagtgacagatcttaccaaagtccacacggaatgctgccatggagatctgctcgagtgtgctgatgacagggcggaccttgccaagtatatctgtgaaaatcaagattcgatctccagtaaactgaaggaatgctgtgaaaaacctctgttggaaaaatcccactgcattgccgaagtggaaaatgatgagatgcctgctgacttgccttcattagctgctgattttgttgaaagtaaggatgtttgcaaaaactatgctgaggcaaaggatgtcttcctgggcatgtttttgtatgaatatgcaagaaggcatcctgattactctgtcgtgctgctgctgagacttgccaagacatatgaaaccactctagagaagtgctgtgccgctgctgatcctcatgaatgctatgccaaagtgttcgatgaatttaaacctcttgtggaagagcctcagaatttaatcaaacaaaattgtgagctttttgagcagcttggagagtacaaattccagaatgcgctattagttcgttacaccaagaaagtaccccaagtgtcaactccaactcttgtagaggtctcaagaaacctaggaaaagtgggatccaaatgttgtaaacatcctgaagcaaaaagaatgccctgtgcagaagactatctatccgtggtcctgaaccagttatgtgtgttgcatgagaaaacgccagtaagtgacagagtcaccaaatgctgcacagaatccttggtgaacaggcgaccatgcttttcagctctggaagtcgacgaaacatacgttcccaaagagtttaatgctgaaacattcaccttccatgcagatatatgcacactttctgagaaggagagacaaatcaagaaacaaactgcacttgttgagctcgtgaaacacaagcccaaggcaacaaaagagcaactgaaagctgttatggatgatttcgcagcttttgtagagaagtgctgcaaggctgacgataaggagacctgctttgccgaggagggtaaaaaacttgttgctgcaagtcaagctgccttaggcttataa

SEQ ID NO: 6 - DNA, 1758 bp, Artificial sequence
  TA2: HA with D1C
tgtgcacacaagagtgaggttgctcatcggtttaaagatttgggagaagaaaatttcaaagccttggtgttgattgcctttgctcagtatcttcagcagtgtccatttgaagatcatgtaaaattagtgaatgaagtaactgaatttgcaaaaacatgtgttgctgatgagtccgcggaaaattgtgacaaatcacttcataccctttttggagacaaattatgcacagttgcaactcttcgtgaaacctatggtgaaatggctgactgctgtgcaaaacaagaacctgagagaaatgaatgcttcttgcaacacaaagatgacaacccaaacctcccccgattggtgagaccagaggttgatgtgatgtgcactgcttttcatgacaatgaagagacatttttgaaaaaatacttatatgaaattgccagaagacatccttacttttatgccccggaactccttttctttgctaaaaggtataaagctgcttttacagaatgttgccaagctgctgataaagctgcctgcctgttgccaaagctcgatgaacttcgggatgaagggaaggctagctctgccaaacagagactcaagtgtgccagtctccaaaaatttggagaaagagctttcaaagcatgggcagtagctcgcctgagccagagatttcccaaagctgagtttgcagaagtttccaagttagtgacagatcttaccaaagtccacacggaatgctgccatggagatctgctcgagtgtgctgatgacagggcggaccttgccaagtatatctgtgaaaatcaagattcgatctccagtaaactgaaggaatgctgtgaaaaacctctgttggaaaaatcccactgcattgccgaagtggaaaatgatgagatgcctgctgacttgccttcattagctgctgattttgttgaaagtaaggatgtttgcaaaaactatgctgaggcaaaggatgtcttcctgggcatgtttttgtatgaatatgcaagaaggcatcctgattactctgtcgtgctgctgctgagacttgccaagacatatgaaaccactctagagaagtgctgtgccgctgctgatcctcatgaatgctatgccaaagtgttcgatgaatttaaacctcttgtggaagagcctcagaatttaatcaaacaaaattgtgagctttttgagcagcttggagagtacaaattccagaatgcgctattagttcgttacaccaagaaagtaccccaagtgtcaactccaactcttgtagaggtctcaagaaacctaggaaaagtgggatccaaatgttgtaaacatcctgaagcaaaaagaatgccctgtgcagaagactatctatccgtggtcctgaaccagttatgtgtgttgcatgagaaaacgccagtaagtgacagagtcaccaaatgctgcacagaatccttggtgaacaggcgaccatgcttttcagctctggaagtcgacgaaacatacgttcccaaagagtttaatgctgaaacattcaccttccatgcagatatatgcacactttctgagaaggagagacaaatcaagaaacaaactgcacttgttgagctcgtgaaacacaagcccaaggcaacaaaagagcaactgaaagctgttatggatgatttcgcagcttttgtagagaagtgctgcaaggctgacgataaggagacctgctttgccgaggagggtaaaaaacttgttgctgcaagtcaagctgccttaggcttataa

SEQ ID NO: 7 - DNA, 1758 bp, Artificial sequence
  TA3: HA with C75S
gatgcacacaagagtgaggttgctcatcggtttaaagatttgggagaagaaaatttcaaagccttggtgttgattgcctttgctcagtatcttcagcagtgtccatttgaagatcatgtaaaattagtgaatgaagtaactgaatttgcaaaaacatgtgttgctgatgagtccgcggaaaattgtgacaaatcacttcataccctttttggagacaaattatctacagttgcaactcttcgtgaaacctatggtgaaatggctgactgctgtgcaaaacaagaacctgagagaaatgaatgcttcttgcaacacaaagatgacaacccaaacctcccccgattggtgagaccagaggttgatgtgatgtgcactgcttttcatgacaatgaagagacatttttgaaaaaatacttatatgaaattgccagaagacatccttacttttatgccccggaactccttttctttgctaaaaggtataaagctgcttttacagaatgttgccaagctgctgataaagctgcctgcctgttgccaaagctcgatgaacttcgggatgaagggaaggctagctctgccaaacagagactcaagtgtgccagtctccaaaaatttggagaaagagctttcaaagcatgggcagtagctcgcctgagccagagatttcccaaagctgagtttgcagaagtttccaagttagtgacagatcttaccaaagtccacacggaatgctgccatggagatctgctcgagtgtgctgatgacagggcggaccttgccaagtatatctgtgaaaatcaagattcgatctccagtaaactgaaggaatgctgtgaaaaacctctgttggaaaaatcccactgcattgccgaagtggaaaatgatgagatgcctgctgacttgccttcattagctgctgattttgttgaaagtaaggatgtttgcaaaaactatgctgaggcaaaggatgtcttcctgggcatgtttttgtatgaatatgcaagaaggcatcctgattactctgtcgtgctgctgctgagacttgccaagacatatgaaaccactctagagaagtgctgtgccgctgctgatcctcatgaatgctatgccaaagtgttcgatgaatttaaacctcttgtggaagagcctcagaatttaatcaaacaaaattgtgagctttttgagcagcttggagagtacaaattccagaatgcgctattagttcgttacaccaagaaagtaccccaagtgtcaactccaactcttgtagaggtctcaagaaacctaggaaaagtgggatccaaatgttgtaaacatcctgaagcaaaaagaatgccctgtgcagaagactatctatccgtggtcctgaaccagttatgtgtgttgcatgagaaaacgccagtaagtgacagagtcaccaaatgctgcacagaatccttggtgaacaggcgaccatgcttttcagctctggaagtcgacgaaacatacgttcccaaagagtttaatgctgaaacattcaccttccatgcagatatatgcacactttctgagaaggagagacaaatcaagaaacaaactgcacttgttgagctcgtgaaacacaagcccaaggcaacaaaagagcaactgaaagctgttatggatgatttcgcagcttttgtagagaagtgctgcaaggctgacgataaggagacctgctttgccgaggagggtaaaaaacttgttgctgcaagtcaagctgccttaggcttataa

SEQ ID NO: 8 - DNA, 1758 bp, Artificial sequence
  TA4: HA with T79C
gatgcacacaagagtgaggttgctcatcggtttaaagatttgggagaagaaaatttcaaagccttggtgttgattgcctttgctcagtatcttcagcagtgtccatttgaagatcatgtaaaattagtgaatgaagtaactgaatttgcaaaaacatgtgttgctgatgagtccgcggaaaattgtgacaaatcacttcataccctttttggagacaaattatgcacagttgcatgtcttcgtgaaacctatggtgaaatggctgactgctgtgcaaaacaagaacctgagagaaatgaatgcttcttgcaacacaaagatgacaacccaaacctcccccgattggtgagaccagaggttgatgtgatgtgcactgcttttcatgacaatgaagagacatttttgaaaaaatacttatatgaaattgccagaagacatccttacttttatgccccggaactccttttctttgctaaaaggtataaagctgcttttacagaatgttgccaagctgctgataaagctgcctgcctgttgccaaagctcgatgaacttcgggatgaagggaaggctagctctgccaaacagagactcaagtgtgccagtctccaaaaatttggagaaagagctttcaaagcatgggcagtagctcgcctgagccagagatttcccaaagctgagtttgcagaagtttccaagttagtgacagatcttaccaaagtccacacggaatgctgccatggagatctgctcgagtgtgctgatgacagggcggaccttgccaagtatatctgtgaaaatcaagattcgatctccagtaaactgaaggaatgctgtgaaaaacctctgttggaaaaatcccactgcattgccgaagtggaaaatgatgagatgcctgctgacttgccttcattagctgctgattttgttgaaagtaaggatgtttgcaaaaactatgctgaggcaaaggatgtcttcctgggcatgtttttgtatgaatatgcaagaaggcatcctgattactctgtcgtgctgctgctgagacttgccaagacatatgaaaccactctagagaagtgctgtgccgctgctgatcctcatgaatgctatgccaaagtgttcgatgaatttaaacctcttgtggaagagcctcagaatttaatcaaacaaaattgtgagctttttgagcagcttggagagtacaaattccagaatgcgctattagttcgttacaccaagaaagtaccccaagtgtcaactccaactcttgtagaggtctcaagaaacctaggaaaagtgggatccaaatgttgtaaacatcctgaagcaaaaagaatgccctgtgcagaagactatctatccgtggtcctgaaccagttatgtgtgttgcatgagaaaacgccagtaagtgacagagtcaccaaatgctgcacagaatccttggtgaacaggcgaccatgcttttcagctctggaagtcgacgaaacatacgttcccaaagagtttaatgctgaaacattcaccttccatgcagatatatgcacactttctgagaaggagagacaaatcaagaaacaaactgcacttgttgagctcgtgaaacacaagcccaaggcaacaaaagagcaactgaaagctgttatggatgatttcgcagcttttgtagagaagtgctgcaaggctgacgataaggagacctgctttgccgaggagggtaaaaaacttgttgctgcaagtcaagctgccttaggcttataa

SEQ ID NO: 9 - DNA, 1758 bp, Artificial sequence
  TA5: HA with E82C
gatgcacacaagagtgaggttgctcatcggtttaaagatttgggagaagaaaatttcaaagccttggtgttgattgcctttgctcagtatcttcagcagtgtccatttgaagatcatgtaaaattagtgaatgaagtaactgaatttgcaaaaacatgtgttgctgatgagtccgcggaaaattgtgacaaatcacttcataccctttttggagacaaattatgcacagttgcaactcttcgttgtacctatggtgaaatggctgactgctgtgcaaaacaagaacctgagagaaatgaatgcttcttgcaacacaaagatgacaacccaaacctcccccgattggtgagaccagaggttgatgtgatgtgcactgcttttcatgacaatgaagagacatttttgaaaaaatacttatatgaaattgccagaagacatccttacttttatgccccggaactccttttctttgctaaaaggtataaagctgcttttacagaatgttgccaagctgctgataaagctgcctgcctgttgccaaagctcgatgaacttcgggatgaagggaaggctagctctgccaaacagagactcaagtgtgccagtctccaaaaatttggagaaagagctttcaaagcatgggcagtagctcgcctgagccagagatttcccaaagctgagtttgcagaagtttccaagttagtgacagatcttaccaaagtccacacggaatgctgccatggagatctgctcgagtgtgctgatgacagggcggaccttgccaagtatatctgtgaaaatcaagattcgatctccagtaaactgaaggaatgctgtgaaaaacctctgttggaaaaatcccactgcattgccgaagtggaaaatgatgagatgcctgctgacttgccttcattagctgctgattttgttgaaagtaaggatgtttgcaaaaactatgctgaggcaaaggatgtcttcctgggcatgtttttgtatgaatatgcaagaaggcatcctgattactctgtcgtgctgctgctgagacttgccaagacatatgaaaccactctagagaagtgctgtgccgctgctgatcctcatgaatgctatgccaaagtgttcgatgaatttaaacctcttgtggaagagcctcagaatttaatcaaacaaaattgtgagctttttgagcagcttggagagtacaaattccagaatgcgctattagttcgttacaccaagaaagtaccccaagtgtcaactccaactcttgtagaggtctcaagaaacctaggaaaagtgggatccaaatgttgtaaacatcctgaagcaaaaagaatgccctgtgcagaagactatctatccgtggtcctgaaccagttatgtgtgttgcatgagaaaacgccagtaagtgacagagtcaccaaatgctgcacagaatccttggtgaacaggcgaccatgcttttcagctctggaagtcgacgaaacatacgttcccaaagagtttaatgctgaaacattcaccttccatgcagatatatgcacactttctgagaaggagagacaaatcaagaaacaaactgcacttgttgagctcgtgaaacacaagcccaaggcaacaaaagagcaactgaaagctgttatggatgatttcgcagcttttgtagagaagtgctgcaaggctgacgataaggagacctgctttgccgaggagggtaaaaaacttgttgctgcaagtcaagctgccttaggcttataa

SEQ ID NO: 10 - DNA, 1758 bp, Artificial sequence
  TA6: HA with E86C
gatgcacacaagagtgaggttgctcatcggtttaaagatttgggagaagaaaatttcaaagccttggtgttgattgcctttgctcagtatcttcagcagtgtccatttgaagatcatgtaaaattagtgaatgaagtaactgaatttgcaaaaacatgtgttgctgatgagtccgcggaaaattgtgacaaatcacttcataccctttttggagacaaattatgcacagttgcaactcttcgtgaaacctatggttgtatggctgactgctgtgcaaaacaagaacctgagagaaatgaatgcttcttgcaacacaaagatgacaacccaaacctcccccgattggtgagaccagaggttgatgtgatgtgcactgcttttcatgacaatgaagagacatttttgaaaaaatacttatatgaaattgccagaagacatccttacttttatgccccggaactccttttctttgctaaaaggtataaagctgcttttacagaatgttgccaagctgctgataaagctgcctgcctgttgccaaagctcgatgaacttcgggatgaagggaaggctagctctgccaaacagagactcaagtgtgccagtctccaaaaatttggagaaagagctttcaaagcatgggcagtagctcgcctgagccagagatttcccaaagctgagtttgcagaagtttccaagttagtgacagatcttaccaaagtccacacggaatgctgccatggagatctgctcgagtgtgctgatgacagggcggaccttgccaagtatatctgtgaaaatcaagattcgatctccagtaaactgaaggaatgctgtgaaaaacctctgttggaaaaatcccactgcattgccgaagtggaaaatgatgagatgcctgctgacttgccttcattagctgctgattttgttgaaagtaaggatgtttgcaaaaactatgctgaggcaaaggatgtcttcctgggcatgtttttgtatgaatatgcaagaaggcatcctgattactctgtcgtgctgctgctgagacttgccaagacatatgaaaccactctagagaagtgctgtgccgctgctgatcctcatgaatgctatgccaaagtgttcgatgaatttaaacctcttgtggaagagcctcagaatttaatcaaacaaaattgtgagctttttgagcagcttggagagtacaaattccagaatgcgctattagttcgttacaccaagaaagtaccccaagtgtcaactccaactcttgtagaggtctcaagaaacctaggaaaagtgggatccaaatgttgtaaacatcctgaagcaaaaagaatgccctgtgcagaagactatctatccgtggtcctgaaccagttatgtgtgttgcatgagaaaacgccagtaagtgacagagtcaccaaatgctgcacagaatccttggtgaacaggcgaccatgcttttcagctctggaagtcgacgaaacatacgttcccaaagagtttaatgctgaaacattcaccttccatgcagatatatgcacactttctgagaaggagagacaaatcaagaaacaaactgcacttgttgagctcgtgaaacacaagcccaaggcaacaaaagagcaactgaaagctgttatggatgatttcgcagcttttgtagagaagtgctgcaaggctgacgataaggagacctgctttgccgaggagggtaaaaaacttgttgctgcaagtcaagctgccttaggcttataa

SEQ ID NO: 11 - DNA, 1758 bp, Artificial sequence
  TA7: HA with C124S
gatgcacacaagagtgaggttgctcatcggtttaaagatttgggagaagaaaatttcaaagccttggtgttgattgcctttgctcagtatcttcagcagtgtccatttgaagatcatgtaaaattagtgaatgaagtaactgaatttgcaaaaacatgtgttgctgatgagtccgcggaaaattgtgacaaatcacttcataccctttttggagacaaattatgcacagttgcaactcttcgtgaaacctatggtgaaatggctgactgctgtgcaaaacaagaacctgagagaaatgaatgcttcttgcaacacaaagatgacaacccaaacctcccccgattggtgagaccagaggttgatgtgatgtctactgcttttcatgacaatgaagagacatttttgaaaaaatacttatatgaaattgccagaagacatccttacttttatgccccggaactccttttctttgctaaaaggtataaagctgcttttacagaatgttgccaagctgctgataaagctgcctgcctgttgccaaagctcgatgaacttcgggatgaagggaaggctagctctgccaaacagagactcaagtgtgccagtctccaaaaatttggagaaagagctttcaaagcatgggcagtagctcgcctgagccagagatttcccaaagctgagtttgcagaagtttccaagttagtgacagatcttaccaaagtccacacggaatgctgccatggagatctgctcgagtgtgctgatgacagggcggaccttgccaagtatatctgtgaaaatcaagattcgatctccagtaaactgaaggaatgctgtgaaaaacctctgttggaaaaatcccactgcattgccgaagtggaaaatgatgagatgcctgctgacttgccttcattagctgctgattttgttgaaagtaaggatgtttgcaaaaactatgctgaggcaaaggatgtcttcctgggcatgtttttgtatgaatatgcaagaaggcatcctgattactctgtcgtgctgctgctgagacttgccaagacatatgaaaccactctagagaagtgctgtgccgctgctgatcctcatgaatgctatgccaaagtgttcgatgaatttaaacctcttgtggaagagcctcagaatttaatcaaacaaaattgtgagctttttgagcagcttggagagtacaaattccagaatgcgctattagttcgttacaccaagaaagtaccccaagtgtcaactccaactcttgtagaggtctcaagaaacctaggaaaagtgggatccaaatgttgtaaacatcctgaagcaaaaagaatgccctgtgcagaagactatctatccgtggtcctgaaccagttatgtgtgttgcatgagaaaacgccagtaagtgacagagtcaccaaatgctgcacagaatccttggtgaacaggcgaccatgcttttcagctctggaagtcgacgaaacatacgttcccaaagagtttaatgctgaaacattcaccttccatgcagatatatgcacactttctgagaaggagagacaaatcaagaaacaaactgcacttgttgagctcgtgaaacacaagcccaaggcaacaaaagagcaactgaaagctgttatggatgatttcgcagcttttgtagagaagtgctgcaaggctgacgataaggagacctgctttgccgaggagggtaaaaaacttgttgctgcaagtcaagctgccttaggcttataa

SEQ ID NO: 12 - DNA, 1758 bp, Artificial sequence
  TA8: HA with C168S
gatgcacacaagagtgaggttgctcatcggtttaaagatttgggagaagaaaatttcaaagccttggtgttgattgcctttgctcagtatcttcagcagtgtccatttgaagatcatgtaaaattagtgaatgaagtaactgaatttgcaaaaacatgtgttgctgatgagtccgcggaaaattgtgacaaatcacttcataccctttttggagacaaattatgcacagttgcaactcttcgtgaaacctatggtgaaatggctgactgctgtgcaaaacaagaacctgagagaaatgaatgcttcttgcaacacaaagatgacaacccaaacctcccccgattggtgagaccagaggttgatgtgatgtgcactgcttttcatgacaatgaagagacatttttgaaaaaatacttatatgaaattgccagaagacatccttacttttatgccccggaactccttttctttgctaaaaggtataaagctgcttttacagaatcttgccaagctgctgataaagctgcctgcctgttgccaaagctcgatgaacttcgggatgaagggaaggctagctctgccaaacagagactcaagtgtgccagtctccaaaaatttggagaaagagctttcaaagcatgggcagtagctcgcctgagccagagatttcccaaagctgagtttgcagaagtttccaagttagtgacagatcttaccaaagtccacacggaatgctgccatggagatctgctcgagtgtgctgatgacagggcggaccttgccaagtatatctgtgaaaatcaagattcgatctccagtaaactgaaggaatgctgtgaaaaacctctgttggaaaaatcccactgcattgccgaagtggaaaatgatgagatgcctgctgacttgccttcattagctgctgattttgttgaaagtaaggatgtttgcaaaaactatgctgaggcaaaggatgtcttcctgggcatgtttttgtatgaatatgcaagaaggcatcctgattactctgtcgtgctgctgctgagacttgccaagacatatgaaaccactctagagaagtgctgtgccgctgctgatcctcatgaatgctatgccaaagtgttcgatgaatttaaacctcttgtggaagagcctcagaatttaatcaaacaaaattgtgagctttttgagcagcttggagagtacaaattccagaatgcgctattagttcgttacaccaagaaagtaccccaagtgtcaactccaactcttgtagaggtctcaagaaacctaggaaaagtgggatccaaatgttgtaaacatcctgaagcaaaaagaatgccctgtgcagaagactatctatccgtggtcctgaaccagttatgtgtgttgcatgagaaaacgccagtaagtgacagagtcaccaaatgctgcacagaatccttggtgaacaggcgaccatgcttttcagctctggaagtcgacgaaacatacgttcccaaagagtttaatgctgaaacattcaccttccatgcagatatatgcacactttctgagaaggagagacaaatcaagaaacaaactgcacttgttgagctcgtgaaacacaagcccaaggcaacaaaagagcaactgaaagctgttatggatgatttcgcagcttttgtagagaagtgctgcaaggctgacgataaggagacctgctttgccgaggagggtaaaaaacttgttgctgcaagtcaagctgccttaggcttataa

SEQ ID NO: 13 - DNA, 1758 bp, Artificial sequence
  TA9: HA with C169S
gatgcacacaagagtgaggttgctcatcggtttaaagatttgggagaagaaaatttcaaagccttggtgttgattgcctttgctcagtatcttcagcagtgtccatttgaagatcatgtaaaattagtgaatgaagtaactgaatttgcaaaaacatgtgttgctgatgagtccgcggaaaattgtgacaaatcacttcataccctttttggagacaaattatgcacagttgcaactcttcgtgaaacctatggtgaaatggctgactgctgtgcaaaacaagaacctgagagaaatgaatgcttcttgcaacacaaagatgacaacccaaacctcccccgattggtgagaccagaggttgatgtgatgtgcactgcttttcatgacaatgaagagacatttttgaaaaaatacttatatgaaattgccagaagacatccttacttttatgccccggaactccttttctttgctaaaaggtataaagctgcttttacagaatgttctcaagctgctgataaagctgcctgcctgttgccaaagctcgatgaacttcgggatgaagggaaggctagctctgccaaacagagactcaagtgtgccagtctccaaaaatttggagaaagagctttcaaagcatgggcagtagctcgcctgagccagagatttcccaaagctgagtttgcagaagtttccaagttagtgacagatcttaccaaagtccacacggaatgctgccatggagatctgctcgagtgtgctgatgacagggcggaccttgccaagtatatctgtgaaaatcaagattcgatctccagtaaactgaaggaatgctgtgaaaaacctctgttggaaaaatcccactgcattgccgaagtggaaaatgatgagatgcctgctgacttgccttcattagctgctgattttgttgaaagtaaggatgtttgcaaaaactatgctgaggcaaaggatgtcttcctgggcatgtttttgtatgaatatgcaagaaggcatcctgattactctgtcgtgctgctgctgagacttgccaagacatatgaaaccactctagagaagtgctgtgccgctgctgatcctcatgaatgctatgccaaagtgttcgatgaatttaaacctcttgtggaagagcctcagaatttaatcaaacaaaattgtgagctttttgagcagcttggagagtacaaattccagaatgcgctattagttcgttacaccaagaaagtaccccaagtgtcaactccaactcttgtagaggtctcaagaaacctaggaaaagtgggatccaaatgttgtaaacatcctgaagcaaaaagaatgccctgtgcagaagactatctatccgtggtcctgaaccagttatgtgtgttgcatgagaaaacgccagtaagtgacagagtcaccaaatgctgcacagaatccttggtgaacaggcgaccatgcttttcagctctggaagtcgacgaaacatacgttcccaaagagtttaatgctgaaacattcaccttccatgcagatatatgcacactttctgagaaggagagacaaatcaagaaacaaactgcacttgttgagctcgtgaaacacaagcccaaggcaacaaaagagcaactgaaagctgttatggatgatttcgcagcttttgtagagaagtgctgcaaggctgacgataaggagacctgctttgccgaggagggtaaaaaacttgttgctgcaagtcaagctgccttaggcttataa

SEQ ID NO: 14 - DNA, 1758 bp, Artificial sequence
  TA10: HA with C91S
gatgcacacaagagtgaggttgctcatcggtttaaagatttgggagaagaaaatttcaaagccttggtgttgattgcctttgctcagtatcttcagcagtgtccatttgaagatcatgtaaaattagtgaatgaagtaactgaatttgcaaaaacatgtgttgctgatgagtccgcggaaaattgtgacaaatcacttcataccctttttggagacaaattatgcacagttgcaactcttcgtgaaacctatggtgaaatggctgactgctctgcaaaacaagaacctgagagaaatgaatgcttcttgcaacacaaagatgacaacccaaacctcccccgattggtgagaccagaggttgatgtgatgtgcactgcttttcatgacaatgaagagacatttttgaaaaaatacttatatgaaattgccagaagacatccttacttttatgccccggaactccttttctttgctaaaaggtataaagctgcttttacagaatgttgccaagctgctgataaagctgcctgcctgttgccaaagctcgatgaacttcgggatgaagggaaggctagctctgccaaacagagactcaagtgtgccagtctccaaaaatttggagaaagagctttcaaagcatgggcagtagctcgcctgagccagagatttcccaaagctgagtttgcagaagtttccaagttagtgacagatcttaccaaagtccacacggaatgctgccatggagatctgctcgagtgtgctgatgacagggcggaccttgccaagtatatctgtgaaaatcaagattcgatctccagtaaactgaaggaatgctgtgaaaaacctctgttggaaaaatcccactgcattgccgaagtggaaaatgatgagatgcctgctgacttgccttcattagctgctgattttgttgaaagtaaggatgtttgcaaaaactatgctgaggcaaaggatgtcttcctgggcatgtttttgtatgaatatgcaagaaggcatcctgattactctgtcgtgctgctgctgagacttgccaagacatatgaaaccactctagagaagtgctgtgccgctgctgatcctcatgaatgctatgccaaagtgttcgatgaatttaaacctcttgtggaagagcctcagaatttaatcaaacaaaattgtgagctttttgagcagcttggagagtacaaattccagaatgcgctattagttcgttacaccaagaaagtaccccaagtgtcaactccaactcttgtagaggtctcaagaaacctaggaaaagtgggatccaaatgttgtaaacatcctgaagcaaaaagaatgccctgtgcagaagactatctatccgtggtcctgaaccagttatgtgtgttgcatgagaaaacgccagtaagtgacagagtcaccaaatgctgcacagaatccttggtgaacaggcgaccatgcttttcagctctggaagtcgacgaaacatacgttcccaaagagtttaatgctgaaacattcaccttccatgcagatatatgcacactttctgagaaggagagacaaatcaagaaacaaactgcacttgttgagctcgtgaaacacaagcccaaggcaacaaaagagcaactgaaagctgttatggatgatttcgcagcttttgtagagaagtgctgcaaggctgacgataaggagacctgctttgccgaggagggtaaaaaacttgttgctgcaagtcaagctgccttaggcttataa

SEQ ID NO: 15 - DNA, 1758 bp, Artificial sequence
  TA11: HA with D121C
gatgcacacaagagtgaggttgctcatcggtttaaagatttgggagaagaaaatttcaaagccttggtgttgattgcctttgctcagtatcttcagcagtgtccatttgaagatcatgtaaaattagtgaatgaagtaactgaatttgcaaaaacatgtgttgctgatgagtccgcggaaaattgtgacaaatcacttcataccctttttggagacaaattatgcacagttgcaactcttcgtgaaacctatggtgaaatggctgactgctgtgcaaaacaagaacctgagagaaatgaatgcttcttgcaacacaaagatgacaacccaaacctcccccgattggtgagaccagaggtttgtgtgatgtgcactgcttttcatgacaatgaagagacatttttgaaaaaatacttatatgaaattgccagaagacatccttacttttatgccccggaactccttttctttgctaaaaggtataaagctgcttttacagaatgttgccaagctgctgataaagctgcctgcctgttgccaaagctcgatgaacttcgggatgaagggaaggctagctctgccaaacagagactcaagtgtgccagtctccaaaaatttggagaaagagctttcaaagcatgggcagtagctcgcctgagccagagatttcccaaagctgagtttgcagaagtttccaagttagtgacagatcttaccaaagtccacacggaatgctgccatggagatctgctcgagtgtgctgatgacagggcggaccttgccaagtatatctgtgaaaatcaagattcgatctccagtaaactgaaggaatgctgtgaaaaacctctgttggaaaaatcccactgcattgccgaagtggaaaatgatgagatgcctgctgacttgccttcattagctgctgattttgttgaaagtaaggatgtttgcaaaaactatgctgaggcaaaggatgtcttcctgggcatgtttttgtatgaatatgcaagaaggcatcctgattactctgtcgtgctgctgctgagacttgccaagacatatgaaaccactctagagaagtgctgtgccgctgctgatcctcatgaatgctatgccaaagtgttcgatgaatttaaacctcttgtggaagagcctcagaatttaatcaaacaaaattgtgagctttttgagcagcttggagagtacaaattccagaatgcgctattagttcgttacaccaagaaagtaccccaagtgtcaactccaactcttgtagaggtctcaagaaacctaggaaaagtgggatccaaatgttgtaaacatcctgaagcaaaaagaatgccctgtgcagaagactatctatccgtggtcctgaaccagttatgtgtgttgcatgagaaaacgccagtaagtgacagagtcaccaaatgctgcacagaatccttggtgaacaggcgaccatgcttttcagctctggaagtcgacgaaacatacgttcccaaagagtttaatgctgaaacattcaccttccatgcagatatatgcacactttctgagaaggagagacaaatcaagaaacaaactgcacttgttgagctcgtgaaacacaagcccaaggcaacaaaagagcaactgaaagctgttatggatgatttcgcagcttttgtagagaagtgctgcaaggctgacgataaggagacctgctttgccgaggagggtaaaaaacttgttgctgcaagtcaagctgccttaggcttataa

SEQ ID NO: 16 - DNA, 1758 bp, Artificial sequence
  TA12: HA with D129C
gatgcacacaagagtgaggttgctcatcggtttaaagatttgggagaagaaaatttcaaagccttggtgttgattgcctttgctcagtatcttcagcagtgtccatttgaagatcatgtaaaattagtgaatgaagtaactgaatttgcaaaaacatgtgttgctgatgagtccgcggaaaattgtgacaaatcacttcataccctttttggagacaaattatgcacagttgcaactcttcgtgaaacctatggtgaaatggctgactgctgtgcaaaacaagaacctgagagaaatgaatgcttcttgcaacacaaagatgacaacccaaacctcccccgattggtgagaccagaggttgatgtgatgtgcactgcttttcattgtaatgaagagacatttttgaaaaaatacttatatgaaattgccagaagacatccttacttttatgccccggaactccttttctttgctaaaaggtataaagctgcttttacagaatgttgccaagctgctgataaagctgcctgcctgttgccaaagctcgatgaacttcgggatgaagggaaggctagctctgccaaacagagactcaagtgtgccagtctccaaaaatttggagaaagagctttcaaagcatgggcagtagctcgcctgagccagagatttcccaaagctgagtttgcagaagtttccaagttagtgacagatcttaccaaagtccacacggaatgctgccatggagatctgctcgagtgtgctgatgacagggcggaccttgccaagtatatctgtgaaaatcaagattcgatctccagtaaactgaaggaatgctgtgaaaaacctctgttggaaaaatcccactgcattgccgaagtggaaaatgatgagatgcctgctgacttgccttcattagctgctgattttgttgaaagtaaggatgtttgcaaaaactatgctgaggcaaaggatgtcttcctgggcatgtttttgtatgaatatgcaagaaggcatcctgattactctgtcgtgctgctgctgagacttgccaagacatatgaaaccactctagagaagtgctgtgccgctgctgatcctcatgaatgctatgccaaagtgttcgatgaatttaaacctcttgtggaagagcctcagaatttaatcaaacaaaattgtgagctttttgagcagcttggagagtacaaattccagaatgcgctattagttcgttacaccaagaaagtaccccaagtgtcaactccaactcttgtagaggtctcaagaaacctaggaaaagtgggatccaaatgttgtaaacatcctgaagcaaaaagaatgccctgtgcagaagactatctatccgtggtcctgaaccagttatgtgtgttgcatgagaaaacgccagtaagtgacagagtcaccaaatgctgcacagaatccttggtgaacaggcgaccatgcttttcagctctggaagtcgacgaaacatacgttcccaaagagtttaatgctgaaacattcaccttccatgcagatatatgcacactttctgagaaggagagacaaatcaagaaacaaactgcacttgttgagctcgtgaaacacaagcccaaggcaacaaaagagcaactgaaagctgttatggatgatttcgcagcttttgtagagaagtgctgcaaggctgacgataaggagacctgctttgccgaggagggtaaaaaacttgttgctgcaagtcaagctgccttaggcttataa

SEQ ID NO: 17 - DNA, 1758 bp, Artificial sequence
  TA13: HA with S270C
gatgcacacaagagtgaggttgctcatcggtttaaagatttgggagaagaaaatttcaaagccttggtgttgattgcctttgctcagtatcttcagcagtgtccatttgaagatcatgtaaaattagtgaatgaagtaactgaatttgcaaaaacatgtgttgctgatgagtccgcggaaaattgtgacaaatcacttcataccctttttggagacaaattatgcacagttgcaactcttcgtgaaacctatggtgaaatggctgactgctgtgcaaaacaagaacctgagagaaatgaatgcttcttgcaacacaaagatgacaacccaaacctcccccgattggtgagaccagaggttgatgtgatgtgcactgcttttcatgacaatgaagagacatttttgaaaaaatacttatatgaaattgccagaagacatccttacttttatgccccggaactccttttctttgctaaaaggtataaagctgcttttacagaatgttgccaagctgctgataaagctgcctgcctgttgccaaagctcgatgaacttcgggatgaagggaaggctagctctgccaaacagagactcaagtgtgccagtctccaaaaatttggagaaagagctttcaaagcatgggcagtagctcgcctgagccagagatttcccaaagctgagtttgcagaagtttccaagttagtgacagatcttaccaaagtccacacggaatgctgccatggagatctgctcgagtgtgctgatgacagggcggaccttgccaagtatatctgtgaaaatcaagattgtatctccagtaaactgaaggaatgctgtgaaaaacctctgttggaaaaatcccactgcattgccgaagtggaaaatgatgagatgcctgctgacttgccttcattagctgctgattttgttgaaagtaaggatgtttgcaaaaactatgctgaggcaaaggatgtcttcctgggcatgtttttgtatgaatatgcaagaaggcatcctgattactctgtcgtgctgctgctgagacttgccaagacatatgaaaccactctagagaagtgctgtgccgctgctgatcctcatgaatgctatgccaaagtgttcgatgaatttaaacctcttgtggaagagcctcagaatttaatcaaacaaaattgtgagctttttgagcagcttggagagtacaaattccagaatgcgctattagttcgttacaccaagaaagtaccccaagtgtcaactccaactcttgtagaggtctcaagaaacctaggaaaagtgggatccaaatgttgtaaacatcctgaagcaaaaagaatgccctgtgcagaagactatctatccgtggtcctgaaccagttatgtgtgttgcatgagaaaacgccagtaagtgacagagtcaccaaatgctgcacagaatccttggtgaacaggcgaccatgcttttcagctctggaagtcgacgaaacatacgttcccaaagagtttaatgctgaaacattcaccttccatgcagatatatgcacactttctgagaaggagagacaaatcaagaaacaaactgcacttgttgagctcgtgaaacacaagcccaaggcaacaaaagagcaactgaaagctgttatggatgatttcgcagcttttgtagagaagtgctgcaaggctgacgataaggagacctgctttgccgaggagggtaaaaaacttgttgctgcaagtcaagctgccttaggcttataa

SEQ ID NO: 18 - DNA, 1758 bp, Artificial sequence
  TA14:HA with C316A
gatgcacacaagagtgaggttgctcatcggtttaaagatttgggagaagaaaatttcaaagccttggtgttgattgcctttgctcagtatcttcagcagtgtccatttgaagatcatgtaaaattagtgaatgaagtaactgaatttgcaaaaacatgtgttgctgatgagtccgcggaaaattgtgacaaatcacttcataccctttttggagacaaattatgcacagttgcaactcttcgtgaaacctatggtgaaatggctgactgctgtgcaaaacaagaacctgagagaaatgaatgcttcttgcaacacaaagatgacaacccaaacctcccccgattggtgagaccagaggttgatgtgatgtgcactgcttttcatgacaatgaagagacatttttgaaaaaatacttatatgaaattgccagaagacatccttacttttatgccccggaactccttttctttgctaaaaggtataaagctgcttttacagaatgttgccaagctgctgataaagctgcctgcctgttgccaaagctcgatgaacttcgggatgaagggaaggctagctctgccaaacagagactcaagtgtgccagtctccaaaaatttggagaaagagctttcaaagcatgggcagtagctcgcctgagccagagatttcccaaagctgagtttgcagaagtttccaagttagtgacagatcttaccaaagtccacacggaatgctgccatggagatctgctcgagtgtgctgatgacagggcggaccttgccaagtatatctgtgaaaatcaagattcgatctccagtaaactgaaggaatgctgtgaaaaacctctgttggaaaaatcccactgcattgccgaagtggaaaatgatgagatgcctgctgacttgccttcattagctgctgattttgttgaaagtaaggatgttgctaaaaactatgctgaggcaaaggatgtcttcctgggcatgtttttgtatgaatatgcaagaaggcatcctgattactctgtcgtgctgctgctgagacttgccaagacatatgaaaccactctagagaagtgctgtgccgctgctgatcctcatgaatgctatgccaaagtgttcgatgaatttaaacctcttgtggaagagcctcagaatttaatcaaacaaaattgtgagctttttgagcagcttggagagtacaaattccagaatgcgctattagttcgttacaccaagaaagtaccccaagtgtcaactccaactcttgtagaggtctcaagaaacctaggaaaagtgggatccaaatgttgtaaacatcctgaagcaaaaagaatgccctgtgcagaagactatctatccgtggtcctgaaccagttatgtgtgttgcatgagaaaacgccagtaagtgacagagtcaccaaatgctgcacagaatccttggtgaacaggcgaccatgcttttcagctctggaagtcgacgaaacatacgttcccaaagagtttaatgctgaaacattcaccttccatgcagatatatgcacactttctgagaaggagagacaaatcaagaaacaaactgcacttgttgagctcgtgaaacacaagcccaaggcaacaaaagagcaactgaaagctgttatggatgatttcgcagcttttgtagagaagtgctgcaaggctgacgataaggagacctgctttgccgaggagggtaaaaaacttgttgctgcaagtcaagctgccttaggcttataa

SEQ ID NO: 19 - DNA, 1758 bp, Artificial sequence
  TA16: HA with C360S
gatgcacacaagagtgaggttgctcatcggtttaaagatttgggagaagaaaatttcaaagccttggtgttgattgcctttgctcagtatcttcagcagtgtccatttgaagatcatgtaaaattagtgaatgaagtaactgaatttgcaaaaacatgtgttgctgatgagtccgcggaaaattgtgacaaatcacttcataccctttttggagacaaattatgcacagttgcaactcttcgtgaaacctatggtgaaatggctgactgctgtgcaaaacaagaacctgagagaaatgaatgcttcttgcaacacaaagatgacaacccaaacctcccccgattggtgagaccagaggttgatgtgatgtgcactgcttttcatgacaatgaagagacatttttgaaaaaatacttatatgaaattgccagaagacatccttacttttatgccccggaactccttttctttgctaaaaggtataaagctgcttttacagaatgttgccaagctgctgataaagctgcctgcctgttgccaaagctcgatgaacttcgggatgaagggaaggctagctctgccaaacagagactcaagtgtgccagtctccaaaaatttggagaaagagctttcaaagcatgggcagtagctcgcctgagccagagatttcccaaagctgagtttgcagaagtttccaagttagtgacagatcttaccaaagtccacacggaatgctgccatggagatctgctcgagtgtgctgatgacagggcggaccttgccaagtatatctgtgaaaatcaagattcgatctccagtaaactgaaggaatgctgtgaaaaacctctgttggaaaaatcccactgcattgccgaagtggaaaatgatgagatgcctgctgacttgccttcattagctgctgattttgttgaaagtaaggatgtttgcaaaaactatgctgaggcaaaggatgtcttcctgggcatgtttttgtatgaatatgcaagaaggcatcctgattactctgtcgtgctgctgctgagacttgccaagacatatgaaaccactctagagaagtcttgtgccgctgctgatcctcatgaatgctatgccaaagtgttcgatgaatttaaacctcttgtggaagagcctcagaatttaatcaaacaaaattgtgagctttttgagcagcttggagagtacaaattccagaatgcgctattagttcgttacaccaagaaagtaccccaagtgtcaactccaactcttgtagaggtctcaagaaacctaggaaaagtgggatccaaatgttgtaaacatcctgaagcaaaaagaatgccctgtgcagaagactatctatccgtggtcctgaaccagttatgtgtgttgcatgagaaaacgccagtaagtgacagagtcaccaaatgctgcacagaatccttggtgaacaggcgaccatgcttttcagctctggaagtcgacgaaacatacgttcccaaagagtttaatgctgaaacattcaccttccatgcagatatatgcacactttctgagaaggagagacaaatcaagaaacaaactgcacttgttgagctcgtgaaacacaagcccaaggcaacaaaagagcaactgaaagctgttatggatgatttcgcagcttttgtagagaagtgctgcaaggctgacgataaggagacctgctttgccgaggagggtaaaaaacttgttgctgcaagtcaagctgccttaggcttataa

SEQ ID NO: 20 - DNA, 1758 bp, Artificial sequence
  TA17: HA with C361A
gatgcacacaagagtgaggttgctcatcggtttaaagatttgggagaagaaaatttcaaagccttggtgttgattgcctttgctcagtatcttcagcagtgtccatttgaagatcatgtaaaattagtgaatgaagtaactgaatttgcaaaaacatgtgttgctgatgagtccgcggaaaattgtgacaaatcacttcataccctttttggagacaaattatgcacagttgcaactcttcgtgaaacctatggtgaaatggctgactgctgtgcaaaacaagaacctgagagaaatgaatgcttcttgcaacacaaagatgacaacccaaacctcccccgattggtgagaccagaggttgatgtgatgtgcactgcttttcatgacaatgaagagacatttttgaaaaaatacttatatgaaattgccagaagacatccttacttttatgccccggaactccttttctttgctaaaaggtataaagctgcttttacagaatgttgccaagctgctgataaagctgcctgcctgttgccaaagctcgatgaacttcgggatgaagggaaggctagctctgccaaacagagactcaagtgtgccagtctccaaaaatttggagaaagagctttcaaagcatgggcagtagctcgcctgagccagagatttcccaaagctgagtttgcagaagtttccaagttagtgacagatcttaccaaagtccacacggaatgctgccatggagatctgctcgagtgtgctgatgacagggcggaccttgccaagtatatctgtgaaaatcaagattcgatctccagtaaactgaaggaatgctgtgaaaaacctctgttggaaaaatcccactgcattgccgaagtggaaaatgatgagatgcctgctgacttgccttcattagctgctgattttgttgaaagtaaggatgtttgcaaaaactatgctgaggcaaaggatgtcttcctgggcatgtttttgtatgaatatgcaagaaggcatcctgattactctgtcgtgctgctgctgagacttgccaagacatatgaaaccactctagagaagtgcgctgccgctgctgatcctcatgaatgctatgccaaagtgttcgatgaatttaaacctcttgtggaagagcctcagaatttaatcaaacaaaattgtgagctttttgagcagcttggagagtacaaattccagaatgcgctattagttcgttacaccaagaaagtaccccaagtgtcaactccaactcttgtagaggtctcaagaaacctaggaaaagtgggatccaaatgttgtaaacatcctgaagcaaaaagaatgccctgtgcagaagactatctatccgtggtcctgaaccagttatgtgtgttgcatgagaaaacgccagtaagtgacagagtcaccaaatgctgcacagaatccttggtgaacaggcgaccatgcttttcagctctggaagtcgacgaaacatacgttcccaaagagtttaatgctgaaacattcaccttccatgcagatatatgcacactttctgagaaggagagacaaatcaagaaacaaactgcacttgttgagctcgtgaaacacaagcccaaggcaacaaaagagcaactgaaagctgttatggatgatttcgcagcttttgtagagaagtgctgcaaggctgacgataaggagacctgctttgccgaggagggtaaaaaacttgttgctgcaagtcaagctgccttaggcttataa

SEQ ID NO: 21 - DNA, 1758 bp, Artificial sequence
  TA18: HA with C361S
gatgcacacaagagtgaggttgctcatcggtttaaagatttgggagaagaaaatttcaaagccttggtgttgattgcctttgctcagtatcttcagcagtgtccatttgaagatcatgtaaaattagtgaatgaagtaactgaatttgcaaaaacatgtgttgctgatgagtccgcggaaaattgtgacaaatcacttcataccctttttggagacaaattatgcacagttgcaactcttcgtgaaacctatggtgaaatggctgactgctgtgcaaaacaagaacctgagagaaatgaatgcttcttgcaacacaaagatgacaacccaaacctcccccgattggtgagaccagaggttgatgtgatgtgcactgcttttcatgacaatgaagagacatttttgaaaaaatacttatatgaaattgccagaagacatccttacttttatgccccggaactccttttctttgctaaaaggtataaagctgcttttacagaatgttgccaagctgctgataaagctgcctgcctgttgccaaagctcgatgaacttcgggatgaagggaaggctagctctgccaaacagagactcaagtgtgccagtctccaaaaatttggagaaagagctttcaaagcatgggcagtagctcgcctgagccagagatttcccaaagctgagtttgcagaagtttccaagttagtgacagatcttaccaaagtccacacggaatgctgccatggagatctgctcgagtgtgctgatgacagggcggaccttgccaagtatatctgtgaaaatcaagattcgatctccagtaaactgaaggaatgctgtgaaaaacctctgttggaaaaatcccactgcattgccgaagtggaaaatgatgagatgcctgctgacttgccttcattagctgctgattttgttgaaagtaaggatgtttgcaaaaactatgctgaggcaaaggatgtcttcctgggcatgtttttgtatgaatatgcaagaaggcatcctgattactctgtcgtgctgctgctgagacttgccaagacatatgaaaccactctagagaagtgctctgccgctgctgatcctcatgaatgctatgccaaagtgttcgatgaatttaaacctcttgtggaagagcctcagaatttaatcaaacaaaattgtgagctttttgagcagcttggagagtacaaattccagaatgcgctattagttcgttacaccaagaaagtaccccaagtgtcaactccaactcttgtagaggtctcaagaaacctaggaaaagtgggatccaaatgttgtaaacatcctgaagcaaaaagaatgccctgtgcagaagactatctatccgtggtcctgaaccagttatgtgtgttgcatgagaaaacgccagtaagtgacagagtcaccaaatgctgcacagaatccttggtgaacaggcgaccatgcttttcagctctggaagtcgacgaaacatacgttcccaaagagtttaatgctgaaacattcaccttccatgcagatatatgcacactttctgagaaggagagacaaatcaagaaacaaactgcacttgttgagctcgtgaaacacaagcccaaggcaacaaaagagcaactgaaagctgttatggatgatttcgcagcttttgtagagaagtgctgcaaggctgacgataaggagacctgctttgccgaggagggtaaaaaacttgttgctgcaagtcaagctgccttaggcttataa

SEQ ID NO: 22 - DNA, 1758 bp, Artificial sequence
  TA19: HA with A364C
gatgcacacaagagtgaggttgctcatcggtttaaagatttgggagaagaaaatttcaaagccttggtgttgattgcctttgctcagtatcttcagcagtgtccatttgaagatcatgtaaaattagtgaatgaagtaactgaatttgcaaaaacatgtgttgctgatgagtccgcggaaaattgtgacaaatcacttcataccctttttggagacaaattatgcacagttgcaactcttcgtgaaacctatggtgaaatggctgactgctgtgcaaaacaagaacctgagagaaatgaatgcttcttgcaacacaaagatgacaacccaaacctcccccgattggtgagaccagaggttgatgtgatgtgcactgcttttcatgacaatgaagagacatttttgaaaaaatacttatatgaaattgccagaagacatccttacttttatgccccggaactccttttctttgctaaaaggtataaagctgcttttacagaatgttgccaagctgctgataaagctgcctgcctgttgccaaagctcgatgaacttcgggatgaagggaaggctagctctgccaaacagagactcaagtgtgccagtctccaaaaatttggagaaagagctttcaaagcatgggcagtagctcgcctgagccagagatttcccaaagctgagtttgcagaagtttccaagttagtgacagatcttaccaaagtccacacggaatgctgccatggagatctgctcgagtgtgctgatgacagggcggaccttgccaagtatatctgtgaaaatcaagattcgatctccagtaaactgaaggaatgctgtgaaaaacctctgttggaaaaatcccactgcattgccgaagtggaaaatgatgagatgcctgctgacttgccttcattagctgctgattttgttgaaagtaaggatgtttgcaaaaactatgctgaggcaaaggatgtcttcctgggcatgtttttgtatgaatatgcaagaaggcatcctgattactctgtcgtgctgctgctgagacttgccaagacatatgaaaccactctagagaagtgctgtgccgcttgtgatcctcatgaatgctatgccaaagtgttcgatgaatttaaacctcttgtggaagagcctcagaatttaatcaaacaaaattgtgagctttttgagcagcttggagagtacaaattccagaatgcgctattagttcgttacaccaagaaagtaccccaagtgtcaactccaactcttgtagaggtctcaagaaacctaggaaaagtgggatccaaatgttgtaaacatcctgaagcaaaaagaatgccctgtgcagaagactatctatccgtggtcctgaaccagttatgtgtgttgcatgagaaaacgccagtaagtgacagagtcaccaaatgctgcacagaatccttggtgaacaggcgaccatgcttttcagctctggaagtcgacgaaacatacgttcccaaagagtttaatgctgaaacattcaccttccatgcagatatatgcacactttctgagaaggagagacaaatcaagaaacaaactgcacttgttgagctcgtgaaacacaagcccaaggcaacaaaagagcaactgaaagctgttatggatgatttcgcagcttttgtagagaagtgctgcaaggctgacgataaggagacctgctttgccgaggagggtaaaaaacttgttgctgcaagtcaagctgccttaggcttataa

SEQ ID NO: 23 - DNA, 1758 bp, Artificial sequence
  TA20: HA with Q397C
gatgcacacaagagtgaggttgctcatcggtttaaagatttgggagaagaaaatttcaaagccttggtgttgattgcctttgctcagtatcttcagcagtgtccatttgaagatcatgtaaaattagtgaatgaagtaactgaatttgcaaaaacatgtgttgctgatgagtccgcggaaaattgtgacaaatcacttcataccctttttggagacaaattatgcacagttgcaactcttcgtgaaacctatggtgaaatggctgactgctgtgcaaaacaagaacctgagagaaatgaatgcttcttgcaacacaaagatgacaacccaaacctcccccgattggtgagaccagaggttgatgtgatgtgcactgcttttcatgacaatgaagagacatttttgaaaaaatacttatatgaaattgccagaagacatccttacttttatgccccggaactccttttctttgctaaaaggtataaagctgcttttacagaatgttgccaagctgctgataaagctgcctgcctgttgccaaagctcgatgaacttcgggatgaagggaaggctagctctgccaaacagagactcaagtgtgccagtctccaaaaatttggagaaagagctttcaaagcatgggcagtagctcgcctgagccagagatttcccaaagctgagtttgcagaagtttccaagttagtgacagatcttaccaaagtccacacggaatgctgccatggagatctgctcgagtgtgctgatgacagggcggaccttgccaagtatatctgtgaaaatcaagattcgatctccagtaaactgaaggaatgctgtgaaaaacctctgttggaaaaatcccactgcattgccgaagtggaaaatgatgagatgcctgctgacttgccttcattagctgctgattttgttgaaagtaaggatgtttgcaaaaactatgctgaggcaaaggatgtcttcctgggcatgtttttgtatgaatatgcaagaaggcatcctgattactctgtcgtgctgctgctgagacttgccaagacatatgaaaccactctagagaagtgctgtgccgctgctgatcctcatgaatgctatgccaaagtgttcgatgaatttaaacctcttgtggaagagcctcagaatttaatcaaacaaaattgtgagctttttgagtgtcttggagagtacaaattccagaatgcgctattagttcgttacaccaagaaagtaccccaagtgtcaactccaactcttgtagaggtctcaagaaacctaggaaaagtgggatccaaatgttgtaaacatcctgaagcaaaaagaatgccctgtgcagaagactatctatccgtggtcctgaaccagttatgtgtgttgcatgagaaaacgccagtaagtgacagagtcaccaaatgctgcacagaatccttggtgaacaggcgaccatgcttttcagctctggaagtcgacgaaacatacgttcccaaagagtttaatgctgaaacattcaccttccatgcagatatatgcacactttctgagaaggagagacaaatcaagaaacaaactgcacttgttgagctcgtgaaacacaagcccaaggcaacaaaagagcaactgaaagctgttatggatgatttcgcagcttttgtagagaagtgctgcaaggctgacgataaggagacctgctttgccgaggagggtaaaaaacttgttgctgcaagtcaagctgccttaggcttataa

SEQ ID NO: 24 - DNA, 1758 bp, Artificial sequence
  TA21: HA with A504C
gatgcacacaagagtgaggttgctcatcggtttaaagatttgggagaagaaaatttcaaagccttggtgttgattgcctttgctcagtatcttcagcagtgtccatttgaagatcatgtaaaattagtgaatgaagtaactgaatttgcaaaaacatgtgttgctgatgagtccgcggaaaattgtgacaaatcacttcataccctttttggagacaaattatgcacagttgcaactcttcgtgaaacctatggtgaaatggctgactgctgtgcaaaacaagaacctgagagaaatgaatgcttcttgcaacacaaagatgacaacccaaacctcccccgattggtgagaccagaggttgatgtgatgtgcactgcttttcatgacaatgaagagacatttttgaaaaaatacttatatgaaattgccagaagacatccttacttttatgccccggaactccttttctttgctaaaaggtataaagctgcttttacagaatgttgccaagctgctgataaagctgcctgcctgttgccaaagctcgatgaacttcgggatgaagggaaggctagctctgccaaacagagactcaagtgtgccagtctccaaaaatttggagaaagagctttcaaagcatgggcagtagctcgcctgagccagagatttcccaaagctgagtttgcagaagtttccaagttagtgacagatcttaccaaagtccacacggaatgctgccatggagatctgctcgagtgtgctgatgacagggcggaccttgccaagtatatctgtgaaaatcaagattcgatctccagtaaactgaaggaatgctgtgaaaaacctctgttggaaaaatcccactgcattgccgaagtggaaaatgatgagatgcctgctgacttgccttcattagctgctgattttgttgaaagtaaggatgtttgcaaaaactatgctgaggcaaaggatgtcttcctgggcatgtttttgtatgaatatgcaagaaggcatcctgattactctgtcgtgctgctgctgagacttgccaagacatatgaaaccactctagagaagtgctgtgccgctgctgatcctcatgaatgctatgccaaagtgttcgatgaatttaaacctcttgtggaagagcctcagaatttaatcaaacaaaattgtgagctttttgagcagcttggagagtacaaattccagaatgcgctattagttcgttacaccaagaaagtaccccaagtgtcaactccaactcttgtagaggtctcaagaaacctaggaaaagtgggatccaaatgttgtaaacatcctgaagcaaaaagaatgccctgtgcagaagactatctatccgtggtcctgaaccagttatgtgtgttgcatgagaaaacgccagtaagtgacagagtcaccaaatgctgcacagaatccttggtgaacaggcgaccatgcttttcagctctggaagtcgacgaaacatacgttcccaaagagtttaattgtgaaacattcaccttccatgcagatatatgcacactttctgagaaggagagacaaatcaagaaacaaactgcacttgttgagctcgtgaaacacaagcccaaggcaacaaaagagcaactgaaagctgttatggatgatttcgcagcttttgtagagaagtgctgcaaggctgacgataaggagacctgctttgccgaggagggtaaaaaacttgttgctgcaagtcaagctgccttaggcttataa

SEQ ID NO: 25 - DNA, 1758 bp, Artificial sequence
  TA22: HA with A578C
gatgcacacaagagtgaggttgctcatcggtttaaagatttgggagaagaaaatttcaaagccttggtgttgattgcctttgctcagtatcttcagcagtgtccatttgaagatcatgtaaaattagtgaatgaagtaactgaatttgcaaaaacatgtgttgctgatgagtccgcggaaaattgtgacaaatcacttcataccctttttggagacaaattatgcacagttgcaactcttcgtgaaacctatggtgaaatggctgactgctgtgcaaaacaagaacctgagagaaatgaatgcttcttgcaacacaaagatgacaacccaaacctcccccgattggtgagaccagaggttgatgtgatgtgcactgcttttcatgacaatgaagagacatttttgaaaaaatacttatatgaaattgccagaagacatccttacttttatgccccggaactccttttctttgctaaaaggtataaagctgcttttacagaatgttgccaagctgctgataaagctgcctgcctgttgccaaagctcgatgaacttcgggatgaagggaaggctagctctgccaaacagagactcaagtgtgccagtctccaaaaatttggagaaagagctttcaaagcatgggcagtagctcgcctgagccagagatttcccaaagctgagtttgcagaagtttccaagttagtgacagatcttaccaaagtccacacggaatgctgccatggagatctgctcgagtgtgctgatgacagggcggaccttgccaagtatatctgtgaaaatcaagattcgatctccagtaaactgaaggaatgctgtgaaaaacctctgttggaaaaatcccactgcattgccgaagtggaaaatgatgagatgcctgctgacttgccttcattagctgctgattttgttgaaagtaaggatgtttgcaaaaactatgctgaggcaaaggatgtcttcctgggcatgtttttgtatgaatatgcaagaaggcatcctgattactctgtcgtgctgctgctgagacttgccaagacatatgaaaccactctagagaagtgctgtgccgctgctgatcctcatgaatgctatgccaaagtgttcgatgaatttaaacctcttgtggaagagcctcagaatttaatcaaacaaaattgtgagctttttgagcagcttggagagtacaaattccagaatgcgctattagttcgttacaccaagaaagtaccccaagtgtcaactccaactcttgtagaggtctcaagaaacctaggaaaagtgggatccaaatgttgtaaacatcctgaagcaaaaagaatgccctgtgcagaagactatctatccgtggtcctgaaccagttatgtgtgttgcatgagaaaacgccagtaagtgacagagtcaccaaatgctgcacagaatccttggtgaacaggcgaccatgcttttcagctctggaagtcgacgaaacatacgttcccaaagagtttaatgctgaaacattcaccttccatgcagatatatgcacactttctgagaaggagagacaaatcaagaaacaaactgcacttgttgagctcgtgaaacacaagcccaaggcaacaaaagagcaactgaaagctgttatggatgatttcgcagcttttgtagagaagtgctgcaaggctgacgataaggagacctgctttgccgaggagggtaaaaaacttgttgcttgtagtcaagctgccttaggcttataa

SEQ ID NO: 26 - DNA, 1758 bp, Artificial sequence
  TA23: HA with A581C
gatgcacacaagagtgaggttgctcatcggtttaaagatttgggagaagaaaatttcaaagccttggtgttgattgcctttgctcagtatcttcagcagtgtccatttgaagatcatgtaaaattagtgaatgaagtaactgaatttgcaaaaacatgtgttgctgatgagtccgcggaaaattgtgacaaatcacttcataccctttttggagacaaattatgcacagttgcaactcttcgtgaaacctatggtgaaatggctgactgctgtgcaaaacaagaacctgagagaaatgaatgcttcttgcaacacaaagatgacaacccaaacctcccccgattggtgagaccagaggttgatgtgatgtgcactgcttttcatgacaatgaagagacatttttgaaaaaatacttatatgaaattgccagaagacatccttacttttatgccccggaactccttttctttgctaaaaggtataaagctgcttttacagaatgttgccaagctgctgataaagctgcctgcctgttgccaaagctcgatgaacttcgggatgaagggaaggctagctctgccaaacagagactcaagtgtgccagtctccaaaaatttggagaaagagctttcaaagcatgggcagtagctcgcctgagccagagatttcccaaagctgagtttgcagaagtttccaagttagtgacagatcttaccaaagtccacacggaatgctgccatggagatctgctcgagtgtgctgatgacagggcggaccttgccaagtatatctgtgaaaatcaagattcgatctccagtaaactgaaggaatgctgtgaaaaacctctgttggaaaaatcccactgcattgccgaagtggaaaatgatgagatgcctgctgacttgccttcattagctgctgattttgttgaaagtaaggatgtttgcaaaaactatgctgaggcaaaggatgtcttcctgggcatgtttttgtatgaatatgcaagaaggcatcctgattactctgtcgtgctgctgctgagacttgccaagacatatgaaaccactctagagaagtgctgtgccgctgctgatcctcatgaatgctatgccaaagtgttcgatgaatttaaacctcttgtggaagagcctcagaatttaatcaaacaaaattgtgagctttttgagcagcttggagagtacaaattccagaatgcgctattagttcgttacaccaagaaagtaccccaagtgtcaactccaactcttgtagaggtctcaagaaacctaggaaaagtgggatccaaatgttgtaaacatcctgaagcaaaaagaatgccctgtgcagaagactatctatccgtggtcctgaaccagttatgtgtgttgcatgagaaaacgccagtaagtgacagagtcaccaaatgctgcacagaatccttggtgaacaggcgaccatgcttttcagctctggaagtcgacgaaacatacgttcccaaagagtttaatgctgaaacattcaccttccatgcagatatatgcacactttctgagaaggagagacaaatcaagaaacaaactgcacttgttgagctcgtgaaacacaagcccaaggcaacaaaagagcaactgaaagctgttatggatgatttcgcagcttttgtagagaagtgctgcaaggctgacgataaggagacctgctttgccgaggagggtaaaaaacttgttgctgcaagtcaatgtgccttaggcttataa

SEQ ID NO: 27 - DNA, 1758 bp, Artificial sequence
  TA24: HA with C558S
gatgcacacaagagtgaggttgctcatcggtttaaagatttgggagaagaaaatttcaaagccttggtgttgattgcctttgctcagtatcttcagcagtgtccatttgaagatcatgtaaaattagtgaatgaagtaactgaatttgcaaaaacatgtgttgctgatgagtccgcggaaaattgtgacaaatcacttcataccctttttggagacaaattatgcacagttgcaactcttcgtgaaacctatggtgaaatggctgactgctgtgcaaaacaagaacctgagagaaatgaatgcttcttgcaacacaaagatgacaacccaaacctcccccgattggtgagaccagaggttgatgtgatgtgcactgcttttcatgacaatgaagagacatttttgaaaaaatacttatatgaaattgccagaagacatccttacttttatgccccggaactccttttctttgctaaaaggtataaagctgcttttacagaatgttgccaagctgctgataaagctgcctgcctgttgccaaagctcgatgaacttcgggatgaagggaaggctagctctgccaaacagagactcaagtgtgccagtctccaaaaatttggagaaagagctttcaaagcatgggcagtagctcgcctgagccagagatttcccaaagctgagtttgcagaagtttccaagttagtgacagatcttaccaaagtccacacggaatgctgccatggagatctgctcgagtgtgctgatgacagggcggaccttgccaagtatatctgtgaaaatcaagattcgatctccagtaaactgaaggaatgctgtgaaaaacctctgttggaaaaatcccactgcattgccgaagtggaaaatgatgagatgcctgctgacttgccttcattagctgctgattttgttgaaagtaaggatgtttgcaaaaactatgctgaggcaaaggatgtcttcctgggcatgtttttgtatgaatatgcaagaaggcatcctgattactctgtcgtgctgctgctgagacttgccaagacatatgaaaccactctagagaagtgctgtgccgctgctgatcctcatgaatgctatgccaaagtgttcgatgaatttaaacctcttgtggaagagcctcagaatttaatcaaacaaaattgtgagctttttgagcagcttggagagtacaaattccagaatgcgctattagttcgttacaccaagaaagtaccccaagtgtcaactccaactcttgtagaggtctcaagaaacctaggaaaagtgggatccaaatgttgtaaacatcctgaagcaaaaagaatgccctgtgcagaagactatctatccgtggtcctgaaccagttatgtgtgttgcatgagaaaacgccagtaagtgacagagtcaccaaatgctgcacagaatccttggtgaacaggcgaccatgcttttcagctctggaagtcgacgaaacatacgttcccaaagagtttaatgctgaaacattcaccttccatgcagatatatgcacactttctgagaaggagagacaaatcaagaaacaaactgcacttgttgagctcgtgaaacacaagcccaaggcaacaaaagagcaactgaaagctgttatggatgatttcgcagcttttgtagagaagtcttgcaaggctgacgataaggagacctgctttgccgaggagggtaaaaaacttgttgctgcaagtcaagctgccttaggcttataa

SEQ ID NO: 28 - DNA, 1758 bp, Artificial sequence
  TA25: HA with C567S
gatgcacacaagagtgaggttgctcatcggtttaaagatttgggagaagaaaatttcaaagccttggtgttgattgcctttgctcagtatcttcagcagtgtccatttgaagatcatgtaaaattagtgaatgaagtaactgaatttgcaaaaacatgtgttgctgatgagtccgcggaaaattgtgacaaatcacttcataccctttttggagacaaattatgcacagttgcaactcttcgtgaaacctatggtgaaatggctgactgctgtgcaaaacaagaacctgagagaaatgaatgcttcttgcaacacaaagatgacaacccaaacctcccccgattggtgagaccagaggttgatgtgatgtgcactgcttttcatgacaatgaagagacatttttgaaaaaatacttatatgaaattgccagaagacatccttacttttatgccccggaactccttttctttgctaaaaggtataaagctgcttttacagaatgttgccaagctgctgataaagctgcctgcctgttgccaaagctcgatgaacttcgggatgaagggaaggctagctctgccaaacagagactcaagtgtgccagtctccaaaaatttggagaaagagctttcaaagcatgggcagtagctcgcctgagccagagatttcccaaagctgagtttgcagaagtttccaagttagtgacagatcttaccaaagtccacacggaatgctgccatggagatctgctcgagtgtgctgatgacagggcggaccttgccaagtatatctgtgaaaatcaagattcgatctccagtaaactgaaggaatgctgtgaaaaacctctgttggaaaaatcccactgcattgccgaagtggaaaatgatgagatgcctgctgacttgccttcattagctgctgattttgttgaaagtaaggatgtttgcaaaaactatgctgaggcaaaggatgtcttcctgggcatgtttttgtatgaatatgcaagaaggcatcctgattactctgtcgtgctgctgctgagacttgccaagacatatgaaaccactctagagaagtgctgtgccgctgctgatcctcatgaatgctatgccaaagtgttcgatgaatttaaacctcttgtggaagagcctcagaatttaatcaaacaaaattgtgagctttttgagcagcttggagagtacaaattccagaatgcgctattagttcgttacaccaagaaagtaccccaagtgtcaactccaactcttgtagaggtctcaagaaacctaggaaaagtgggatccaaatgttgtaaacatcctgaagcaaaaagaatgccctgtgcagaagactatctatccgtggtcctgaaccagttatgtgtgttgcatgagaaaacgccagtaagtgacagagtcaccaaatgctgcacagaatccttggtgaacaggcgaccatgcttttcagctctggaagtcgacgaaacatacgttcccaaagagtttaatgctgaaacattcaccttccatgcagatatatgcacactttctgagaaggagagacaaatcaagaaacaaactgcacttgttgagctcgtgaaacacaagcccaaggcaacaaaagagcaactgaaagctgttatggatgatttcgcagcttttgtagagaagtgctgcaaggctgacgataaggagacctcttttgccgaggagggtaaaaaacttgttgctgcaagtcaagctgccttaggcttataa

SEQ ID NO: 29 - DNA, 1758 bp, Artificial sequence
  TA26: HA with D549C
gatgcacacaagagtgaggttgctcatcggtttaaagatttgggagaagaaaatttcaaagccttggtgttgattgcctttgctcagtatcttcagcagtgtccatttgaagatcatgtaaaattagtgaatgaagtaactgaatttgcaaaaacatgtgttgctgatgagtccgcggaaaattgtgacaaatcacttcataccctttttggagacaaattatgcacagttgcaactcttcgtgaaacctatggtgaaatggctgactgctgtgcaaaacaagaacctgagagaaatgaatgcttcttgcaacacaaagatgacaacccaaacctcccccgattggtgagaccagaggttgatgtgatgtgcactgcttttcatgacaatgaagagacatttttgaaaaaatacttatatgaaattgccagaagacatccttacttttatgccccggaactccttttctttgctaaaaggtataaagctgcttttacagaatgttgccaagctgctgataaagctgcctgcctgttgccaaagctcgatgaacttcgggatgaagggaaggctagctctgccaaacagagactcaagtgtgccagtctccaaaaatttggagaaagagctttcaaagcatgggcagtagctcgcctgagccagagatttcccaaagctgagtttgcagaagtttccaagttagtgacagatcttaccaaagtccacacggaatgctgccatggagatctgctcgagtgtgctgatgacagggcggaccttgccaagtatatctgtgaaaatcaagattcgatctccagtaaactgaaggaatgctgtgaaaaacctctgttggaaaaatcccactgcattgccgaagtggaaaatgatgagatgcctgctgacttgccttcattagctgctgattttgttgaaagtaaggatgtttgcaaaaactatgctgaggcaaaggatgtcttcctgggcatgtttttgtatgaatatgcaagaaggcatcctgattactctgtcgtgctgctgctgagacttgccaagacatatgaaaccactctagagaagtgctgtgccgctgctgatcctcatgaatgctatgccaaagtgttcgatgaatttaaacctcttgtggaagagcctcagaatttaatcaaacaaaattgtgagctttttgagcagcttggagagtacaaattccagaatgcgctattagttcgttacaccaagaaagtaccccaagtgtcaactccaactcttgtagaggtctcaagaaacctaggaaaagtgggatccaaatgttgtaaacatcctgaagcaaaaagaatgccctgtgcagaagactatctatccgtggtcctgaaccagttatgtgtgttgcatgagaaaacgccagtaagtgacagagtcaccaaatgctgcacagaatccttggtgaacaggcgaccatgcttttcagctctggaagtcgacgaaacatacgttcccaaagagtttaatgctgaaacattcaccttccatgcagatatatgcacactttctgagaaggagagacaaatcaagaaacaaactgcacttgttgagctcgtgaaacacaagcccaaggcaacaaaagagcaactgaaagctgttatgtgtgatttcgcagcttttgtagagaagtgctgcaaggctgacgataaggagacctgctttgccgaggagggtaaaaaacttgttgctgcaagtcaagctgccttaggcttataa

SEQ ID NO: 30 - DNA, 1758 bp, Artificial sequence
  TA27: HA with D562C
gatgcacacaagagtgaggttgctcatcggtttaaagatttgggagaagaaaatttcaaagccttggtgttgattgcctttgctcagtatcttcagcagtgtccatttgaagatcatgtaaaattagtgaatgaagtaactgaatttgcaaaaacatgtgttgctgatgagtccgcggaaaattgtgacaaatcacttcataccctttttggagacaaattatgcacagttgcaactcttcgtgaaacctatggtgaaatggctgactgctgtgcaaaacaagaacctgagagaaatgaatgcttcttgcaacacaaagatgacaacccaaacctcccccgattggtgagaccagaggttgatgtgatgtgcactgcttttcatgacaatgaagagacatttttgaaaaaatacttatatgaaattgccagaagacatccttacttttatgccccggaactccttttctttgctaaaaggtataaagctgcttttacagaatgttgccaagctgctgataaagctgcctgcctgttgccaaagctcgatgaacttcgggatgaagggaaggctagctctgccaaacagagactcaagtgtgccagtctccaaaaatttggagaaagagctttcaaagcatgggcagtagctcgcctgagccagagatttcccaaagctgagtttgcagaagtttccaagttagtgacagatcttaccaaagtccacacggaatgctgccatggagatctgctcgagtgtgctgatgacagggcggaccttgccaagtatatctgtgaaaatcaagattcgatctccagtaaactgaaggaatgctgtgaaaaacctctgttggaaaaatcccactgcattgccgaagtggaaaatgatgagatgcctgctgacttgccttcattagctgctgattttgttgaaagtaaggatgtttgcaaaaactatgctgaggcaaaggatgtcttcctgggcatgtttttgtatgaatatgcaagaaggcatcctgattactctgtcgtgctgctgctgagacttgccaagacatatgaaaccactctagagaagtgctgtgccgctgctgatcctcatgaatgctatgccaaagtgttcgatgaatttaaacctcttgtggaagagcctcagaatttaatcaaacaaaattgtgagctttttgagcagcttggagagtacaaattccagaatgcgctattagttcgttacaccaagaaagtaccccaagtgtcaactccaactcttgtagaggtctcaagaaacctaggaaaagtgggatccaaatgttgtaaacatcctgaagcaaaaagaatgccctgtgcagaagactatctatccgtggtcctgaaccagttatgtgtgttgcatgagaaaacgccagtaagtgacagagtcaccaaatgctgcacagaatccttggtgaacaggcgaccatgcttttcagctctggaagtcgacgaaacatacgttcccaaagagtttaatgctgaaacattcaccttccatgcagatatatgcacactttctgagaaggagagacaaatcaagaaacaaactgcacttgttgagctcgtgaaacacaagcccaaggcaacaaaagagcaactgaaagctgttatggatgatttcgcagcttttgtagagaagtgctgcaaggcttgtgataaggagacctgctttgccgaggagggtaaaaaacttgttgctgcaagtcaagctgccttaggcttataa

SEQ ID NO: 31 - DNA, 1758 bp, Artificial sequence
  TA28: HA with E505C
gatgcacacaagagtgaggttgctcatcggtttaaagatttgggagaagaaaatttcaaagccttggtgttgattgcctttgctcagtatcttcagcagtgtccatttgaagatcatgtaaaattagtgaatgaagtaactgaatttgcaaaaacatgtgttgctgatgagtccgcggaaaattgtgacaaatcacttcataccctttttggagacaaattatgcacagttgcaactcttcgtgaaacctatggtgaaatggctgactgctgtgcaaaacaagaacctgagagaaatgaatgcttcttgcaacacaaagatgacaacccaaacctcccccgattggtgagaccagaggttgatgtgatgtgcactgcttttcatgacaatgaagagacatttttgaaaaaatacttatatgaaattgccagaagacatccttacttttatgccccggaactccttttctttgctaaaaggtataaagctgcttttacagaatgttgccaagctgctgataaagctgcctgcctgttgccaaagctcgatgaacttcgggatgaagggaaggctagctctgccaaacagagactcaagtgtgccagtctccaaaaatttggagaaagagctttcaaagcatgggcagtagctcgcctgagccagagatttcccaaagctgagtttgcagaagtttccaagttagtgacagatcttaccaaagtccacacggaatgctgccatggagatctgctcgagtgtgctgatgacagggcggaccttgccaagtatatctgtgaaaatcaagattcgatctccagtaaactgaaggaatgctgtgaaaaacctctgttggaaaaatcccactgcattgccgaagtggaaaatgatgagatgcctgctgacttgccttcattagctgctgattttgttgaaagtaaggatgtttgcaaaaactatgctgaggcaaaggatgtcttcctgggcatgtttttgtatgaatatgcaagaaggcatcctgattactctgtcgtgctgctgctgagacttgccaagacatatgaaaccactctagagaagtgctgtgccgctgctgatcctcatgaatgctatgccaaagtgttcgatgaatttaaacctcttgtggaagagcctcagaatttaatcaaacaaaattgtgagctttttgagcagcttggagagtacaaattccagaatgcgctattagttcgttacaccaagaaagtaccccaagtgtcaactccaactcttgtagaggtctcaagaaacctaggaaaagtgggatccaaatgttgtaaacatcctgaagcaaaaagaatgccctgtgcagaagactatctatccgtggtcctgaaccagttatgtgtgttgcatgagaaaacgccagtaagtgacagagtcaccaaatgctgcacagaatccttggtgaacaggcgaccatgcttttcagctctggaagtcgacgaaacatacgttcccaaagagtttaatgcttgtacattcaccttccatgcagatatatgcacactttctgagaaggagagacaaatcaagaaacaaactgcacttgttgagctcgtgaaacacaagcccaaggcaacaaaagagcaactgaaagctgttatggatgatttcgcagcttttgtagagaagtgctgcaaggctgacgataaggagacctgctttgccgaggagggtaaaaaacttgttgctgcaagtcaagctgccttaggcttataa

SEQ ID NO: 32 - DNA, 1758 bp, Artificial sequence
  TA29: HA with L585C
gatgcacacaagagtgaggttgctcatcggtttaaagatttgggagaagaaaatttcaaagccttggtgttgattgcctttgctcagtatcttcagcagtgtccatttgaagatcatgtaaaattagtgaatgaagtaactgaatttgcaaaaacatgtgttgctgatgagtccgcggaaaattgtgacaaatcacttcataccctttttggagacaaattatgcacagttgcaactcttcgtgaaacctatggtgaaatggctgactgctgtgcaaaacaagaacctgagagaaatgaatgcttcttgcaacacaaagatgacaacccaaacctcccccgattggtgagaccagaggttgatgtgatgtgcactgcttttcatgacaatgaagagacatttttgaaaaaatacttatatgaaattgccagaagacatccttacttttatgccccggaactccttttctttgctaaaaggtataaagctgcttttacagaatgttgccaagctgctgataaagctgcctgcctgttgccaaagctcgatgaacttcgggatgaagggaaggctagctctgccaaacagagactcaagtgtgccagtctccaaaaatttggagaaagagctttcaaagcatgggcagtagctcgcctgagccagagatttcccaaagctgagtttgcagaagtttccaagttagtgacagatcttaccaaagtccacacggaatgctgccatggagatctgctcgagtgtgctgatgacagggcggaccttgccaagtatatctgtgaaaatcaagattcgatctccagtaaactgaaggaatgctgtgaaaaacctctgttggaaaaatcccactgcattgccgaagtggaaaatgatgagatgcctgctgacttgccttcattagctgctgattttgttgaaagtaaggatgtttgcaaaaactatgctgaggcaaaggatgtcttcctgggcatgtttttgtatgaatatgcaagaaggcatcctgattactctgtcgtgctgctgctgagacttgccaagacatatgaaaccactctagagaagtgctgtgccgctgctgatcctcatgaatgctatgccaaagtgttcgatgaatttaaacctcttgtggaagagcctcagaatttaatcaaacaaaattgtgagctttttgagcagcttggagagtacaaattccagaatgcgctattagttcgttacaccaagaaagtaccccaagtgtcaactccaactcttgtagaggtctcaagaaacctaggaaaagtgggatccaaatgttgtaaacatcctgaagcaaaaagaatgccctgtgcagaagactatctatccgtggtcctgaaccagttatgtgtgttgcatgagaaaacgccagtaagtgacagagtcaccaaatgctgcacagaatccttggtgaacaggcgaccatgcttttcagctctggaagtcgacgaaacatacgttcccaaagagtttaatgctgaaacattcaccttccatgcagatatatgcacactttctgagaaggagagacaaatcaagaaacaaactgcacttgttgagctcgtgaaacacaagcccaaggcaacaaaagagcaactgaaagctgttatggatgatttcgcagcttttgtagagaagtgctgcaaggctgacgataaggagacctgctttgccgaggagggtaaaaaacttgttgctgcaagtcaagctgccttaggctgttaa

SEQ ID NO: 33 - DNA, 1758 bp, Artificial sequence
  TA33: HA with A2C and L585C
gattgtcacaagagtgaggttgctcatcggtttaaagatttgggagaagaaaatttcaaagccttggtgttgattgcctttgctcagtatcttcagcagtgtccatttgaagatcatgtaaaattagtgaatgaagtaactgaatttgcaaaaacatgtgttgctgatgagtccgcggaaaattgtgacaaatcacttcataccctttttggagacaaattatgcacagttgcaactcttcgtgaaacctatggtgaaatggctgactgctgtgcaaaacaagaacctgagagaaatgaatgcttcttgcaacacaaagatgacaacccaaacctcccccgattggtgagaccagaggttgatgtgatgtgcactgcttttcatgacaatgaagagacatttttgaaaaaatacttatatgaaattgccagaagacatccttacttttatgccccggaactccttttctttgctaaaaggtataaagctgcttttacagaatgttgccaagctgctgataaagctgcctgcctgttgccaaagctcgatgaacttcgggatgaagggaaggctagctctgccaaacagagactcaagtgtgccagtctccaaaaatttggagaaagagctttcaaagcatgggcagtagctcgcctgagccagagatttcccaaagctgagtttgcagaagtttccaagttagtgacagatcttaccaaagtccacacggaatgctgccatggagatctgctcgagtgtgctgatgacagggcggaccttgccaagtatatctgtgaaaatcaagattcgatctccagtaaactgaaggaatgctgtgaaaaacctctgttggaaaaatcccactgcattgccgaagtggaaaatgatgagatgcctgctgacttgccttcattagctgctgattttgttgaaagtaaggatgtttgcaaaaactatgctgaggcaaaggatgtcttcctgggcatgtttttgtatgaatatgcaagaaggcatcctgattactctgtcgtgctgctgctgagacttgccaagacatatgaaaccactctagagaagtgctgtgccgctgctgatcctcatgaatgctatgccaaagtgttcgatgaatttaaacctcttgtggaagagcctcagaatttaatcaaacaaaattgtgagctttttgagcagcttggagagtacaaattccagaatgcgctattagttcgttacaccaagaaagtaccccaagtgtcaactccaactcttgtagaggtctcaagaaacctaggaaaagtgggatccaaatgttgtaaacatcctgaagcaaaaagaatgccctgtgcagaagactatctatccgtggtcctgaaccagttatgtgtgttgcatgagaaaacgccagtaagtgacagagtcaccaaatgctgcacagaatccttggtgaacaggcgaccatgcttttcagctctggaagtcgacgaaacatacgttcccaaagagtttaatgctgaaacattcaccttccatgcagatatatgcacactttctgagaaggagagacaaatcaagaaacaaactgcacttgttgagctcgtgaaacacaagcccaaggcaacaaaagagcaactgaaagctgttatggatgatttcgcagcttttgtagagaagtgctgcaaggctgacgataaggagacctgctttgccgaggagggtaaaaaacttgttgctgcaagtcaagctgccttaggctgttaa

SEQ ID NO: 34 - DNA, 1758 bp, Artificial sequence
  TA34: HA with A2C and A504C
gattgtcacaagagtgaggttgctcatcggtttaaagatttgggagaagaaaatttcaaagccttggtgttgattgcctttgctcagtatcttcagcagtgtccatttgaagatcatgtaaaattagtgaatgaagtaactgaatttgcaaaaacatgtgttgctgatgagtccgcggaaaattgtgacaaatcacttcataccctttttggagacaaattatgcacagttgcaactcttcgtgaaacctatggtgaaatggctgactgctgtgcaaaacaagaacctgagagaaatgaatgcttcttgcaacacaaagatgacaacccaaacctcccccgattggtgagaccagaggttgatgtgatgtgcactgcttttcatgacaatgaagagacatttttgaaaaaatacttatatgaaattgccagaagacatccttacttttatgccccggaactccttttctttgctaaaaggtataaagctgcttttacagaatgttgccaagctgctgataaagctgcctgcctgttgccaaagctcgatgaacttcgggatgaagggaaggctagctctgccaaacagagactcaagtgtgccagtctccaaaaatttggagaaagagctttcaaagcatgggcagtagctcgcctgagccagagatttcccaaagctgagtttgcagaagtttccaagttagtgacagatcttaccaaagtccacacggaatgctgccatggagatctgctcgagtgtgctgatgacagggcggaccttgccaagtatatctgtgaaaatcaagattcgatctccagtaaactgaaggaatgctgtgaaaaacctctgttggaaaaatcccactgcattgccgaagtggaaaatgatgagatgcctgctgacttgccttcattagctgctgattttgttgaaagtaaggatgtttgcaaaaactatgctgaggcaaaggatgtcttcctgggcatgtttttgtatgaatatgcaagaaggcatcctgattactctgtcgtgctgctgctgagacttgccaagacatatgaaaccactctagagaagtgctgtgccgctgctgatcctcatgaatgctatgccaaagtgttcgatgaatttaaacctcttgtggaagagcctcagaatttaatcaaacaaaattgtgagctttttgagcagcttggagagtacaaattccagaatgcgctattagttcgttacaccaagaaagtaccccaagtgtcaactccaactcttgtagaggtctcaagaaacctaggaaaagtgggatccaaatgttgtaaacatcctgaagcaaaaagaatgccctgtgcagaagactatctatccgtggtcctgaaccagttatgtgtgttgcatgagaaaacgccagtaagtgacagagtcaccaaatgctgcacagaatccttggtgaacaggcgaccatgcttttcagctctggaagtcgacgaaacatacgttcccaaagagtttaattgtgaaacattcaccttccatgcagatatatgcacactttctgagaaggagagacaaatcaagaaacaaactgcacttgttgagctcgtgaaacacaagcccaaggcaacaaaagagcaactgaaagctgttatggatgatttcgcagcttttgtagagaagtgctgcaaggctgacgataaggagacctgctttgccgaggagggtaaaaaacttgttgctgcaagtcaagctgccttaggcttataa

SEQ ID NO: 35 - DNA, 1758 bp, Artificial sequence
  TA35: HA with A2C, A364C and D562C
gattgtcacaagagtgaggttgctcatcggtttaaagatttgggagaagaaaatttcaaagccttggtgttgattgcctttgctcagtatcttcagcagtgtccatttgaagatcatgtaaaattagtgaatgaagtaactgaatttgcaaaaacatgtgttgctgatgagtccgcggaaaattgtgacaaatcacttcataccctttttggagacaaattatgcacagttgcaactcttcgtgaaacctatggtgaaatggctgactgctgtgcaaaacaagaacctgagagaaatgaatgcttcttgcaacacaaagatgacaacccaaacctcccccgattggtgagaccagaggttgatgtgatgtgcactgcttttcatgacaatgaagagacatttttgaaaaaatacttatatgaaattgccagaagacatccttacttttatgccccggaactccttttctttgctaaaaggtataaagctgcttttacagaatgttgccaagctgctgataaagctgcctgcctgttgccaaagctcgatgaacttcgggatgaagggaaggctagctctgccaaacagagactcaagtgtgccagtctccaaaaatttggagaaagagctttcaaagcatgggcagtagctcgcctgagccagagatttcccaaagctgagtttgcagaagtttccaagttagtgacagatcttaccaaagtccacacggaatgctgccatggagatctgctcgagtgtgctgatgacagggcggaccttgccaagtatatctgtgaaaatcaagattcgatctccagtaaactgaaggaatgctgtgaaaaacctctgttggaaaaatcccactgcattgccgaagtggaaaatgatgagatgcctgctgacttgccttcattagctgctgattttgttgaaagtaaggatgtttgcaaaaactatgctgaggcaaaggatgtcttcctgggcatgtttttgtatgaatatgcaagaaggcatcctgattactctgtcgtgctgctgctgagacttgccaagacatatgaaaccactctagagaagtgctgtgccgcttgtgatcctcatgaatgctatgccaaagtgttcgatgaatttaaacctcttgtggaagagcctcagaatttaatcaaacaaaattgtgagctttttgagcagcttggagagtacaaattccagaatgcgctattagttcgttacaccaagaaagtaccccaagtgtcaactccaactcttgtagaggtctcaagaaacctaggaaaagtgggatccaaatgttgtaaacatcctgaagcaaaaagaatgccctgtgcagaagactatctatccgtggtcctgaaccagttatgtgtgttgcatgagaaaacgccagtaagtgacagagtcaccaaatgctgcacagaatccttggtgaacaggcgaccatgcttttcagctctggaagtcgacgaaacatacgttcccaaagagtttaatgctgaaacattcaccttccatgcagatatatgcacactttctgagaaggagagacaaatcaagaaacaaactgcacttgttgagctcgtgaaacacaagcccaaggcaacaaaagagcaactgaaagctgttatggatgatttcgcagcttttgtagagaagtgctgcaaggcttgtgataaggagacctgctttgccgaggagggtaaaaaacttgttgctgcaagtcaagctgccttaggcttataa

SEQ ID NO: 36 - DNA, 1758 bp, Artificial sequence
  TA36: HA with A2C, C34A, A364C and D562C
gattgtcacaagagtgaggttgctcatcggtttaaagatttgggagaagaaaatttcaaagccttggtgttgattgcctttgctcagtatcttcagcaggctccatttgaagatcatgtaaaattagtgaatgaagtaactgaatttgcaaaaacatgtgttgctgatgagtccgcggaaaattgtgacaaatcacttcataccctttttggagacaaattatgcacagttgcaactcttcgtgaaacctatggtgaaatggctgactgctgtgcaaaacaagaacctgagagaaatgaatgcttcttgcaacacaaagatgacaacccaaacctcccccgattggtgagaccagaggttgatgtgatgtgcactgcttttcatgacaatgaagagacatttttgaaaaaatacttatatgaaattgccagaagacatccttacttttatgccccggaactccttttctttgctaaaaggtataaagctgcttttacagaatgttgccaagctgctgataaagctgcctgcctgttgccaaagctcgatgaacttcgggatgaagggaaggctagctctgccaaacagagactcaagtgtgccagtctccaaaaatttggagaaagagctttcaaagcatgggcagtagctcgcctgagccagagatttcccaaagctgagtttgcagaagtttccaagttagtgacagatcttaccaaagtccacacggaatgctgccatggagatctgctcgagtgtgctgatgacagggcggaccttgccaagtatatctgtgaaaatcaagattcgatctccagtaaactgaaggaatgctgtgaaaaacctctgttggaaaaatcccactgcattgccgaagtggaaaatgatgagatgcctgctgacttgccttcattagctgctgattttgttgaaagtaaggatgtttgcaaaaactatgctgaggcaaaggatgtcttcctgggcatgtttttgtatgaatatgcaagaaggcatcctgattactctgtcgtgctgctgctgagacttgccaagacatatgaaaccactctagagaagtgctgtgccgcttgtgatcctcatgaatgctatgccaaagtgttcgatgaatttaaacctcttgtggaagagcctcagaatttaatcaaacaaaattgtgagctttttgagcagcttggagagtacaaattccagaatgcgctattagttcgttacaccaagaaagtaccccaagtgtcaactccaactcttgtagaggtctcaagaaacctaggaaaagtgggatccaaatgttgtaaacatcctgaagcaaaaagaatgccctgtgcagaagactatctatccgtggtcctgaaccagttatgtgtgttgcatgagaaaacgccagtaagtgacagagtcaccaaatgctgcacagaatccttggtgaacaggcgaccatgcttttcagctctggaagtcgacgaaacatacgttcccaaagagtttaatgctgaaacattcaccttccatgcagatatatgcacactttctgagaaggagagacaaatcaagaaacaaactgcacttgttgagctcgtgaaacacaagcccaaggcaacaaaagagcaactgaaagctgttatggatgatttcgcagcttttgtagagaagtgctgcaaggcttgtgataaggagacctgctttgccgaggagggtaaaaaacttgttgctgcaagtcaagctgccttaggcttataa

SEQ ID NO: 37 - DNA, 1758 bp, Artificial sequence
  TA38: HA withA2C, A364C, D562C and L585C
gattgtcacaagagtgaggttgctcatcggtttaaagatttgggagaagaaaatttcaaagccttggtgttgattgcctttgctcagtatcttcagcagtgtccatttgaagatcatgtaaaattagtgaatgaagtaactgaatttgcaaaaacatgtgttgctgatgagtccgcggaaaattgtgacaaatcacttcataccctttttggagacaaattatgcacagttgcaactcttcgtgaaacctatggtgaaatggctgactgctgtgcaaaacaagaacctgagagaaatgaatgcttcttgcaacacaaagatgacaacccaaacctcccccgattggtgagaccagaggttgatgtgatgtgcactgcttttcatgacaatgaagagacatttttgaaaaaatacttatatgaaattgccagaagacatccttacttttatgccccggaactccttttctttgctaaaaggtataaagctgcttttacagaatgttgccaagctgctgataaagctgcctgcctgttgccaaagctcgatgaacttcgggatgaagggaaggctagctctgccaaacagagactcaagtgtgccagtctccaaaaatttggagaaagagctttcaaagcatgggcagtagctcgcctgagccagagatttcccaaagctgagtttgcagaagtttccaagttagtgacagatcttaccaaagtccacacggaatgctgccatggagatctgctcgagtgtgctgatgacagggcggaccttgccaagtatatctgtgaaaatcaagattcgatctccagtaaactgaaggaatgctgtgaaaaacctctgttggaaaaatcccactgcattgccgaagtggaaaatgatgagatgcctgctgacttgccttcattagctgctgattttgttgaaagtaaggatgtttgcaaaaactatgctgaggcaaaggatgtcttcctgggcatgtttttgtatgaatatgcaagaaggcatcctgattactctgtcgtgctgctgctgagacttgccaagacatatgaaaccactctagagaagtgctgtgccgcttgtgatcctcatgaatgctatgccaaagtgttcgatgaatttaaacctcttgtggaagagcctcagaatttaatcaaacaaaattgtgagctttttgagcagcttggagagtacaaattccagaatgcgctattagttcgttacaccaagaaagtaccccaagtgtcaactccaactcttgtagaggtctcaagaaacctaggaaaagtgggatccaaatgttgtaaacatcctgaagcaaaaagaatgccctgtgcagaagactatctatccgtggtcctgaaccagttatgtgtgttgcatgagaaaacgccagtaagtgacagagtcaccaaatgctgcacagaatccttggtgaacaggcgaccatgcttttcagctctggaagtcgacgaaacatacgttcccaaagagtttaatgctgaaacattcaccttccatgcagatatatgcacactttctgagaaggagagacaaatcaagaaacaaactgcacttgttgagctcgtgaaacacaagcccaaggcaacaaaagagcaactgaaagctgttatggatgatttcgcagcttttgtagagaagtgctgcaaggcttgtgataaggagacctgctttgccgaggagggtaaaaaacttgttgctgcaagtcaagctgccttaggctgttaa

SEQ ID NO: 38 - DNA, 1758 bp, Artificial sequence
  TA39: HA with C34A, A504C and E505C.
gatgcacacaagagtgaggttgctcatcggtttaaagatttgggagaagaaaatttcaaagccttggtgttgattgcctttgctcagtatcttcagcaggctccatttgaagatcatgtaaaattagtgaatgaagtaactgaatttgcaaaaacatgtgttgctgatgagtccgcggaaaattgtgacaaatcacttcataccctttttggagacaaattatgcacagttgcaactcttcgtgaaacctatggtgaaatggctgactgctgtgcaaaacaagaacctgagagaaatgaatgcttcttgcaacacaaagatgacaacccaaacctcccccgattggtgagaccagaggttgatgtgatgtgcactgcttttcatgacaatgaagagacatttttgaaaaaatacttatatgaaattgccagaagacatccttacttttatgccccggaactccttttctttgctaaaaggtataaagctgcttttacagaatgttgccaagctgctgataaagctgcctgcctgttgccaaagctcgatgaacttcgggatgaagggaaggctagctctgccaaacagagactcaagtgtgccagtctccaaaaatttggagaaagagctttcaaagcatgggcagtagctcgcctgagccagagatttcccaaagctgagtttgcagaagtttccaagttagtgacagatcttaccaaagtccacacggaatgctgccatggagatctgctcgagtgtgctgatgacagggcggaccttgccaagtatatctgtgaaaatcaagattcgatctccagtaaactgaaggaatgctgtgaaaaacctctgttggaaaaatcccactgcattgccgaagtggaaaatgatgagatgcctgctgacttgccttcattagctgctgattttgttgaaagtaaggatgtttgcaaaaactatgctgaggcaaaggatgtcttcctgggcatgtttttgtatgaatatgcaagaaggcatcctgattactctgtcgtgctgctgctgagacttgccaagacatatgaaaccactctagagaagtgctgtgccgctgctgatcctcatgaatgctatgccaaagtgttcgatgaatttaaacctcttgtggaagagcctcagaatttaatcaaacaaaattgtgagctttttgagcagcttggagagtacaaattccagaatgcgctattagttcgttacaccaagaaagtaccccaagtgtcaactccaactcttgtagaggtctcaagaaacctaggaaaagtgggatccaaatgttgtaaacatcctgaagcaaaaagaatgccctgtgcagaagactatctatccgtggtcctgaaccagttatgtgtgttgcatgagaaaacgccagtaagtgacagagtcaccaaatgctgcacagaatccttggtgaacaggcgaccatgcttttcagctctggaagtcgacgaaacatacgttcccaaagagtttaattgttgtacattcaccttccatgcagatatatgcacactttctgagaaggagagacaaatcaagaaacaaactgcacttgttgagctcgtgaaacacaagcccaaggcaacaaaagagcaactgaaagctgttatggatgatttcgcagcttttgtagagaagtgctgcaaggctgacgataaggagacctgctttgccgaggagggtaaaaaacttgttgctgcaagtcaagctgccttaggcttataa

SEQ ID NO: 39 - DNA, 1758 bp, Artificial sequence
  TA41: HA with S270C and A581C
gatgcacacaagagtgaggttgctcatcggtttaaagatttgggagaagaaaatttcaaagccttggtgttgattgcctttgctcagtatcttcagcagtgtccatttgaagatcatgtaaaattagtgaatgaagtaactgaatttgcaaaaacatgtgttgctgatgagtccgcggaaaattgtgacaaatcacttcataccctttttggagacaaattatgcacagttgcaactcttcgtgaaacctatggtgaaatggctgactgctgtgcaaaacaagaacctgagagaaatgaatgcttcttgcaacacaaagatgacaacccaaacctcccccgattggtgagaccagaggttgatgtgatgtgcactgcttttcatgacaatgaagagacatttttgaaaaaatacttatatgaaattgccagaagacatccttacttttatgccccggaactccttttctttgctaaaaggtataaagctgcttttacagaatgttgccaagctgctgataaagctgcctgcctgttgccaaagctcgatgaacttcgggatgaagggaaggctagctctgccaaacagagactcaagtgtgccagtctccaaaaatttggagaaagagctttcaaagcatgggcagtagctcgcctgagccagagatttcccaaagctgagtttgcagaagtttccaagttagtgacagatcttaccaaagtccacacggaatgctgccatggagatctgctcgagtgtgctgatgacagggcggaccttgccaagtatatctgtgaaaatcaagattgtatctccagtaaactgaaggaatgctgtgaaaaacctctgttggaaaaatcccactgcattgccgaagtggaaaatgatgagatgcctgctgacttgccttcattagctgctgattttgttgaaagtaaggatgtttgcaaaaactatgctgaggcaaaggatgtcttcctgggcatgtttttgtatgaatatgcaagaaggcatcctgattactctgtcgtgctgctgctgagacttgccaagacatatgaaaccactctagagaagtgctgtgccgctgctgatcctcatgaatgctatgccaaagtgttcgatgaatttaaacctcttgtggaagagcctcagaatttaatcaaacaaaattgtgagctttttgagcagcttggagagtacaaattccagaatgcgctattagttcgttacaccaagaaagtaccccaagtgtcaactccaactcttgtagaggtctcaagaaacctaggaaaagtgggatccaaatgttgtaaacatcctgaagcaaaaagaatgccctgtgcagaagactatctatccgtggtcctgaaccagttatgtgtgttgcatgagaaaacgccagtaagtgacagagtcaccaaatgctgcacagaatccttggtgaacaggcgaccatgcttttcagctctggaagtcgacgaaacatacgttcccaaagagtttaatgctgaaacattcaccttccatgcagatatatgcacactttctgagaaggagagacaaatcaagaaacaaactgcacttgttgagctcgtgaaacacaagcccaaggcaacaaaagagcaactgaaagctgttatggatgatttcgcagcttttgtagagaagtgctgcaaggctgacgataaggagacctgctttgccgaggagggtaaaaaacttgttgctgcaagtcaatgtgccttaggcttataa

SEQ ID NO: 40 - DNA, 1758 bp, Artificial sequence
  TA43: HA with D129C, S270C and A581C
gatgcacacaagagtgaggttgctcatcggtttaaagatttgggagaagaaaatttcaaagccttggtgttgattgcctttgctcagtatcttcagcagtgtccatttgaagatcatgtaaaattagtgaatgaagtaactgaatttgcaaaaacatgtgttgctgatgagtccgcggaaaattgtgacaaatcacttcataccctttttggagacaaattatgcacagttgcaactcttcgtgaaacctatggtgaaatggctgactgctgtgcaaaacaagaacctgagagaaatgaatgcttcttgcaacacaaagatgacaacccaaacctcccccgattggtgagaccagaggttgatgtgatgtgcactgcttttcattgtaatgaagagacatttttgaaaaaatacttatatgaaattgccagaagacatccttacttttatgccccggaactccttttctttgctaaaaggtataaagctgcttttacagaatgttgccaagctgctgataaagctgcctgcctgttgccaaagctcgatgaacttcgggatgaagggaaggctagctctgccaaacagagactcaagtgtgccagtctccaaaaatttggagaaagagctttcaaagcatgggcagtagctcgcctgagccagagatttcccaaagctgagtttgcagaagtttccaagttagtgacagatcttaccaaagtccacacggaatgctgccatggagatctgctcgagtgtgctgatgacagggcggaccttgccaagtatatctgtgaaaatcaagattgtatctccagtaaactgaaggaatgctgtgaaaaacctctgttggaaaaatcccactgcattgccgaagtggaaaatgatgagatgcctgctgacttgccttcattagctgctgattttgttgaaagtaaggatgtttgcaaaaactatgctgaggcaaaggatgtcttcctgggcatgtttttgtatgaatatgcaagaaggcatcctgattactctgtcgtgctgctgctgagacttgccaagacatatgaaaccactctagagaagtgctgtgccgctgctgatcctcatgaatgctatgccaaagtgttcgatgaatttaaacctcttgtggaagagcctcagaatttaatcaaacaaaattgtgagctttttgagcagcttggagagtacaaattccagaatgcgctattagttcgttacaccaagaaagtaccccaagtgtcaactccaactcttgtagaggtctcaagaaacctaggaaaagtgggatccaaatgttgtaaacatcctgaagcaaaaagaatgccctgtgcagaagactatctatccgtggtcctgaaccagttatgtgtgttgcatgagaaaacgccagtaagtgacagagtcaccaaatgctgcacagaatccttggtgaacaggcgaccatgcttttcagctctggaagtcgacgaaacatacgttcccaaagagtttaatgctgaaacattcaccttccatgcagatatatgcacactttctgagaaggagagacaaatcaagaaacaaactgcacttgttgagctcgtgaaacacaagcccaaggcaacaaaagagcaactgaaagctgttatggatgatttcgcagcttttgtagagaagtgctgcaaggctgacgataaggagacctgctttgccgaggagggtaaaaaacttgttgctgcaagtcaatgtgccttaggcttataa

SEQ ID NO: 41 - DNA, 1758 bp, Artificial sequence
  TA46: HA with C169S
gatgcacacaagagtgaggttgctcatcggtttaaagatttgggagaagaaaatttcaaagccttggtgttgattgcctttgctcagtatcttcagcagtgtccatttgaagatcatgtaaaattagtgaatgaagtaactgaatttgcaaaaacatgtgttgctgatgagtccgcggaaaattgtgacaaatcacttcataccctttttggagacaaattatgcacagttgcaactcttcgtgaaacctatggtgaaatggctgactgctgtgcaaaacaagaacctgagagaaatgaatgcttcttgcaacacaaagatgacaacccaaacctcccccgattggtgagaccagaggttgatgtgatgtgcactgcttttcatgacaatgaagagacatttttgaaaaaatacttatatgaaattgccagaagacatccttacttttatgccccggaactccttttctttgctaaaaggtataaagctgcttttacagaatgttctcaagctgctgataaagctgcctgcctgttgccaaagctcgatgaacttcgggatgaagggaaggctagctctgccaaacagagactcaagtgtgccagtctccaaaaatttggagaaagagctttcaaagcatgggcagtagctcgcctgagccagagatttcccaaagctgagtttgcagaagtttccaagttagtgacagatcttaccaaagtccacacggaatgctgccatggagatctgctcgagtgtgctgatgacagggcggaccttgccaagtatatctgtgaaaatcaagattcgatctccagtaaactgaaggaatgctgtgaaaaacctctgttggaaaaatcccactgcattgccgaagtggaaaatgatgagatgcctgctgacttgccttcattagctgctgattttgttgaaagtaaggatgttgctaaaaactatgctgaggcaaaggatgtcttcctgggcatgtttttgtatgaatatgcaagaaggcatcctgattactctgtcgtgctgctgctgagacttgccaagacatatgaaaccactctagagaagtgctgtgccgctgctgatcctcatgaatgctatgccaaagtgttcgatgaatttaaacctcttgtggaagagcctcagaatttaatcaaacaaaattgtgagctttttgagcagcttggagagtacaaattccagaatgcgctattagttcgttacaccaagaaagtaccccaagtgtcaactccaactcttgtagaggtctcaagaaacctaggaaaagtgggatccaaatgttgtaaacatcctgaagcaaaaagaatgccctgtgcagaagactatctatccgtggtcctgaaccagttatgtgtgttgcatgagaaaacgccagtaagtgacagagtcaccaaatgctgcacagaatccttggtgaacaggcgaccatgcttttcagctctggaagtcgacgaaacatacgttcccaaagagtttaatgctgaaacattcaccttccatgcagatatatgcacactttctgagaaggagagacaaatcaagaaacaaactgcacttgttgagctcgtgaaacacaagcccaaggcaacaaaagagcaactgaaagctgttatggatgatttcgcagcttttgtagagaagtgctgcaaggctgacgataaggagacctgctttgccgaggagggtaaaaaacttgttgctgcaagtcaagctgccttaggcttataa

SEQ ID NO: 42 - DNA, 1758 bp, Artificial sequence
  TA47: HA with D129C, C360S and L585C
gatgcacacaagagtgaggttgctcatcggtttaaagatttgggagaagaaaatttcaaagccttggtgttgattgcctttgctcagtatcttcagcagtgtccatttgaagatcatgtaaaattagtgaatgaagtaactgaatttgcaaaaacatgtgttgctgatgagtccgcggaaaattgtgacaaatcacttcataccctttttggagacaaattatgcacagttgcaactcttcgtgaaacctatggtgaaatggctgactgctgtgcaaaacaagaacctgagagaaatgaatgcttcttgcaacacaaagatgacaacccaaacctcccccgattggtgagaccagaggttgatgtgatgtgcactgcttttcattgtaatgaagagacatttttgaaaaaatacttatatgaaattgccagaagacatccttacttttatgccccggaactccttttctttgctaaaaggtataaagctgcttttacagaatgttgccaagctgctgataaagctgcctgcctgttgccaaagctcgatgaacttcgggatgaagggaaggctagctctgccaaacagagactcaagtgtgccagtctccaaaaatttggagaaagagctttcaaagcatgggcagtagctcgcctgagccagagatttcccaaagctgagtttgcagaagtttccaagttagtgacagatcttaccaaagtccacacggaatgctgccatggagatctgctcgagtgtgctgatgacagggcggaccttgccaagtatatctgtgaaaatcaagattcgatctccagtaaactgaaggaatgctgtgaaaaacctctgttggaaaaatcccactgcattgccgaagtggaaaatgatgagatgcctgctgacttgccttcattagctgctgattttgttgaaagtaaggatgtttgcaaaaactatgctgaggcaaaggatgtcttcctgggcatgtttttgtatgaatatgcaagaaggcatcctgattactctgtcgtgctgctgctgagacttgccaagacatatgaaaccactctagagaagtcttgtgccgctgctgatcctcatgaatgctatgccaaagtgttcgatgaatttaaacctcttgtggaagagcctcagaatttaatcaaacaaaattgtgagctttttgagcagcttggagagtacaaattccagaatgcgctattagttcgttacaccaagaaagtaccccaagtgtcaactccaactcttgtagaggtctcaagaaacctaggaaaagtgggatccaaatgttgtaaacatcctgaagcaaaaagaatgccctgtgcagaagactatctatccgtggtcctgaaccagttatgtgtgttgcatgagaaaacgccagtaagtgacagagtcaccaaatgctgcacagaatccttggtgaacaggcgaccatgcttttcagctctggaagtcgacgaaacatacgttcccaaagagtttaatgctgaaacattcaccttccatgcagatatatgcacactttctgagaaggagagacaaatcaagaaacaaactgcacttgttgagctcgtgaaacacaagcccaaggcaacaaaagagcaactgaaagctgttatggatgatttcgcagcttttgtagagaagtgctgcaaggctgacgataaggagacctgctttgccgaggagggtaaaaaacttgttgctgcaagtcaagctgccttaggctgttaa

SEQ ID NO: 43 - DNA, 1761 bp, Artificial sequence
  TA51: HA with A2C and a cysteine immediately before the stop codon
gattgtcacaagagtgaggttgctcatcggtttaaagatttgggagaagaaaatttcaaagccttggtgttgattgcctttgctcagtatcttcagcagtgtccatttgaagatcatgtaaaattagtgaatgaagtaactgaatttgcaaaaacatgtgttgctgatgagtccgcggaaaattgtgacaaatcacttcataccctttttggagacaaattatgcacagttgcaactcttcgtgaaacctatggtgaaatggctgactgctgtgcaaaacaagaacctgagagaaatgaatgcttcttgcaacacaaagatgacaacccaaacctcccccgattggtgagaccagaggttgatgtgatgtgcactgcttttcatgacaatgaagagacatttttgaaaaaatacttatatgaaattgccagaagacatccttacttttatgccccggaactccttttctttgctaaaaggtataaagctgcttttacagaatgttgccaagctgctgataaagctgcctgcctgttgccaaagctcgatgaacttcgggatgaagggaaggctagctctgccaaacagagactcaagtgtgccagtctccaaaaatttggagaaagagctttcaaagcatgggcagtagctcgcctgagccagagatttcccaaagctgagtttgcagaagtttccaagttagtgacagatcttaccaaagtccacacggaatgctgccatggagatctgctcgagtgtgctgatgacagggcggaccttgccaagtatatctgtgaaaatcaagattcgatctccagtaaactgaaggaatgctgtgaaaaacctctgttggaaaaatcccactgcattgccgaagtggaaaatgatgagatgcctgctgacttgccttcattagctgctgattttgttgaaagtaaggatgtttgcaaaaactatgctgaggcaaaggatgtcttcctgggcatgtttttgtatgaatatgcaagaaggcatcctgattactctgtcgtgctgctgctgagacttgccaagacatatgaaaccactctagagaagtgctgtgccgctgctgatcctcatgaatgctatgccaaagtgttcgatgaatttaaacctcttgtggaagagcctcagaatttaatcaaacaaaattgtgagctttttgagcagcttggagagtacaaattccagaatgcgctattagttcgttacaccaagaaagtaccccaagtgtcaactccaactcttgtagaggtctcaagaaacctaggaaaagtgggatccaaatgttgtaaacatcctgaagcaaaaagaatgccctgtgcagaagactatctatccgtggtcctgaaccagttatgtgtgttgcatgagaaaacgccagtaagtgacagagtcaccaaatgctgcacagaatccttggtgaacaggcgaccatgcttttcagctctggaagtcgacgaaacatacgttcccaaagagtttaatgctgaaacattcaccttccatgcagatatatgcacactttctgagaaggagagacaaatcaagaaacaaactgcacttgttgagctcgtgaaacacaagcccaaggcaacaaaagagcaactgaaagctgttatggatgatttcgcagcttttgtagagaagtgctgcaaggctgacgataaggagacctgctttgccgaggagggtaaaaaacttgttgctgcaagtcaagctgccttaggcttatgttaa

SEQ ID NO: 44 - DNA, 1761 bp, Artificial sequence
  TA57: HA with A2C and a Cys insertion between G584 and L585
gattgtcacaagagtgaggttgctcatcggtttaaagatttgggagaagaaaatttcaaagccttggtgttgattgcctttgctcagtatcttcagcagtgtccatttgaagatcatgtaaaattagtgaatgaagtaactgaatttgcaaaaacatgtgttgctgatgagtccgcggaaaattgtgacaaatcacttcataccctttttggagacaaattatgcacagttgcaactcttcgtgaaacctatggtgaaatggctgactgctgtgcaaaacaagaacctgagagaaatgaatgcttcttgcaacacaaagatgacaacccaaacctcccccgattggtgagaccagaggttgatgtgatgtgcactgcttttcatgacaatgaagagacatttttgaaaaaatacttatatgaaattgccagaagacatccttacttttatgccccggaactccttttctttgctaaaaggtataaagctgcttttacagaatgttgccaagctgctgataaagctgcctgcctgttgccaaagctcgatgaacttcgggatgaagggaaggctagctctgccaaacagagactcaagtgtgccagtctccaaaaatttggagaaagagctttcaaagcatgggcagtagctcgcctgagccagagatttcccaaagctgagtttgcagaagtttccaagttagtgacagatcttaccaaagtccacacggaatgctgccatggagatctgctcgagtgtgctgatgacagggcggaccttgccaagtatatctgtgaaaatcaagattcgatctccagtaaactgaaggaatgctgtgaaaaacctctgttggaaaaatcccactgcattgccgaagtggaaaatgatgagatgcctgctgacttgccttcattagctgctgattttgttgaaagtaaggatgtttgcaaaaactatgctgaggcaaaggatgtcttcctgggcatgtttttgtatgaatatgcaagaaggcatcctgattactctgtcgtgctgctgctgagacttgccaagacatatgaaaccactctagagaagtgctgtgccgctgctgatcctcatgaatgctatgccaaagtgttcgatgaatttaaacctcttgtggaagagcctcagaatttaatcaaacaaaattgtgagctttttgagcagcttggagagtacaaattccagaatgcgctattagttcgttacaccaagaaagtaccccaagtgtcaactccaactcttgtagaggtctcaagaaacctaggaaaagtgggatccaaatgttgtaaacatcctgaagcaaaaagaatgccctgtgcagaagactatctatccgtggtcctgaaccagttatgtgtgttgcatgagaaaacgccagtaagtgacagagtcaccaaatgctgcacagaatccttggtgaacaggcgaccatgcttttcagctctggaagtcgacgaaacatacgttcccaaagagtttaatgctgaaacattcaccttccatgcagatatatgcacactttctgagaaggagagacaaatcaagaaacaaactgcacttgttgagctcgtgaaacacaagcccaaggcaacaaaagagcaactgaaagctgttatggatgatttcgcagcttttgtagagaagtgctgcaaggctgacgataaggagacctgctttgccgaggagggtaaaaaacttgttgctgcaagtcaagctgccttaggctgtttataa

SEQ ID NO: 45 - DNA, 1755 bp, Artificial sequence
  TA60: HA with A2C deltion of C316
gattgtcacaagagtgaggttgctcatcggtttaaagatttgggagaagaaaatttcaaagccttggtgttgattgcctttgctcagtatcttcagcagtgtccatttgaagatcatgtaaaattagtgaatgaagtaactgaatttgcaaaaacatgtgttgctgatgagtccgcggaaaattgtgacaaatcacttcataccctttttggagacaaattatgcacagttgcaactcttcgtgaaacctatggtgaaatggctgactgctgtgcaaaacaagaacctgagagaaatgaatgcttcttgcaacacaaagatgacaacccaaacctcccccgattggtgagaccagaggttgatgtgatgtgcactgcttttcatgacaatgaagagacatttttgaaaaaatacttatatgaaattgccagaagacatccttacttttatgccccggaactccttttctttgctaaaaggtataaagctgcttttacagaatgttgccaagctgctgataaagctgcctgcctgttgccaaagctcgatgaacttcgggatgaagggaaggctagctctgccaaacagagactcaagtgtgccagtctccaaaaatttggagaaagagctttcaaagcatgggcagtagctcgcctgagccagagatttcccaaagctgagtttgcagaagtttccaagttagtgacagatcttaccaaagtccacacggaatgctgccatggagatctgctcgagtgtgctgatgacagggcggaccttgccaagtatatctgtgaaaatcaagattcgatctccagtaaactgaaggaatgctgtgaaaaacctctgttggaaaaatcccactgcattgccgaagtggaaaatgatgagatgcctgctgacttgccttcattagctgctgattttgttgaaagtaaggatgttaaaaactatgctgaggcaaaggatgtcttcctgggcatgtttttgtatgaatatgcaagaaggcatcctgattactctgtcgtgctgctgctgagacttgccaagacatatgaaaccactctagagaagtgctgtgccgctgctgatcctcatgaatgctatgccaaagtgttcgatgaatttaaacctcttgtggaagagcctcagaatttaatcaaacaaaattgtgagctttttgagcagcttggagagtacaaattccagaatgcgctattagttcgttacaccaagaaagtaccccaagtgtcaactccaactcttgtagaggtctcaagaaacctaggaaaagtgggatccaaatgttgtaaacatcctgaagcaaaaagaatgccctgtgcagaagactatctatccgtggtcctgaaccagttatgtgtgttgcatgagaaaacgccagtaagtgacagagtcaccaaatgctgcacagaatccttggtgaacaggcgaccatgcttttcagctctggaagtcgacgaaacatacgttcccaaagagtttaatgctgaaacattcaccttccatgcagatatatgcacactttctgagaaggagagacaaatcaagaaacaaactgcacttgttgagctcgtgaaacacaagcccaaggcaacaaaagagcaactgaaagctgttatggatgatttcgcagcttttgtagagaagtgctgcaaggctgacgataaggagacctgctttgccgaggagggtaaaaaacttgttgctgcaagtcaagctgccttaggcttataa

SEQ ID NO: 46 - DNA, 1758 bp, Artificial sequence
  TA63: HA with H39C and C253P
gatgcacacaagagtgaggttgctcatcggtttaaagatttgggagaagaaaatttcaaagccttggtgttgattgcctttgctcagtatcttcagcagtgtccatttgaagattgtgtaaaattagtgaatgaagtaactgaatttgcaaaaacatgtgttgctgatgagtccgcggaaaattgtgacaaatcacttcataccctttttggagacaaattatgcacagttgcaactcttcgtgaaacctatggtgaaatggctgactgctgtgcaaaacaagaacctgagagaaatgaatgcttcttgcaacacaaagatgacaacccaaacctcccccgattggtgagaccagaggttgatgtgatgtgcactgcttttcatgacaatgaagagacatttttgaaaaaatacttatatgaaattgccagaagacatccttacttttatgccccggaactccttttctttgctaaaaggtataaagctgcttttacagaatgttgccaagctgctgataaagctgcctgcctgttgccaaagctcgatgaacttcgggatgaagggaaggctagctctgccaaacagagactcaagtgtgccagtctccaaaaatttggagaaagagctttcaaagcatgggcagtagctcgcctgagccagagatttcccaaagctgagtttgcagaagtttccaagttagtgacagatcttaccaaagtccacacggaatgctgccatggagatctgctcgagccagctgatgacagggcggaccttgccaagtatatctgtgaaaatcaagattcgatctccagtaaactgaaggaatgctgtgaaaaacctctgttggaaaaatcccactgcattgccgaagtggaaaatgatgagatgcctgctgacttgccttcattagctgctgattttgttgaaagtaaggatgtttgcaaaaactatgctgaggcaaaggatgtcttcctgggcatgtttttgtatgaatatgcaagaaggcatcctgattactctgtcgtgctgctgctgagacttgccaagacatatgaaaccactctagagaagtgctgtgccgctgctgatcctcatgaatgctatgccaaagtgttcgatgaatttaaacctcttgtggaagagcctcagaatttaatcaaacaaaattgtgagctttttgagcagcttggagagtacaaattccagaatgcgctattagttcgttacaccaagaaagtaccccaagtgtcaactccaactcttgtagaggtctcaagaaacctaggaaaagtgggatccaaatgttgtaaacatcctgaagcaaaaagaatgccctgtgcagaagactatctatccgtggtcctgaaccagttatgtgtgttgcatgagaaaacgccagtaagtgacagagtcaccaaatgctgcacagaatccttggtgaacaggcgaccatgcttttcagctctggaagtcgacgaaacatacgttcccaaagagtttaatgctgaaacattcaccttccatgcagatatatgcacactttctgagaaggagagacaaatcaagaaacaaactgcacttgttgagctcgtgaaacacaagcccaaggcaacaaaagagcaactgaaagctgttatggatgatttcgcagcttttgtagagaagtgctgcaaggctgacgataaggagacctgctttgccgaggagggtaaaaaacttgttgctgcaagtcaagctgccttaggcttataa

SEQ ID NO: 47 - DNA, 1758 bp, Artificial sequence
  TA64: HA with C177F
gatgcacacaagagtgaggttgctcatcggtttaaagatttgggagaagaaaatttcaaagccttggtgttgattgcctttgctcagtatcttcagcagtgtccatttgaagatcatgtaaaattagtgaatgaagtaactgaatttgcaaaaacatgtgttgctgatgagtccgcggaaaattgtgacaaatcacttcataccctttttggagacaaattatgcacagttgcaactcttcgtgaaacctatggtgaaatggctgactgctgtgcaaaacaagaacctgagagaaatgaatgcttcttgcaacacaaagatgacaacccaaacctcccccgattggtgagaccagaggttgatgtgatgtgcactgcttttcatgacaatgaagagacatttttgaaaaaatacttatatgaaattgccagaagacatccttacttttatgccccggaactccttttctttgctaaaaggtataaagctgcttttacagaatgttgccaagctgctgataaagctgcctttctgttgccaaagctcgatgaacttcgggatgaagggaaggctagctctgccaaacagagactcaagtgtgccagtctccaaaaatttggagaaagagctttcaaagcatgggcagtagctcgcctgagccagagatttcccaaagctgagtttgcagaagtttccaagttagtgacagatcttaccaaagtccacacggaatgctgccatggagatctgctcgagtgtgctgatgacagggcggaccttgccaagtatatctgtgaaaatcaagattcgatctccagtaaactgaaggaatgctgtgaaaaacctctgttggaaaaatcccactgcattgccgaagtggaaaatgatgagatgcctgctgacttgccttcattagctgctgattttgttgaaagtaaggatgtttgcaaaaactatgctgaggcaaaggatgtcttcctgggcatgtttttgtatgaatatgcaagaaggcatcctgattactctgtcgtgctgctgctgagacttgccaagacatatgaaaccactctagagaagtgctgtgccgctgctgatcctcatgaatgctatgccaaagtgttcgatgaatttaaacctcttgtggaagagcctcagaatttaatcaaacaaaattgtgagctttttgagcagcttggagagtacaaattccagaatgcgctattagttcgttacaccaagaaagtaccccaagtgtcaactccaactcttgtagaggtctcaagaaacctaggaaaagtgggatccaaatgttgtaaacatcctgaagcaaaaagaatgccctgtgcagaagactatctatccgtggtcctgaaccagttatgtgtgttgcatgagaaaacgccagtaagtgacagagtcaccaaatgctgcacagaatccttggtgaacaggcgaccatgcttttcagctctggaagtcgacgaaacatacgttcccaaagagtttaatgctgaaacattcaccttccatgcagatatatgcacactttctgagaaggagagacaaatcaagaaacaaactgcacttgttgagctcgtgaaacacaagcccaaggcaacaaaagagcaactgaaagctgttatggatgatttcgcagcttttgtagagaagtgctgcaaggctgacgataaggagacctgctttgccgaggagggtaaaaaacttgttgctgcaagtcaagctgccttaggcttataa

SEQ ID NO: 48 - DNA, 1767 bp, Artificial sequence
  TA65: HA with a Cys at the N-terminus and an Ala-Cys extension at the C-terminus
tgtgatgcacacaagagtgaggttgctcatcggtttaaagatttgggagaagaaaatttcaaagccttggtgttgattgcctttgctcagtatcttcagcagtgtccatttgaagatcatgtaaaattagtgaatgaagtaactgaatttgcaaaaacatgtgttgctgatgagtccgcggaaaattgtgacaaatcacttcataccctttttggagacaaattatgcacagttgcaactcttcgtgaaacctatggtgaaatggctgactgctgtgcaaaacaagaacctgagagaaatgaatgcttcttgcaacacaaagatgacaacccaaacctcccccgattggtgagaccagaggttgatgtgatgtgcactgcttttcatgacaatgaagagacatttttgaaaaaatacttatatgaaattgccagaagacatccttacttttatgccccggaactccttttctttgctaaaaggtataaagctgcttttacagaatgttgccaagctgctgataaagctgcctgcctgttgccaaagctcgatgaacttcgggatgaagggaaggctagctctgccaaacagagactcaagtgtgccagtctccaaaaatttggagaaagagctttcaaagcatgggcagtagctcgcctgagccagagatttcccaaagctgagtttgcagaagtttccaagttagtgacagatcttaccaaagtccacacggaatgctgccatggagatctgctcgagtgtgctgatgacagggcggaccttgccaagtatatctgtgaaaatcaagattcgatctccagtaaactgaaggaatgctgtgaaaaacctctgttggaaaaatcccactgcattgccgaagtggaaaatgatgagatgcctgctgacttgccttcattagctgctgattttgttgaaagtaaggatgtttgcaaaaactatgctgaggcaaaggatgtcttcctgggcatgtttttgtatgaatatgcaagaaggcatcctgattactctgtcgtgctgctgctgagacttgccaagacatatgaaaccactctagagaagtgctgtgccgctgctgatcctcatgaatgctatgccaaagtgttcgatgaatttaaacctcttgtggaagagcctcagaatttaatcaaacaaaattgtgagctttttgagcagcttggagagtacaaattccagaatgcgctattagttcgttacaccaagaaagtaccccaagtgtcaactccaactcttgtagaggtctcaagaaacctaggaaaagtgggatccaaatgttgtaaacatcctgaagcaaaaagaatgccctgtgcagaagactatctatccgtggtcctgaaccagttatgtgtgttgcatgagaaaacgccagtaagtgacagagtcaccaaatgctgcacagaatccttggtgaacaggcgaccatgcttttcagctctggaagtcgacgaaacatacgttcccaaagagtttaatgctgaaacattcaccttccatgcagatatatgcacactttctgagaaggagagacaaatcaagaaacaaactgcacttgttgagctcgtgaaacacaagcccaaggcaacaaaagagcaactgaaagctgttatggatgatttcgcagcttttgtagagaagtgctgcaaggctgacgataaggagacctgctttgccgaggagggtaaaaaacttgttgctgcaagtcaagctgccttaggcttagcttgttaa

SEQ ID NO: 49 - protein, 609 aa, Artificial Sequence
  HA with fusion leader sequence
MKWVSFISLLFLFSSAYSRSLDKRDAHKSEVAHRFKDLGEENFKALVLIAFAQYLQQCPFEDHVKLVNEVTEFAKTCVADESAENCDKSLHTLFGDKLCTVATLRETYGEMADCCAKQEPERNECFLQHKDDNPNLPRLVRPEVDVMCTAFHDNEETFLKKYLYEIARRHPYFYAPELLFFAKRYKAAFTECCQAADKAACLLPKLDELRDEGKASSAKQRLKCASLQKFGERAFKAWAVARLSQRFPKAEFAEVSKLVTDLTKVHTECCHGDLLECADDRADLAKYICENQDSISSKLKECCEKPLLEKSHCIAEVENDEMPADLPSLAADFVESKDVCKNYAEAKDVFLGMFLYEYARRHPDYSVVLLLRLAKTYETTLEKCCAAADPHECYAKVFDEFKPLVEEPQNLIKQNCELFEQLGEYKFQNALLVRYTKKVPQVSTPTLVEVSRNLGKVGSKCCKHPEAKRMPCAEDYLSVVLNQLCVLHEKTPVSDRVTKCCTESLVNRRPCFSALEVDETYVPKEFNAETFTFHADICTLSEKERQIKKQTALVELVKHKPKATKEQLKAVMDDFAAFVEKCCKADDKETCFAEEGKKLVAASQAALGL

SEQ ID NO: 50 - protein, 585 aa, Artificial sequence
  TA1: HA with A2C
DCHKSEVAHRFKDLGEENFKALVLIAFAQYLQQCPFEDHVKLVNEVTEFAKTCVADESAENCDKSLHTLFGDKLCTVATLRETYGEMADCCAKQEPERNECFLQHKDDNPNLPRLVRPEVDVMCTAFHDNEETFLKKYLYEIARRHPYFYAPELLFFAKRYKAAFTECCQAADKAACLLPKLDELRDEGKASSAKQRLKCASLQKFGERAFKAWAVARLSQRFPKAEFAEVSKLVTDLTKVHTECCHGDLLECADDRADLAKYICENQDSISSKLKECCEKPLLEKSHCIAEVENDEMPADLPSLAADFVESKDVCKNYAEAKDVFLGMFLYEYARRHPDYSVVLLLRLAKTYETTLEKCCAAADPHECYAKVFDEFKPLVEEPQNLIKQNCELFEQLGEYKFQNALLVRYTKKVPQVSTPTLVEVSRNLGKVGSKCCKHPEAKRMPCAEDYLSVVLNQLCVLHEKTPVSDRVTKCCTESLVNRRPCFSALEVDETYVPKEFNAETFTFHADICTLSEKERQIKKQTALVELVKHKPKATKEQLKAVMDDFAAFVEKCCKADDKETCFAEEGKKLVAASQAALGL

SEQ ID NO: 51 - protein, 585 aa, Artificial sequence
  TA2: HA with  D1C
CAHKSEVAHRFKDLGEENFKALVLIAFAQYLQQCPFEDHVKLVNEVTEFAKTCVADESAENCDKSLHTLFGDKLCTVATLRETYGEMADCCAKQEPERNECFLQHKDDNPNLPRLVRPEVDVMCTAFHDNEETFLKKYLYEIARRHPYFYAPELLFFAKRYKAAFTECCQAADKAACLLPKLDELRDEGKASSAKQRLKCASLQKFGERAFKAWAVARLSQRFPKAEFAEVSKLVTDLTKVHTECCHGDLLECADDRADLAKYICENQDSISSKLKECCEKPLLEKSHCIAEVENDEMPADLPSLAADFVESKDVCKNYAEAKDVFLGMFLYEYARRHPDYSVVLLLRLAKTYETTLEKCCAAADPHECYAKVFDEFKPLVEEPQNLIKQNCELFEQLGEYKFQNALLVRYTKKVPQVSTPTLVEVSRNLGKVGSKCCKHPEAKRMPCAEDYLSVVLNQLCVLHEKTPVSDRVTKCCTESLVNRRPCFSALEVDETYVPKEFNAETFTFHADICTLSEKERQIKKQTALVELVKHKPKATKEQLKAVMDDFAAFVEKCCKADDKETCFAEEGKKLVAASQAALGL

SEQ ID NO: 52 - protein, 585 aa, Artificial sequence
  TA3: HA with C75S
DAHKSEVAHRFKDLGEENFKALVLIAFAQYLQQCPFEDHVKLVNEVTEFAKTCVADESAENCDKSLHTLFGDKLSTVATLRETYGEMADCCAKQEPERNECFLQHKDDNPNLPRLVRPEVDVMCTAFHDNEETFLKKYLYEIARRHPYFYAPELLFFAKRYKAAFTECCQAADKAACLLPKLDELRDEGKASSAKQRLKCASLQKFGERAFKAWAVARLSQRFPKAEFAEVSKLVTDLTKVHTECCHGDLLECADDRADLAKYICENQDSISSKLKECCEKPLLEKSHCIAEVENDEMPADLPSLAADFVESKDVCKNYAEAKDVFLGMFLYEYARRHPDYSVVLLLRLAKTYETTLEKCCAAADPHECYAKVFDEFKPLVEEPQNLIKQNCELFEQLGEYKFQNALLVRYTKKVPQVSTPTLVEVSRNLGKVGSKCCKHPEAKRMPCAEDYLSVVLNQLCVLHEKTPVSDRVTKCCTESLVNRRPCFSALEVDETYVPKEFNAETFTFHADICTLSEKERQIKKQTALVELVKHKPKATKEQLKAVMDDFAAFVEKCCKADDKETCFAEEGKKLVAASQAALGL

SEQ ID NO: 53 - protein, 585 aa, Artificial sequence
  TA4: HA with T79C
DAHKSEVAHRFKDLGEENFKALVLIAFAQYLQQCPFEDHVKLVNEVTEFAKTCVADESAENCDKSLHTLFGDKLCTVACLRETYGEMADCCAKQEPERNECFLQHKDDNPNLPRLVRPEVDVMCTAFHDNEETFLKKYLYEIARRHPYFYAPELLFFAKRYKAAFTECCQAADKAACLLPKLDELRDEGKASSAKQRLKCASLQKFGERAFKAWAVARLSQRFPKAEFAEVSKLVTDLTKVHTECCHGDLLECADDRADLAKYICENQDSISSKLKECCEKPLLEKSHCIAEVENDEMPADLPSLAADFVESKDVCKNYAEAKDVFLGMFLYEYARRHPDYSVVLLLRLAKTYETTLEKCCAAADPHECYAKVFDEFKPLVEEPQNLIKQNCELFEQLGEYKFQNALLVRYTKKVPQVSTPTLVEVSRNLGKVGSKCCKHPEAKRMPCAEDYLSVVLNQLCVLHEKTPVSDRVTKCCTESLVNRRPCFSALEVDETYVPKEFNAETFTFHADICTLSEKERQIKKQTALVELVKHKPKATKEQLKAVMDDFAAFVEKCCKADDKETCFAEEGKKLVAASQAALGL

SEQ ID NO: 54 - protein, 585 aa, Artificial sequence
  TA5: HA with E82C
DAHKSEVAHRFKDLGEENFKALVLIAFAQYLQQCPFEDHVKLVNEVTEFAKTCVADESAENCDKSLHTLFGDKLCTVATLRCTYGEMADCCAKQEPERNECFLQHKDDNPNLPRLVRPEVDVMCTAFHDNEETFLKKYLYEIARRHPYFYAPELLFFAKRYKAAFTECCQAADKAACLLPKLDELRDEGKASSAKQRLKCASLQKFGERAFKAWAVARLSQRFPKAEFAEVSKLVTDLTKVHTECCHGDLLECADDRADLAKYICENQDSISSKLKECCEKPLLEKSHCIAEVENDEMPADLPSLAADFVESKDVCKNYAEAKDVFLGMFLYEYARRHPDYSVVLLLRLAKTYETTLEKCCAAADPHECYAKVFDEFKPLVEEPQNLIKQNCELFEQLGEYKFQNALLVRYTKKVPQVSTPTLVEVSRNLGKVGSKCCKHPEAKRMPCAEDYLSVVLNQLCVLHEKTPVSDRVTKCCTESLVNRRPCFSALEVDETYVPKEFNAETFTFHADICTLSEKERQIKKQTALVELVKHKPKATKEQLKAVMDDFAAFVEKCCKADDKETCFAEEGKKLVAASQAALGL

SEQ ID NO: 55 - protein, 585 aa, Artificial sequence
  TA6: HA with E86C
DAHKSEVAHRFKDLGEENFKALVLIAFAQYLQQCPFEDHVKLVNEVTEFAKTCVADESAENCDKSLHTLFGDKLCTVATLRETYGCMADCCAKQEPERNECFLQHKDDNPNLPRLVRPEVDVMCTAFHDNEETFLKKYLYEIARRHPYFYAPELLFFAKRYKAAFTECCQAADKAACLLPKLDELRDEGKASSAKQRLKCASLQKFGERAFKAWAVARLSQRFPKAEFAEVSKLVTDLTKVHTECCHGDLLECADDRADLAKYICENQDSISSKLKECCEKPLLEKSHCIAEVENDEMPADLPSLAADFVESKDVCKNYAEAKDVFLGMFLYEYARRHPDYSVVLLLRLAKTYETTLEKCCAAADPHECYAKVFDEFKPLVEEPQNLIKQNCELFEQLGEYKFQNALLVRYTKKVPQVSTPTLVEVSRNLGKVGSKCCKHPEAKRMPCAEDYLSVVLNQLCVLHEKTPVSDRVTKCCTESLVNRRPCFSALEVDETYVPKEFNAETFTFHADICTLSEKERQIKKQTALVELVKHKPKATKEQLKAVMDDFAAFVEKCCKADDKETCFAEEGKKLVAASQAALGL

SEQ ID NO: 56 - protein, 585 aa, Artificial sequence
  TA7: HA with C124S
DAHKSEVAHRFKDLGEENFKALVLIAFAQYLQQCPFEDHVKLVNEVTEFAKTCVADESAENCDKSLHTLFGDKLCTVATLRETYGEMADCCAKQEPERNECFLQHKDDNPNLPRLVRPEVDVMSTAFHDNEETFLKKYLYEIARRHPYFYAPELLFFAKRYKAAFTECCQAADKAACLLPKLDELRDEGKASSAKQRLKCASLQKFGERAFKAWAVARLSQRFPKAEFAEVSKLVTDLTKVHTECCHGDLLECADDRADLAKYICENQDSISSKLKECCEKPLLEKSHCIAEVENDEMPADLPSLAADFVESKDVCKNYAEAKDVFLGMFLYEYARRHPDYSVVLLLRLAKTYETTLEKCCAAADPHECYAKVFDEFKPLVEEPQNLIKQNCELFEQLGEYKFQNALLVRYTKKVPQVSTPTLVEVSRNLGKVGSKCCKHPEAKRMPCAEDYLSVVLNQLCVLHEKTPVSDRVTKCCTESLVNRRPCFSALEVDETYVPKEFNAETFTFHADICTLSEKERQIKKQTALVELVKHKPKATKEQLKAVMDDFAAFVEKCCKADDKETCFAEEGKKLVAASQAALGL

SEQ ID NO: 57 - protein, 585 aa, Artificial sequence
  TA8: HA with C168S
DAHKSEVAHRFKDLGEENFKALVLIAFAQYLQQCPFEDHVKLVNEVTEFAKTCVADESAENCDKSLHTLFGDKLCTVATLRETYGEMADCCAKQEPERNECFLQHKDDNPNLPRLVRPEVDVMCTAFHDNEETFLKKYLYEIARRHPYFYAPELLFFAKRYKAAFTESCQAADKAACLLPKLDELRDEGKASSAKQRLKCASLQKFGERAFKAWAVARLSQRFPKAEFAEVSKLVTDLTKVHTECCHGDLLECADDRADLAKYICENQDSISSKLKECCEKPLLEKSHCIAEVENDEMPADLPSLAADFVESKDVCKNYAEAKDVFLGMFLYEYARRHPDYSVVLLLRLAKTYETTLEKCCAAADPHECYAKVFDEFKPLVEEPQNLIKQNCELFEQLGEYKFQNALLVRYTKKVPQVSTPTLVEVSRNLGKVGSKCCKHPEAKRMPCAEDYLSVVLNQLCVLHEKTPVSDRVTKCCTESLVNRRPCFSALEVDETYVPKEFNAETFTFHADICTLSEKERQIKKQTALVELVKHKPKATKEQLKAVMDDFAAFVEKCCKADDKETCFAEEGKKLVAASQAALGL

SEQ ID NO: 58 - protein, 585 aa, Artificial sequence
  TA9: HA with C169S
DAHKSEVAHRFKDLGEENFKALVLIAFAQYLQQCPFEDHVKLVNEVTEFAKTCVADESAENCDKSLHTLFGDKLCTVATLRETYGEMADCCAKQEPERNECFLQHKDDNPNLPRLVRPEVDVMCTAFHDNEETFLKKYLYEIARRHPYFYAPELLFFAKRYKAAFTECSQAADKAACLLPKLDELRDEGKASSAKQRLKCASLQKFGERAFKAWAVARLSQRFPKAEFAEVSKLVTDLTKVHTECCHGDLLECADDRADLAKYICENQDSISSKLKECCEKPLLEKSHCIAEVENDEMPADLPSLAADFVESKDVCKNYAEAKDVFLGMFLYEYARRHPDYSVVLLLRLAKTYETTLEKCCAAADPHECYAKVFDEFKPLVEEPQNLIKQNCELFEQLGEYKFQNALLVRYTKKVPQVSTPTLVEVSRNLGKVGSKCCKHPEAKRMPCAEDYLSVVLNQLCVLHEKTPVSDRVTKCCTESLVNRRPCFSALEVDETYVPKEFNAETFTFHADICTLSEKERQIKKQTALVELVKHKPKATKEQLKAVMDDFAAFVEKCCKADDKETCFAEEGKKLVAASQAALGL

SEQ ID NO: 59 - protein, 585 aa, Artificial sequence
  TA10: HA with C91S
DAHKSEVAHRFKDLGEENFKALVLIAFAQYLQQCPFEDHVKLVNEVTEFAKTCVADESAENCDKSLHTLFGDKLCTVATLRETYGEMADCSAKQEPERNECFLQHKDDNPNLPRLVRPEVDVMCTAFHDNEETFLKKYLYEIARRHPYFYAPELLFFAKRYKAAFTECCQAADKAACLLPKLDELRDEGKASSAKQRLKCASLQKFGERAFKAWAVARLSQRFPKAEFAEVSKLVTDLTKVHTECCHGDLLECADDRADLAKYICENQDSISSKLKECCEKPLLEKSHCIAEVENDEMPADLPSLAADFVESKDVCKNYAEAKDVFLGMFLYEYARRHPDYSVVLLLRLAKTYETTLEKCCAAADPHECYAKVFDEFKPLVEEPQNLIKQNCELFEQLGEYKFQNALLVRYTKKVPQVSTPTLVEVSRNLGKVGSKCCKHPEAKRMPCAEDYLSVVLNQLCVLHEKTPVSDRVTKCCTESLVNRRPCFSALEVDETYVPKEFNAETFTFHADICTLSEKERQIKKQTALVELVKHKPKATKEQLKAVMDDFAAFVEKCCKADDKETCFAEEGKKLVAASQAALGL

SEQ ID NO: 60 - protein, 585 aa, Artificial sequence
  TA11: HA with D121C
DAHKSEVAHRFKDLGEENFKALVLIAFAQYLQQCPFEDHVKLVNEVTEFAKTCVADESAENCDKSLHTLFGDKLCTVATLRETYGEMADCCAKQEPERNECFLQHKDDNPNLPRLVRPEVCVMCTAFHDNEETFLKKYLYEIARRHPYFYAPELLFFAKRYKAAFTECCQAADKAACLLPKLDELRDEGKASSAKQRLKCASLQKFGERAFKAWAVARLSQRFPKAEFAEVSKLVTDLTKVHTECCHGDLLECADDRADLAKYICENQDSISSKLKECCEKPLLEKSHCIAEVENDEMPADLPSLAADFVESKDVCKNYAEAKDVFLGMFLYEYARRHPDYSVVLLLRLAKTYETTLEKCCAAADPHECYAKVFDEFKPLVEEPQNLIKQNCELFEQLGEYKFQNALLVRYTKKVPQVSTPTLVEVSRNLGKVGSKCCKHPEAKRMPCAEDYLSVVLNQLCVLHEKTPVSDRVTKCCTESLVNRRPCFSALEVDETYVPKEFNAETFTFHADICTLSEKERQIKKQTALVELVKHKPKATKEQLKAVMDDFAAFVEKCCKADDKETCFAEEGKKLVAASQAALGL

SEQ ID NO: 61 - protein, 585 aa, Artificial sequence
  TA12: HA with D129C
DAHKSEVAHRFKDLGEENFKALVLIAFAQYLQQCPFEDHVKLVNEVTEFAKTCVADESAENCDKSLHTLFGDKLCTVATLRETYGEMADCCAKQEPERNECFLQHKDDNPNLPRLVRPEVDVMCTAFHCNEETFLKKYLYEIARRHPYFYAPELLFFAKRYKAAFTECCQAADKAACLLPKLDELRDEGKASSAKQRLKCASLQKFGERAFKAWAVARLSQRFPKAEFAEVSKLVTDLTKVHTECCHGDLLECADDRADLAKYICENQDSISSKLKECCEKPLLEKSHCIAEVENDEMPADLPSLAADFVESKDVCKNYAEAKDVFLGMFLYEYARRHPDYSVVLLLRLAKTYETTLEKCCAAADPHECYAKVFDEFKPLVEEPQNLIKQNCELFEQLGEYKFQNALLVRYTKKVPQVSTPTLVEVSRNLGKVGSKCCKHPEAKRMPCAEDYLSVVLNQLCVLHEKTPVSDRVTKCCTESLVNRRPCFSALEVDETYVPKEFNAETFTFHADICTLSEKERQIKKQTALVELVKHKPKATKEQLKAVMDDFAAFVEKCCKADDKETCFAEEGKKLVAASQAALGL

SEQ ID NO: 62 - protein, 585 aa, Artificial sequence
  TA13: HA with S270C
DAHKSEVAHRFKDLGEENFKALVLIAFAQYLQQCPFEDHVKLVNEVTEFAKTCVADESAENCDKSLHTLFGDKLCTVATLRETYGEMADCCAKQEPERNECFLQHKDDNPNLPRLVRPEVDVMCTAFHDNEETFLKKYLYEIARRHPYFYAPELLFFAKRYKAAFTECCQAADKAACLLPKLDELRDEGKASSAKQRLKCASLQKFGERAFKAWAVARLSQRFPKAEFAEVSKLVTDLTKVHTECCHGDLLECADDRADLAKYICENQDCISSKLKECCEKPLLEKSHCIAEVENDEMPADLPSLAADFVESKDVCKNYAEAKDVFLGMFLYEYARRHPDYSVVLLLRLAKTYETTLEKCCAAADPHECYAKVFDEFKPLVEEPQNLIKQNCELFEQLGEYKFQNALLVRYTKKVPQVSTPTLVEVSRNLGKVGSKCCKHPEAKRMPCAEDYLSVVLNQLCVLHEKTPVSDRVTKCCTESLVNRRPCFSALEVDETYVPKEFNAETFTFHADICTLSEKERQIKKQTALVELVKHKPKATKEQLKAVMDDFAAFVEKCCKADDKETCFAEEGKKLVAASQAALGL

SEQ ID NO: 63 - protein, 585 aa, Artificial sequence
  TA14: HA with C316A
DAHKSEVAHRFKDLGEENFKALVLIAFAQYLQQCPFEDHVKLVNEVTEFAKTCVADESAENCDKSLHTLFGDKLCTVATLRETYGEMADCCAKQEPERNECFLQHKDDNPNLPRLVRPEVDVMCTAFHDNEETFLKKYLYEIARRHPYFYAPELLFFAKRYKAAFTECCQAADKAACLLPKLDELRDEGKASSAKQRLKCASLQKFGERAFKAWAVARLSQRFPKAEFAEVSKLVTDLTKVHTECCHGDLLECADDRADLAKYICENQDSISSKLKECCEKPLLEKSHCIAEVENDEMPADLPSLAADFVESKDVAKNYAEAKDVFLGMFLYEYARRHPDYSVVLLLRLAKTYETTLEKCCAAADPHECYAKVFDEFKPLVEEPQNLIKQNCELFEQLGEYKFQNALLVRYTKKVPQVSTPTLVEVSRNLGKVGSKCCKHPEAKRMPCAEDYLSVVLNQLCVLHEKTPVSDRVTKCCTESLVNRRPCFSALEVDETYVPKEFNAETFTFHADICTLSEKERQIKKQTALVELVKHKPKATKEQLKAVMDDFAAFVEKCCKADDKETCFAEEGKKLVAASQAALGL

SEQ ID NO: 64 - protein, 585 aa, Artificial sequence
  TA16: HA with C360S
DAHKSEVAHRFKDLGEENFKALVLIAFAQYLQQCPFEDHVKLVNEVTEFAKTCVADESAENCDKSLHTLFGDKLCTVATLRETYGEMADCCAKQEPERNECFLQHKDDNPNLPRLVRPEVDVMCTAFHDNEETFLKKYLYEIARRHPYFYAPELLFFAKRYKAAFTECCQAADKAACLLPKLDELRDEGKASSAKQRLKCASLQKFGERAFKAWAVARLSQRFPKAEFAEVSKLVTDLTKVHTECCHGDLLECADDRADLAKYICENQDSISSKLKECCEKPLLEKSHCIAEVENDEMPADLPSLAADFVESKDVCKNYAEAKDVFLGMFLYEYARRHPDYSVVLLLRLAKTYETTLEKSCAAADPHECYAKVFDEFKPLVEEPQNLIKQNCELFEQLGEYKFQNALLVRYTKKVPQVSTPTLVEVSRNLGKVGSKCCKHPEAKRMPCAEDYLSVVLNQLCVLHEKTPVSDRVTKCCTESLVNRRPCFSALEVDETYVPKEFNAETFTFHADICTLSEKERQIKKQTALVELVKHKPKATKEQLKAVMDDFAAFVEKCCKADDKETCFAEEGKKLVAASQAALGL

SEQ ID NO: 65 - protein, 585 aa, Artificial sequence
  TA17: HA with C361A
DAHKSEVAHRFKDLGEENFKALVLIAFAQYLQQCPFEDHVKLVNEVTEFAKTCVADESAENCDKSLHTLFGDKLCTVATLRETYGEMADCCAKQEPERNECFLQHKDDNPNLPRLVRPEVDVMCTAFHDNEETFLKKYLYEIARRHPYFYAPELLFFAKRYKAAFTECCQAADKAACLLPKLDELRDEGKASSAKQRLKCASLQKFGERAFKAWAVARLSQRFPKAEFAEVSKLVTDLTKVHTECCHGDLLECADDRADLAKYICENQDSISSKLKECCEKPLLEKSHCIAEVENDEMPADLPSLAADFVESKDVCKNYAEAKDVFLGMFLYEYARRHPDYSVVLLLRLAKTYETTLEKCAAAADPHECYAKVFDEFKPLVEEPQNLIKQNCELFEQLGEYKFQNALLVRYTKKVPQVSTPTLVEVSRNLGKVGSKCCKHPEAKRMPCAEDYLSVVLNQLCVLHEKTPVSDRVTKCCTESLVNRRPCFSALEVDETYVPKEFNAETFTFHADICTLSEKERQIKKQTALVELVKHKPKATKEQLKAVMDDFAAFVEKCCKADDKETCFAEEGKKLVAASQAALGL

SEQ ID NO: 66 - protein, 585 aa, Artificial sequence
  TA18: HA with C361S
DAHKSEVAHRFKDLGEENFKALVLIAFAQYLQQCPFEDHVKLVNEVTEFAKTCVADESAENCDKSLHTLFGDKLCTVATLRETYGEMADCCAKQEPERNECFLQHKDDNPNLPRLVRPEVDVMCTAFHDNEETFLKKYLYEIARRHPYFYAPELLFFAKRYKAAFTECCQAADKAACLLPKLDELRDEGKASSAKQRLKCASLQKFGERAFKAWAVARLSQRFPKAEFAEVSKLVTDLTKVHTECCHGDLLECADDRADLAKYICENQDSISSKLKECCEKPLLEKSHCIAEVENDEMPADLPSLAADFVESKDVCKNYAEAKDVFLGMFLYEYARRHPDYSVVLLLRLAKTYETTLEKCSAAADPHECYAKVFDEFKPLVEEPQNLIKQNCELFEQLGEYKFQNALLVRYTKKVPQVSTPTLVEVSRNLGKVGSKCCKHPEAKRMPCAEDYLSVVLNQLCVLHEKTPVSDRVTKCCTESLVNRRPCFSALEVDETYVPKEFNAETFTFHADICTLSEKERQIKKQTALVELVKHKPKATKEQLKAVMDDFAAFVEKCCKADDKETCFAEEGKKLVAASQAALGL

SEQ ID NO: 67 - protein, 585 aa, Artificial sequence
  TA19: HA with A364C
DAHKSEVAHRFKDLGEENFKALVLIAFAQYLQQCPFEDHVKLVNEVTEFAKTCVADESAENCDKSLHTLFGDKLCTVATLRETYGEMADCCAKQEPERNECFLQHKDDNPNLPRLVRPEVDVMCTAFHDNEETFLKKYLYEIARRHPYFYAPELLFFAKRYKAAFTECCQAADKAACLLPKLDELRDEGKASSAKQRLKCASLQKFGERAFKAWAVARLSQRFPKAEFAEVSKLVTDLTKVHTECCHGDLLECADDRADLAKYICENQDSISSKLKECCEKPLLEKSHCIAEVENDEMPADLPSLAADFVESKDVCKNYAEAKDVFLGMFLYEYARRHPDYSVVLLLRLAKTYETTLEKCCAACDPHECYAKVFDEFKPLVEEPQNLIKQNCELFEQLGEYKFQNALLVRYTKKVPQVSTPTLVEVSRNLGKVGSKCCKHPEAKRMPCAEDYLSVVLNQLCVLHEKTPVSDRVTKCCTESLVNRRPCFSALEVDETYVPKEFNAETFTFHADICTLSEKERQIKKQTALVELVKHKPKATKEQLKAVMDDFAAFVEKCCKADDKETCFAEEGKKLVAASQAALGL

SEQ ID NO: 68 - protein, 585 aa, Artificial sequence
  TA20: HA with Q397C
DAHKSEVAHRFKDLGEENFKALVLIAFAQYLQQCPFEDHVKLVNEVTEFAKTCVADESAENCDKSLHTLFGDKLCTVATLRETYGEMADCCAKQEPERNECFLQHKDDNPNLPRLVRPEVDVMCTAFHDNEETFLKKYLYEIARRHPYFYAPELLFFAKRYKAAFTECCQAADKAACLLPKLDELRDEGKASSAKQRLKCASLQKFGERAFKAWAVARLSQRFPKAEFAEVSKLVTDLTKVHTECCHGDLLECADDRADLAKYICENQDSISSKLKECCEKPLLEKSHCIAEVENDEMPADLPSLAADFVESKDVCKNYAEAKDVFLGMFLYEYARRHPDYSVVLLLRLAKTYETTLEKCCAAADPHECYAKVFDEFKPLVEEPQNLIKQNCELFECLGEYKFQNALLVRYTKKVPQVSTPTLVEVSRNLGKVGSKCCKHPEAKRMPCAEDYLSVVLNQLCVLHEKTPVSDRVTKCCTESLVNRRPCFSALEVDETYVPKEFNAETFTFHADICTLSEKERQIKKQTALVELVKHKPKATKEQLKAVMDDFAAFVEKCCKADDKETCFAEEGKKLVAASQAALGL

SEQ ID NO: 69 - protein, 585 aa, Artificial sequence
  TA21: HA with A504C
DAHKSEVAHRFKDLGEENFKALVLIAFAQYLQQCPFEDHVKLVNEVTEFAKTCVADESAENCDKSLHTLFGDKLCTVATLRETYGEMADCCAKQEPERNECFLQHKDDNPNLPRLVRPEVDVMCTAFHDNEETFLKKYLYEIARRHPYFYAPELLFFAKRYKAAFTECCQAADKAACLLPKLDELRDEGKASSAKQRLKCASLQKFGERAFKAWAVARLSQRFPKAEFAEVSKLVTDLTKVHTECCHGDLLECADDRADLAKYICENQDSISSKLKECCEKPLLEKSHCIAEVENDEMPADLPSLAADFVESKDVCKNYAEAKDVFLGMFLYEYARRHPDYSVVLLLRLAKTYETTLEKCCAAADPHECYAKVFDEFKPLVEEPQNLIKQNCELFEQLGEYKFQNALLVRYTKKVPQVSTPTLVEVSRNLGKVGSKCCKHPEAKRMPCAEDYLSVVLNQLCVLHEKTPVSDRVTKCCTESLVNRRPCFSALEVDETYVPKEFNCETFTFHADICTLSEKERQIKKQTALVELVKHKPKATKEQLKAVMDDFAAFVEKCCKADDKETCFAEEGKKLVAASQAALGL

SEQ ID NO: 70 - protein, 585 aa, Artificial sequence
  TA22: HA with A578C
DAHKSEVAHRFKDLGEENFKALVLIAFAQYLQQCPFEDHVKLVNEVTEFAKTCVADESAENCDKSLHTLFGDKLCTVATLRETYGEMADCCAKQEPERNECFLQHKDDNPNLPRLVRPEVDVMCTAFHDNEETFLKKYLYEIARRHPYFYAPELLFFAKRYKAAFTECCQAADKAACLLPKLDELRDEGKASSAKQRLKCASLQKFGERAFKAWAVARLSQRFPKAEFAEVSKLVTDLTKVHTECCHGDLLECADDRADLAKYICENQDSISSKLKECCEKPLLEKSHCIAEVENDEMPADLPSLAADFVESKDVCKNYAEAKDVFLGMFLYEYARRHPDYSVVLLLRLAKTYETTLEKCCAAADPHECYAKVFDEFKPLVEEPQNLIKQNCELFEQLGEYKFQNALLVRYTKKVPQVSTPTLVEVSRNLGKVGSKCCKHPEAKRMPCAEDYLSVVLNQLCVLHEKTPVSDRVTKCCTESLVNRRPCFSALEVDETYVPKEFNAETFTFHADICTLSEKERQIKKQTALVELVKHKPKATKEQLKAVMDDFAAFVEKCCKADDKETCFAEEGKKLVACSQAALGL

SEQ ID NO: 71 - protein, 585 aa, Artificial sequence
  TA23: HA with A581C
DAHKSEVAHRFKDLGEENFKALVLIAFAQYLQQCPFEDHVKLVNEVTEFAKTCVADESAENCDKSLHTLFGDKLCTVATLRETYGEMADCCAKQEPERNECFLQHKDDNPNLPRLVRPEVDVMCTAFHDNEETFLKKYLYEIARRHPYFYAPELLFFAKRYKAAFTECCQAADKAACLLPKLDELRDEGKASSAKQRLKCASLQKFGERAFKAWAVARLSQRFPKAEFAEVSKLVTDLTKVHTECCHGDLLECADDRADLAKYICENQDSISSKLKECCEKPLLEKSHCIAEVENDEMPADLPSLAADFVESKDVCKNYAEAKDVFLGMFLYEYARRHPDYSVVLLLRLAKTYETTLEKCCAAADPHECYAKVFDEFKPLVEEPQNLIKQNCELFEQLGEYKFQNALLVRYTKKVPQVSTPTLVEVSRNLGKVGSKCCKHPEAKRMPCAEDYLSVVLNQLCVLHEKTPVSDRVTKCCTESLVNRRPCFSALEVDETYVPKEFNAETFTFHADICTLSEKERQIKKQTALVELVKHKPKATKEQLKAVMDDFAAFVEKCCKADDKETCFAEEGKKLVAASQCALGL

SEQ ID NO: 72 - protein, 585 aa, Artificial sequence
  TA24: HA with C558S
DAHKSEVAHRFKDLGEENFKALVLIAFAQYLQQCPFEDHVKLVNEVTEFAKTCVADESAENCDKSLHTLFGDKLCTVATLRETYGEMADCCAKQEPERNECFLQHKDDNPNLPRLVRPEVDVMCTAFHDNEETFLKKYLYEIARRHPYFYAPELLFFAKRYKAAFTECCQAADKAACLLPKLDELRDEGKASSAKQRLKCASLQKFGERAFKAWAVARLSQRFPKAEFAEVSKLVTDLTKVHTECCHGDLLECADDRADLAKYICENQDSISSKLKECCEKPLLEKSHCIAEVENDEMPADLPSLAADFVESKDVCKNYAEAKDVFLGMFLYEYARRHPDYSVVLLLRLAKTYETTLEKCCAAADPHECYAKVFDEFKPLVEEPQNLIKQNCELFEQLGEYKFQNALLVRYTKKVPQVSTPTLVEVSRNLGKVGSKCCKHPEAKRMPCAEDYLSVVLNQLCVLHEKTPVSDRVTKCCTESLVNRRPCFSALEVDETYVPKEFNAETFTFHADICTLSEKERQIKKQTALVELVKHKPKATKEQLKAVMDDFAAFVEKSCKADDKETCFAEEGKKLVAASQAALGL

SEQ ID NO: 73 - protein, 585 aa, Artificial sequence
  TA25: HA with C567S
DAHKSEVAHRFKDLGEENFKALVLIAFAQYLQQCPFEDHVKLVNEVTEFAKTCVADESAENCDKSLHTLFGDKLCTVATLRETYGEMADCCAKQEPERNECFLQHKDDNPNLPRLVRPEVDVMCTAFHDNEETFLKKYLYEIARRHPYFYAPELLFFAKRYKAAFTECCQAADKAACLLPKLDELRDEGKASSAKQRLKCASLQKFGERAFKAWAVARLSQRFPKAEFAEVSKLVTDLTKVHTECCHGDLLECADDRADLAKYICENQDSISSKLKECCEKPLLEKSHCIAEVENDEMPADLPSLAADFVESKDVCKNYAEAKDVFLGMFLYEYARRHPDYSVVLLLRLAKTYETTLEKCCAAADPHECYAKVFDEFKPLVEEPQNLIKQNCELFEQLGEYKFQNALLVRYTKKVPQVSTPTLVEVSRNLGKVGSKCCKHPEAKRMPCAEDYLSVVLNQLCVLHEKTPVSDRVTKCCTESLVNRRPCFSALEVDETYVPKEFNAETFTFHADICTLSEKERQIKKQTALVELVKHKPKATKEQLKAVMDDFAAFVEKCCKADDKETSFAEEGKKLVAASQAALGL

SEQ ID NO: 74 - protein, 585 aa, Artificial sequence
  TA26: HA with D549C
DAHKSEVAHRFKDLGEENFKALVLIAFAQYLQQCPFEDHVKLVNEVTEFAKTCVADESAENCDKSLHTLFGDKLCTVATLRETYGEMADCCAKQEPERNECFLQHKDDNPNLPRLVRPEVDVMCTAFHDNEETFLKKYLYEIARRHPYFYAPELLFFAKRYKAAFTECCQAADKAACLLPKLDELRDEGKASSAKQRLKCASLQKFGERAFKAWAVARLSQRFPKAEFAEVSKLVTDLTKVHTECCHGDLLECADDRADLAKYICENQDSISSKLKECCEKPLLEKSHCIAEVENDEMPADLPSLAADFVESKDVCKNYAEAKDVFLGMFLYEYARRHPDYSVVLLLRLAKTYETTLEKCCAAADPHECYAKVFDEFKPLVEEPQNLIKQNCELFEQLGEYKFQNALLVRYTKKVPQVSTPTLVEVSRNLGKVGSKCCKHPEAKRMPCAEDYLSVVLNQLCVLHEKTPVSDRVTKCCTESLVNRRPCFSALEVDETYVPKEFNAETFTFHADICTLSEKERQIKKQTALVELVKHKPKATKEQLKAVMCDFAAFVEKCCKADDKETCFAEEGKKLVAASQAALGL

SEQ ID NO: 75 - protein, 585 aa, Artificial sequence
  TA27: HA with D562C
DAHKSEVAHRFKDLGEENFKALVLIAFAQYLQQCPFEDHVKLVNEVTEFAKTCVADESAENCDKSLHTLFGDKLCTVATLRETYGEMADCCAKQEPERNECFLQHKDDNPNLPRLVRPEVDVMCTAFHDNEETFLKKYLYEIARRHPYFYAPELLFFAKRYKAAFTECCQAADKAACLLPKLDELRDEGKASSAKQRLKCASLQKFGERAFKAWAVARLSQRFPKAEFAEVSKLVTDLTKVHTECCHGDLLECADDRADLAKYICENQDSISSKLKECCEKPLLEKSHCIAEVENDEMPADLPSLAADFVESKDVCKNYAEAKDVFLGMFLYEYARRHPDYSVVLLLRLAKTYETTLEKCCAAADPHECYAKVFDEFKPLVEEPQNLIKQNCELFEQLGEYKFQNALLVRYTKKVPQVSTPTLVEVSRNLGKVGSKCCKHPEAKRMPCAEDYLSVVLNQLCVLHEKTPVSDRVTKCCTESLVNRRPCFSALEVDETYVPKEFNAETFTFHADICTLSEKERQIKKQTALVELVKHKPKATKEQLKAVMDDFAAFVEKCCKACDKETCFAEEGKKLVAASQAALGL

SEQ ID NO: 76 - protein, 585 aa, Artificial sequence
  TA28: HA with E505C
DAHKSEVAHRFKDLGEENFKALVLIAFAQYLQQCPFEDHVKLVNEVTEFAKTCVADESAENCDKSLHTLFGDKLCTVATLRETYGEMADCCAKQEPERNECFLQHKDDNPNLPRLVRPEVDVMCTAFHDNEETFLKKYLYEIARRHPYFYAPELLFFAKRYKAAFTECCQAADKAACLLPKLDELRDEGKASSAKQRLKCASLQKFGERAFKAWAVARLSQRFPKAEFAEVSKLVTDLTKVHTECCHGDLLECADDRADLAKYICENQDSISSKLKECCEKPLLEKSHCIAEVENDEMPADLPSLAADFVESKDVCKNYAEAKDVFLGMFLYEYARRHPDYSVVLLLRLAKTYETTLEKCCAAADPHECYAKVFDEFKPLVEEPQNLIKQNCELFEQLGEYKFQNALLVRYTKKVPQVSTPTLVEVSRNLGKVGSKCCKHPEAKRMPCAEDYLSVVLNQLCVLHEKTPVSDRVTKCCTESLVNRRPCFSALEVDETYVPKEFNACTFTFHADICTLSEKERQIKKQTALVELVKHKPKATKEQLKAVMDDFAAFVEKCCKADDKETCFAEEGKKLVAASQAALGL

SEQ ID NO: 77 - protein, 585 aa, Artificial sequence
  TA29: HA with L585C
DAHKSEVAHRFKDLGEENFKALVLIAFAQYLQQCPFEDHVKLVNEVTEFAKTCVADESAENCDKSLHTLFGDKLCTVATLRETYGEMADCCAKQEPERNECFLQHKDDNPNLPRLVRPEVDVMCTAFHDNEETFLKKYLYEIARRHPYFYAPELLFFAKRYKAAFTECCQAADKAACLLPKLDELRDEGKASSAKQRLKCASLQKFGERAFKAWAVARLSQRFPKAEFAEVSKLVTDLTKVHTECCHGDLLECADDRADLAKYICENQDSISSKLKECCEKPLLEKSHCIAEVENDEMPADLPSLAADFVESKDVCKNYAEAKDVFLGMFLYEYARRHPDYSVVLLLRLAKTYETTLEKCCAAADPHECYAKVFDEFKPLVEEPQNLIKQNCELFEQLGEYKFQNALLVRYTKKVPQVSTPTLVEVSRNLGKVGSKCCKHPEAKRMPCAEDYLSVVLNQLCVLHEKTPVSDRVTKCCTESLVNRRPCFSALEVDETYVPKEFNAETFTFHADICTLSEKERQIKKQTALVELVKHKPKATKEQLKAVMDDFAAFVEKCCKADDKETCFAEEGKKLVAASQAALGC

SEQ ID NO: 78 - protein, 585 aa, Artificial sequence
  TA33: HA with A2C and L585C
DCHKSEVAHRFKDLGEENFKALVLIAFAQYLQQCPFEDHVKLVNEVTEFAKTCVADESAENCDKSLHTLFGDKLCTVATLRETYGEMADCCAKQEPERNECFLQHKDDNPNLPRLVRPEVDVMCTAFHDNEETFLKKYLYEIARRHPYFYAPELLFFAKRYKAAFTECCQAADKAACLLPKLDELRDEGKASSAKQRLKCASLQKFGERAFKAWAVARLSQRFPKAEFAEVSKLVTDLTKVHTECCHGDLLECADDRADLAKYICENQDSISSKLKECCEKPLLEKSHCIAEVENDEMPADLPSLAADFVESKDVCKNYAEAKDVFLGMFLYEYARRHPDYSVVLLLRLAKTYETTLEKCCAAADPHECYAKVFDEFKPLVEEPQNLIKQNCELFEQLGEYKFQNALLVRYTKKVPQVSTPTLVEVSRNLGKVGSKCCKHPEAKRMPCAEDYLSVVLNQLCVLHEKTPVSDRVTKCCTESLVNRRPCFSALEVDETYVPKEFNAETFTFHADICTLSEKERQIKKQTALVELVKHKPKATKEQLKAVMDDFAAFVEKCCKADDKETCFAEEGKKLVAASQAALGC

SEQ ID NO: 79 - protein, 585 aa, Artificial sequence
  TA34: HA with A2C and A504C
DCHKSEVAHRFKDLGEENFKALVLIAFAQYLQQCPFEDHVKLVNEVTEFAKTCVADESAENCDKSLHTLFGDKLCTVATLRETYGEMADCCAKQEPERNECFLQHKDDNPNLPRLVRPEVDVMCTAFHDNEETFLKKYLYEIARRHPYFYAPELLFFAKRYKAAFTECCQAADKAACLLPKLDELRDEGKASSAKQRLKCASLQKFGERAFKAWAVARLSQRFPKAEFAEVSKLVTDLTKVHTECCHGDLLECADDRADLAKYICENQDSISSKLKECCEKPLLEKSHCIAEVENDEMPADLPSLAADFVESKDVCKNYAEAKDVFLGMFLYEYARRHPDYSVVLLLRLAKTYETTLEKCCAAADPHECYAKVFDEFKPLVEEPQNLIKQNCELFEQLGEYKFQNALLVRYTKKVPQVSTPTLVEVSRNLGKVGSKCCKHPEAKRMPCAEDYLSVVLNQLCVLHEKTPVSDRVTKCCTESLVNRRPCFSALEVDETYVPKEFNCETFTFHADICTLSEKERQIKKQTALVELVKHKPKATKEQLKAVMDDFAAFVEKCCKADDKETCFAEEGKKLVAASQAALGL

SEQ ID NO: 80 - protein, 585 aa, Artificial sequence
  TA35: HA with A2C, A364C and D562C
DCHKSEVAHRFKDLGEENFKALVLIAFAQYLQQCPFEDHVKLVNEVTEFAKTCVADESAENCDKSLHTLFGDKLCTVATLRETYGEMADCCAKQEPERNECFLQHKDDNPNLPRLVRPEVDVMCTAFHDNEETFLKKYLYEIARRHPYFYAPELLFFAKRYKAAFTECCQAADKAACLLPKLDELRDEGKASSAKQRLKCASLQKFGERAFKAWAVARLSQRFPKAEFAEVSKLVTDLTKVHTECCHGDLLECADDRADLAKYICENQDSISSKLKECCEKPLLEKSHCIAEVENDEMPADLPSLAADFVESKDVCKNYAEAKDVFLGMFLYEYARRHPDYSVVLLLRLAKTYETTLEKCCAACDPHECYAKVFDEFKPLVEEPQNLIKQNCELFEQLGEYKFQNALLVRYTKKVPQVSTPTLVEVSRNLGKVGSKCCKHPEAKRMPCAEDYLSVVLNQLCVLHEKTPVSDRVTKCCTESLVNRRPCFSALEVDETYVPKEFNAETFTFHADICTLSEKERQIKKQTALVELVKHKPKATKEQLKAVMDDFAAFVEKCCKACDKETCFAEEGKKLVAASQAALGL

SEQ ID NO: 81 - protein, 585 aa, Artificial sequence
  TA36: HA with A2C, A364C and D562C
DCHKSEVAHRFKDLGEENFKALVLIAFAQYLQQAPFEDHVKLVNEVTEFAKTCVADESAENCDKSLHTLFGDKLCTVATLRETYGEMADCCAKQEPERNECFLQHKDDNPNLPRLVRPEVDVMCTAFHDNEETFLKKYLYEIARRHPYFYAPELLFFAKRYKAAFTECCQAADKAACLLPKLDELRDEGKASSAKQRLKCASLQKFGERAFKAWAVARLSQRFPKAEFAEVSKLVTDLTKVHTECCHGDLLECADDRADLAKYICENQDSISSKLKECCEKPLLEKSHCIAEVENDEMPADLPSLAADFVESKDVCKNYAEAKDVFLGMFLYEYARRHPDYSVVLLLRLAKTYETTLEKCCAACDPHECYAKVFDEFKPLVEEPQNLIKQNCELFEQLGEYKFQNALLVRYTKKVPQVSTPTLVEVSRNLGKVGSKCCKHPEAKRMPCAEDYLSVVLNQLCVLHEKTPVSDRVTKCCTESLVNRRPCFSALEVDETYVPKEFNAETFTFHADICTLSEKERQIKKQTALVELVKHKPKATKEQLKAVMDDFAAFVEKCCKACDKETCFAEEGKKLVAASQAALGL

SEQ ID NO: 82 - protein, 585 aa, Artificial sequence
  TA38: HA with A2C, A364C, D562C and L585C
DCHKSEVAHRFKDLGEENFKALVLIAFAQYLQQCPFEDHVKLVNEVTEFAKTCVADESAENCDKSLHTLFGDKLCTVATLRETYGEMADCCAKQEPERNECFLQHKDDNPNLPRLVRPEVDVMCTAFHDNEETFLKKYLYEIARRHPYFYAPELLFFAKRYKAAFTECCQAADKAACLLPKLDELRDEGKASSAKQRLKCASLQKFGERAFKAWAVARLSQRFPKAEFAEVSKLVTDLTKVHTECCHGDLLECADDRADLAKYICENQDSISSKLKECCEKPLLEKSHCIAEVENDEMPADLPSLAADFVESKDVCKNYAEAKDVFLGMFLYEYARRHPDYSVVLLLRLAKTYETTLEKCCAACDPHECYAKVFDEFKPLVEEPQNLIKQNCELFEQLGEYKFQNALLVRYTKKVPQVSTPTLVEVSRNLGKVGSKCCKHPEAKRMPCAEDYLSVVLNQLCVLHEKTPVSDRVTKCCTESLVNRRPCFSALEVDETYVPKEFNAETFTFHADICTLSEKERQIKKQTALVELVKHKPKATKEQLKAVMDDFAAFVEKCCKACDKETCFAEEGKKLVAASQAALGC

SEQ ID NO: 83 - protein, 585 aa, Artificial sequence
  TA39: HA with C34A, A504C and E505C.
DAHKSEVAHRFKDLGEENFKALVLIAFAQYLQQAPFEDHVKLVNEVTEFAKTCVADESAENCDKSLHTLFGDKLCTVATLRETYGEMADCCAKQEPERNECFLQHKDDNPNLPRLVRPEVDVMCTAFHDNEETFLKKYLYEIARRHPYFYAPELLFFAKRYKAAFTECCQAADKAACLLPKLDELRDEGKASSAKQRLKCASLQKFGERAFKAWAVARLSQRFPKAEFAEVSKLVTDLTKVHTECCHGDLLECADDRADLAKYICENQDSISSKLKECCEKPLLEKSHCIAEVENDEMPADLPSLAADFVESKDVCKNYAEAKDVFLGMFLYEYARRHPDYSVVLLLRLAKTYETTLEKCCAAADPHECYAKVFDEFKPLVEEPQNLIKQNCELFEQLGEYKFQNALLVRYTKKVPQVSTPTLVEVSRNLGKVGSKCCKHPEAKRMPCAEDYLSVVLNQLCVLHEKTPVSDRVTKCCTESLVNRRPCFSALEVDETYVPKEFNCCTFTFHADICTLSEKERQIKKQTALVELVKHKPKATKEQLKAVMDDFAAFVEKCCKADDKETCFAEEGKKLVAASQAALGL

SEQ ID NO: 84 - protein, 585 aa, Artificial sequence
  TA41: HA with S270C and A581C
DAHKSEVAHRFKDLGEENFKALVLIAFAQYLQQCPFEDHVKLVNEVTEFAKTCVADESAENCDKSLHTLFGDKLCTVATLRETYGEMADCCAKQEPERNECFLQHKDDNPNLPRLVRPEVDVMCTAFHDNEETFLKKYLYEIARRHPYFYAPELLFFAKRYKAAFTECCQAADKAACLLPKLDELRDEGKASSAKQRLKCASLQKFGERAFKAWAVARLSQRFPKAEFAEVSKLVTDLTKVHTECCHGDLLECADDRADLAKYICENQDCISSKLKECCEKPLLEKSHCIAEVENDEMPADLPSLAADFVESKDVCKNYAEAKDVFLGMFLYEYARRHPDYSVVLLLRLAKTYETTLEKCCAAADPHECYAKVFDEFKPLVEEPQNLIKQNCELFEQLGEYKFQNALLVRYTKKVPQVSTPTLVEVSRNLGKVGSKCCKHPEAKRMPCAEDYLSVVLNQLCVLHEKTPVSDRVTKCCTESLVNRRPCFSALEVDETYVPKEFNAETFTFHADICTLSEKERQIKKQTALVELVKHKPKATKEQLKAVMDDFAAFVEKCCKADDKETCFAEEGKKLVAASQCALGL

SEQ ID NO: 85 - protein, 585 aa, Artificial sequence
  TA43: HA with D129C, S270C and A581C
DAHKSEVAHRFKDLGEENFKALVLIAFAQYLQQCPFEDHVKLVNEVTEFAKTCVADESAENCDKSLHTLFGDKLCTVATLRETYGEMADCCAKQEPERNECFLQHKDDNPNLPRLVRPEVDVMCTAFHCNEETFLKKYLYEIARRHPYFYAPELLFFAKRYKAAFTECCQAADKAACLLPKLDELRDEGKASSAKQRLKCASLQKFGERAFKAWAVARLSQRFPKAEFAEVSKLVTDLTKVHTECCHGDLLECADDRADLAKYICENQDCISSKLKECCEKPLLEKSHCIAEVENDEMPADLPSLAADFVESKDVCKNYAEAKDVFLGMFLYEYARRHPDYSVVLLLRLAKTYETTLEKCCAAADPHECYAKVFDEFKPLVEEPQNLIKQNCELFEQLGEYKFQNALLVRYTKKVPQVSTPTLVEVSRNLGKVGSKCCKHPEAKRMPCAEDYLSVVLNQLCVLHEKTPVSDRVTKCCTESLVNRRPCFSALEVDETYVPKEFNAETFTFHADICTLSEKERQIKKQTALVELVKHKPKATKEQLKAVMDDFAAFVEKCCKADDKETCFAEEGKKLVAASQCALGL

SEQ ID NO: 86 - protein, 585 aa, Artificial sequence
  TA46: HA with C169S
DAHKSEVAHRFKDLGEENFKALVLIAFAQYLQQCPFEDHVKLVNEVTEFAKTCVADESAENCDKSLHTLFGDKLCTVATLRETYGEMADCCAKQEPERNECFLQHKDDNPNLPRLVRPEVDVMCTAFHDNEETFLKKYLYEIARRHPYFYAPELLFFAKRYKAAFTECSQAADKAACLLPKLDELRDEGKASSAKQRLKCASLQKFGERAFKAWAVARLSQRFPKAEFAEVSKLVTDLTKVHTECCHGDLLECADDRADLAKYICENQDSISSKLKECCEKPLLEKSHCIAEVENDEMPADLPSLAADFVESKDVAKNYAEAKDVFLGMFLYEYARRHPDYSVVLLLRLAKTYETTLEKCCAAADPHECYAKVFDEFKPLVEEPQNLIKQNCELFEQLGEYKFQNALLVRYTKKVPQVSTPTLVEVSRNLGKVGSKCCKHPEAKRMPCAEDYLSVVLNQLCVLHEKTPVSDRVTKCCTESLVNRRPCFSALEVDETYVPKEFNAETFTFHADICTLSEKERQIKKQTALVELVKHKPKATKEQLKAVMDDFAAFVEKCCKADDKETCFAEEGKKLVAASQAALGL

SEQ ID NO: 87 - protein, 585 aa, Artificial sequence
  TA47: HA with D129C and L585C
DAHKSEVAHRFKDLGEENFKALVLIAFAQYLQQCPFEDHVKLVNEVTEFAKTCVADESAENCDKSLHTLFGDKLCTVATLRETYGEMADCCAKQEPERNECFLQHKDDNPNLPRLVRPEVDVMCTAFHCNEETFLKKYLYEIARRHPYFYAPELLFFAKRYKAAFTECCQAADKAACLLPKLDELRDEGKASSAKQRLKCASLQKFGERAFKAWAVARLSQRFPKAEFAEVSKLVTDLTKVHTECCHGDLLECADDRADLAKYICENQDSISSKLKECCEKPLLEKSHCIAEVENDEMPADLPSLAADFVESKDVCKNYAEAKDVFLGMFLYEYARRHPDYSVVLLLRLAKTYETTLEKSCAAADPHECYAKVFDEFKPLVEEPQNLIKQNCELFEQLGEYKFQNALLVRYTKKVPQVSTPTLVEVSRNLGKVGSKCCKHPEAKRMPCAEDYLSVVLNQLCVLHEKTPVSDRVTKCCTESLVNRRPCFSALEVDETYVPKEFNAETFTFHADICTLSEKERQIKKQTALVELVKHKPKATKEQLKAVMDDFAAFVEKCCKADDKETCFAEEGKKLVAASQAALGC

SEQ ID NO: 88 - protein, 586 aa, Artificial sequence
  TA51: HA with A2C and a cysteine immediately before the stop codon
DCHKSEVAHRFKDLGEENFKALVLIAFAQYLQQCPFEDHVKLVNEVTEFAKTCVADESAENCDKSLHTLFGDKLCTVATLRETYGEMADCCAKQEPERNECFLQHKDDNPNLPRLVRPEVDVMCTAFHDNEETFLKKYLYEIARRHPYFYAPELLFFAKRYKAAFTECCQAADKAACLLPKLDELRDEGKASSAKQRLKCASLQKFGERAFKAWAVARLSQRFPKAEFAEVSKLVTDLTKVHTECCHGDLLECADDRADLAKYICENQDSISSKLKECCEKPLLEKSHCIAEVENDEMPADLPSLAADFVESKDVCKNYAEAKDVFLGMFLYEYARRHPDYSVVLLLRLAKTYETTLEKCCAAADPHECYAKVFDEFKPLVEEPQNLIKQNCELFEQLGEYKFQNALLVRYTKKVPQVSTPTLVEVSRNLGKVGSKCCKHPEAKRMPCAEDYLSVVLNQLCVLHEKTPVSDRVTKCCTESLVNRRPCFSALEVDETYVPKEFNAETFTFHADICTLSEKERQIKKQTALVELVKHKPKATKEQLKAVMDDFAAFVEKCCKADDKETCFAEEGKKLVAASQAALGLC

SEQ ID NO: 89 - protein, 586 aa, Artificial sequence
  TA57: HA with A2C and an insertion between G584 and L585
DCHKSEVAHRFKDLGEENFKALVLIAFAQYLQQCPFEDHVKLVNEVTEFAKTCVADESAENCDKSLHTLFGDKLCTVATLRETYGEMADCCAKQEPERNECFLQHKDDNPNLPRLVRPEVDVMCTAFHDNEETFLKKYLYEIARRHPYFYAPELLFFAKRYKAAFTECCQAADKAACLLPKLDELRDEGKASSAKQRLKCASLQKFGERAFKAWAVARLSQRFPKAEFAEVSKLVTDLTKVHTECCHGDLLECADDRADLAKYICENQDSISSKLKECCEKPLLEKSHCIAEVENDEMPADLPSLAADFVESKDVCKNYAEAKDVFLGMFLYEYARRHPDYSVVLLLRLAKTYETTLEKCCAAADPHECYAKVFDEFKPLVEEPQNLIKQNCELFEQLGEYKFQNALLVRYTKKVPQVSTPTLVEVSRNLGKVGSKCCKHPEAKRMPCAEDYLSVVLNQLCVLHEKTPVSDRVTKCCTESLVNRRPCFSALEVDETYVPKEFNAETFTFHADICTLSEKERQIKKQTALVELVKHKPKATKEQLKAVMDDFAAFVEKCCKADDKETCFAEEGKKLVAASQAALGCL

SEQ ID NO: 90 - protein, 584 aa, Artificial sequence
  TA60: HA with A2C and deletion of C316
DCHKSEVAHRFKDLGEENFKALVLIAFAQYLQQCPFEDHVKLVNEVTEFAKTCVADESAENCDKSLHTLFGDKLCTVATLRETYGEMADCCAKQEPERNECFLQHKDDNPNLPRLVRPEVDVMCTAFHDNEETFLKKYLYEIARRHPYFYAPELLFFAKRYKAAFTECCQAADKAACLLPKLDELRDEGKASSAKQRLKCASLQKFGERAFKAWAVARLSQRFPKAEFAEVSKLVTDLTKVHTECCHGDLLECADDRADLAKYICENQDSISSKLKECCEKPLLEKSHCIAEVENDEMPADLPSLAADFVESKDVKNYAEAKDVFLGMFLYEYARRHPDYSVVLLLRLAKTYETTLEKCCAAADPHECYAKVFDEFKPLVEEPQNLIKQNCELFEQLGEYKFQNALLVRYTKKVPQVSTPTLVEVSRNLGKVGSKCCKHPEAKRMPCAEDYLSVVLNQLCVLHEKTPVSDRVTKCCTESLVNRRPCFSALEVDETYVPKEFNAETFTFHADICTLSEKERQIKKQTALVELVKHKPKATKEQLKAVMDDFAAFVEKCCKADDKETCFAEEGKKLVAASQAALGL

SEQ ID NO: 91 - protein, 585 aa, Artificial sequence
  TA63: HA with H39C and C253P
DAHKSEVAHRFKDLGEENFKALVLIAFAQYLQQCPFEDCVKLVNEVTEFAKTCVADESAENCDKSLHTLFGDKLCTVATLRETYGEMADCCAKQEPERNECFLQHKDDNPNLPRLVRPEVDVMCTAFHDNEETFLKKYLYEIARRHPYFYAPELLFFAKRYKAAFTECCQAADKAACLLPKLDELRDEGKASSAKQRLKCASLQKFGERAFKAWAVARLSQRFPKAEFAEVSKLVTDLTKVHTECCHGDLLEPADDRADLAKYICENQDSISSKLKECCEKPLLEKSHCIAEVENDEMPADLPSLAADFVESKDVCKNYAEAKDVFLGMFLYEYARRHPDYSVVLLLRLAKTYETTLEKCCAAADPHECYAKVFDEFKPLVEEPQNLIKQNCELFEQLGEYKFQNALLVRYTKKVPQVSTPTLVEVSRNLGKVGSKCCKHPEAKRMPCAEDYLSVVLNQLCVLHEKTPVSDRVTKCCTESLVNRRPCFSALEVDETYVPKEFNAETFTFHADICTLSEKERQIKKQTALVELVKHKPKATKEQLKAVMDDFAAFVEKCCKADDKETCFAEEGKKLVAASQAALGL

SEQ ID NO: 92 - protein, 585 aa, Artificial sequence
  TA64: HA with C177F
DAHKSEVAHRFKDLGEENFKALVLIAFAQYLQQCPFEDHVKLVNEVTEFAKTCVADESAENCDKSLHTLFGDKLCTVATLRETYGEMADCCAKQEPERNECFLQHKDDNPNLPRLVRPEVDVMCTAFHDNEETFLKKYLYEIARRHPYFYAPELLFFAKRYKAAFTECCQAADKAAFLLPKLDELRDEGKASSAKQRLKCASLQKFGERAFKAWAVARLSQRFPKAEFAEVSKLVTDLTKVHTECCHGDLLECADDRADLAKYICENQDSISSKLKECCEKPLLEKSHCIAEVENDEMPADLPSLAADFVESKDVCKNYAEAKDVFLGMFLYEYARRHPDYSVVLLLRLAKTYETTLEKCCAAADPHECYAKVFDEFKPLVEEPQNLIKQNCELFEQLGEYKFQNALLVRYTKKVPQVSTPTLVEVSRNLGKVGSKCCKHPEAKRMPCAEDYLSVVLNQLCVLHEKTPVSDRVTKCCTESLVNRRPCFSALEVDETYVPKEFNAETFTFHADICTLSEKERQIKKQTALVELVKHKPKATKEQLKAVMDDFAAFVEKCCKADDKETCFAEEGKKLVAASQAALGL

SEQ ID NO: 93 - protein, 588 aa, Artificial sequence
  TA65: HA with a Cys at the N-terminus and an Ala-Cys extension at the C-terminus of HA
CDAHKSEVAHRFKDLGEENFKALVLIAFAQYLQQCPFEDHVKLVNEVTEFAKTCVADESAENCDKSLHTLFGDKLCTVATLRETYGEMADCCAKQEPERNECFLQHKDDNPNLPRLVRPEVDVMCTAFHDNEETFLKKYLYEIARRHPYFYAPELLFFAKRYKAAFTECCQAADKAACLLPKLDELRDEGKASSAKQRLKCASLQKFGERAFKAWAVARLSQRFPKAEFAEVSKLVTDLTKVHTECCHGDLLECADDRADLAKYICENQDSISSKLKECCEKPLLEKSHCIAEVENDEMPADLPSLAADFVESKDVCKNYAEAKDVFLGMFLYEYARRHPDYSVVLLLRLAKTYETTLEKCCAAADPHECYAKVFDEFKPLVEEPQNLIKQNCELFEQLGEYKFQNALLVRYTKKVPQVSTPTLVEVSRNLGKVGSKCCKHPEAKRMPCAEDYLSVVLNQLCVLHEKTPVSDRVTKCCTESLVNRRPCFSALEVDETYVPKEFNAETFTFHADICTLSEKERQIKKQTALVELVKHKPKATKEQLKAVMDDFAAFVEKCCKADDKETCFAEEGKKLVAASQAALGLAC

SEQ ID NO: 94 - protein, 607 aa, Bos taurus
MKWVTFISLLLLFSSAYSRGVFRRDTHKSEIAHRFKDLGEEHFKGLVLIAFSQYLQQCPFDEHVKLVNELTEFAKTCVADESHAGCEKSLHTLFGDELCKVASLRETYGDMADCCEKQEPERNECFLSHKDDSPDLPKLKPDPNTLCDEFKADEKKFWGKYLYEIARRHPYFYAPELLYYANKYNGVFQECCQAEDKGACLLPKIETMREKVLASSARQRLRCASIQKFGERALKAWSVARLSQKFPKAEFVEVTKLVTDLTKVHKECCHGDLLECADDRADLAKYICDNQDTISSKLKECCDKPLLEKSHCIAEVEKDAIPENLPPLTADFAEDKDVCKNYQEAKDAFLGSFLYEYSRRHPEYAVSVLLRLAKEYEATLEECCAKDDPHACYSTVFDKLKHLVDEPQNLIKQNCDQFEKLGEYGFQNALIVRYTRKVPQVSTPTLVEVSRSLGKVGTRCCTKPESERMPCTEDYLSLILNRLCVLHEKTPVSEKVTKCCTESLVNRRPCFSALTPDETYVPKAFDEKLFTFHADICTLPDTEKQIKKQTALVELLKHKPKATEEQLKTVMENFVAFVDKCCAADDKEACFAVEGPKLVVSTQTALA

SEQ ID NO: 95 - protein, 608 aa, Felis catus
MKWVTFISLLLLFSSAYSRGVTRREAHQSEIAHRFNDLGEEHFRGLVLVAFSQYLQQCPFEDHVKLVNEVTEFAKGCVADQSAANCEKSLHELLGDKLCTVASLRDKYGEMADCCEKKEPERNECFLQHKDDNPGFGQLVTPEADAMCTAFHENEQRFLGKYLYEIARRHPYFYAPELLYYAEEYKGVFTECCEAADKAACLTPKVDALREKVLASSAKERLKCASLQKFGERAFKAWSVARLSQKFPKAEFAEISKLVTDLAKIHKECCHGDLLECADDRADLAKYICENQDSISTKLKECCGKPVLEKSHCISEVERDELPADLPPLAVDFVEDKEVCKNYQEAKDVFLGTFLYEYSRRHPEYSVSLLLRLAKEYEATLEKCCATDDPPACYAHVFDEFKPLVEEPHNLVKTNCELFEKLGEYGFQNALLVRYTKKVPQVSTPTLVEVSRSLGKVGSKCCTHPEAERLSCAEDYLSVVLNRLCVLHEKTPVSERVTKCCTESLVNRRPCFSALQVDETYVPKEFSAETFTFHADLCTLPEAEKQIKKQSALVELLKHKPKATEEQLKTVMGDFGSFVDKCCAAEDKEACFAEEGPKLVAAAQAALA

SEQ ID NO: 96 - protein, 608 aa, Canis lupus familaris
MKWVTFISLFFLFSSAYSRGLVRREAYKSEIAHRYNDLGEEHFRGLVLVAFSQYLQQCPFEDHVKLAKEVTEFAKACAAEESGANCDKSLHTLFGDKLCTVASLRDKYGDMADCCEKQEPDRNECFLAHKDDNPGFPPLVAPEPDALCAAFQDNEQLFLGKYLYEIARRHPYFYAPELLYYAQQYKGVFAECCQAADKAACLGPKIEALREKVLLSSAKERFKCASLQKFGDRAFKAWSVARLSQRFPKADFAEISKVVTDLTKVHKECCHGDLLECADDRADLAKYMCENQDSISTKLKECCDKPVLEKSQCLAEVERDELPGDLPSLAADFVEDKEVCKNYQEAKDVFLGTFLYEYARRHPEYSVSLLLRLAKEYEATLEKCCATDDPPTCYAKVLDEFKPLVDEPQNLVKTNCELFEKLGEYGFQNALLVRYTKKAPQVSTPTLVEVSRKLGKVGTKCCKKPESERMSCAEDFLSVVLNRLCVLHEKTPVSERVTKCCSESLVNRRPCFSGLEVDETYVPKEFNAETFTFHADLCTLPEAEKQVKKQTALVELLKHKPKATDEQLKTVMGDFGAFVEKCCAAENKEGCFSEEGPKLVAAAQAALV

SEQ ID NO: 97 - protein, 607 aa, Equus asinus
MKWVTFVSLLFLFSSAYFRGVLRRDTHKSEIAHRFNDLGEKHFKGLVLVAFSQYLQQCPFEDHVKLVNEVTEFAKKCAADESAENCDKSLHTLFGDKLCTVATLRATYGELADCCEKQEPERNECFLTHKDDHPNLPKLKPEPDAQCAAFQEDPDKFLGKYLYEVARRHPYFYGPELLFHAEEYKADFTECCPADDKAGCLIPKLDALKERILLSSAKERLKCSSFQKFGERAFKAWSVARLSQKFPKADFAEVSKIVTDLTKVHKECCHGDLLECADDRADLTKYICEHQDSISGKLKACCDKPLLQKSHCIAEVKEDDLPSDLPALAADFAEDKEICKHYKDAKDVFLGTFLYEYSRRHPDYSVSLLLRIAKTYEATLEKCCAEADPPACYATVFDQFTPLVEEPKSLVKKNCDLFEEVGEYDFQNALIVRYTKKAPQVSTPTLVEIGRTLGKVGSRCCKLPESERLPCSENHLALALNRLCVLHEKTPVSEKITKCCTDSLAERRPCFSALELDEGYIPKEFKAETFTFHADICTLPEDEKQIKKQSALAELVKHKPKATKEQLKTVLGNFSAFVAKCCGAEDKEACFAEEGPKLVASSQLALA

SEQ ID NO: 98 - protein, 609 aa, Meriones unguiculatus
MKWVTFLLLLFVSGSAFSRGVFRRDAAHKSEIAHRYKDLGEKYFKGLVLYTFSQYLQKCSYEEHVKLVREVTDFASNCAKDESAENCDKSLHTLFGDKLCSLPNFGEKYAEMADCCAKQEPERNECFLQHKDDNPQLPPFKRAEPDAMCTAFQENAEAFMGHYLHEVARRHPYFYGPELLYLADKYTAVLTECCAADDKGACLTPKLDALKEKALVSAVRQRLKCSSMKKFGERAFKAWAVARMSQTFPNADFAEITKLATDLTKVTQECCHGDLLECADDRAELAKYMCENQASISSKLQACCDKEMLQKSQCLAEVEHDDMPADLPALTADFVEDKDVCKNYAEAKDVFLGTFLYEYSRRHPEYSVSLLLRLAKKYEATLEKCCAEADPHACYGHVFDEFKPLVEEPQNLVKSNCELYEKLGEYGFQNAVLVRYTKKAPQVSTPTLVEAARSLGRVGTHCCALPEKKRLPCVEDYLSAILNRVCLLHEKTPVSEQVTKCCSGSLVERRPCFSALPVDETYVPKEFKAETFTFHANICTLPEKEKQMEKQTALAELVKHKPQATEEQLKKVMGDFAEFLEKCCKQEDKEACFSTEGPKLVAESQKALA

SEQ ID NO: 99 - protein, 583 aa, Capra hircus
DTHKSEIAHRFNDLGEENFQGLVLIAFSQYLQQCPFDEHVKLVKELTEFAKTCVADESHAGCDKSLHTLFGDELCKVATLRETYGDMADCCEKQEPERNECFLKHKDDSPDLPKLKPEPDTLCAEFKADEKKFWGKYLYEVARRHPYFYAPELLYYANKYNGVFQECCQAEDKGACLLPKIETMREKVLASSARQRLRCASIQKFGERALKAWSVARLSQKFPKADFTDVTKIVTDLTKVHKECCHGDLLECADDRADLAKYICDHQDTLSSKLKECCDKPVLEKSHCIAEIDKDAVPENLPPLTADFAEDKEVCKNYQEAKDVFLGSFLYEYSRRHPEYAVSVLLRLAKEYEATLEDCCAKEDPHACYATVFDKLKHLVDEPQNLIKKNCELFEKHGEYGFQNALIVRYTRKAPQVSTPTLVEISRSLGKVGTKCCAKPESERMPCTEDYLSLILNRLCVLHEKTPVSEKVTKCCTESLVNRRPCFSDLTLDETYVPKPFDGESFTFHADICTLPDTEKQIKKQTALVELLKHKPKATDEQLKTVMENFVAFVDKCCAADDKEGCFLLEGPKLVASTQAALA

SEQ ID NO: 100 - protein, 608 aa, Cavia porcellus
MKWVTFISLLFLFSSVYSRGVFRREAHKSEIAHRFNDLGEGHFKGLVLITLSQHLQKSPFEEHVKLVNEVTDFAKACVADESAQNCGKAIATLFGDKVCAIPSLRETYGELADCCAKEDPDRVECFLQHKDDNPNLPPFERPEPEALCTAFKENNDRFIGHYLYEVSRRHPYFYAPELLYYAEKYKNALTECCEAADKAACLTPKLDAIKEKALVSSAQQRLKCASLQKFGERAFKAWSVARLSQKFPKAEFAEISTIVTSLTKVTKECCHGDLLECADDRQELAKYMCEHQDSISSKLKECCVKPTLQKAHCILEIQRDELPTELPDLAVDFVEDKEVCKNFAEAKDVFLGTFLYEYSRRHPEYSIGMLLRIAKGYEAKLEKCCAEADPHACYAKVFDELQPLIDEPKKLVQQNCELFDKLGEYGFQNALAVRYTQKAPQVSTPTLVEYARKLGSVGTKCCSLPETERLSCTENYLALILNRLCILHEKTPVSERVTKCCTESLVNRRPCFSALHVDETYVPKPFHADSFTFHADICTLPEKEKQVKKQMALVELVKHKPKASEEQMKTVMGDFAAFLKKCCDADNKEACFTEDGPKLVAKCQATLA

SEQ ID NO: 101 - protein, 607 aa, Equus caballus
MKWVTFVSLLFLFSSAYSRGVLRRDTHKSEIAHRFNDLGEKHFKGLVLVAFSQYLQQCPFEDHVKLVNEVTEFAKKCAADESAENCDKSLHTLFGDKLCTVATLRATYGELADCCEKQEPERNECFLTHKDDHPNLPKLKPEPDAQCAAFQEDPDKFLGKYLYEVARRHPYFYGPELLFHAEEYKADFTECCPADDKLACLIPKLDALKERILLSSAKERLKCSSFQNFGERAVKAWSVARLSQKFPKADFAEVSKIVTDLTKVHKECCHGDLLECADDRADLAKYICEHQDSISGKLKACCDKPLLQKSHCIAEVKEDDLPSDLPALAADFAEDKEICKHYKDAKDVFLGTFLYEYSRRHPDYSVSLLLRIAKTYEATLEKCCAEADPPACYRTVFDQFTPLVEEPKSLVKKNCDLFEEVGEYDFQNALIVRYTKKAPQVSTPTLVEIGRTLGKVGSRCCKLPESERLPCSENHLALALNRLCVLHEKTPVSEKITKCCTDSLAERRPCFSALELDEGYVPKEFKAETFTFHADICTLPEDEKQIKKQSALAELVKHKPKATKEQLKTVLGNFSAFVAKCCGREDKEACFAEEGPKLVASSQLALA

SEQ ID NO: 102 - protein, 609 aa, Homo sapiens [sequence omitted]

SEQ ID NO: 103 - protein, 600 aa, Macca mulatta
LLFLFSSAYSRGVFRRDTHKSEVAHRFKDLGEEHFKGLVLVAFSQYLQQCPFEEHVKLVNEVTEFAKTCVADESAENCDKSLHTLFGDKLCTVATLRETYGEMADCCAKQEPERNECFLQHKDDNPNLPPLVRPEVDVMCTAFHDNEATFLKKYLYEVARRHPYFYAPELLFFAARYKAAFAECCQAADKAACLLPKLDELRDEGKASSAKQRLKCASLQKFGDRAFKAWAVARLSQKFPKAEFAEVSKLVTDLTKVHTECCHGDLLECADDRADLAKYMCENQDSISSKLKECCDKPLLEKSHCLAEVENDEMPADLPSLAADYVESKDVCKNYAEAKDVFLGMFLYEYARRHPDYSVMLLLRLAKAYEATLEKCCAAADPHECYAKVFDEFQPLVEEPQNLVKQNCELFEQLGEYKFQNALLVRYTKKVPQVSTPTLVEVSRNLGKVGAKCCKLPEAKRMPCAEDYLSVVLNRLCVLHEKTPVSEKVTKCCTESLVNRRPCFSALELDEAYVPKAFNAETFTFHADMCTLSEKEKQVKKQTALVELVKHKPKATKEQLKGVMDNFAAFVEKCCKADDKEACFAEEGPKFVAASQAALA

SEQ ID NO: 104 - protein, 608 aa, Mus musculus
MKWVTFLLLLFVSGSAFSRGVFRREAHKSEIAHRYNDLGEQHFKGLVLIAFSQYLQKCSYDEHAKLVQEVTDFAKTCVADESAANCDKSLHTLFGDKLCAIPNLRENYGELADCCTKQEPERNECFLQHKDDNPSLPPFERPEAEAMCTSFKENPTTFMGHYLHEVARRHPYFYAPELLYYAEQYNEILTQCCAEADKESCLTPKLDGVKEKALVSSVRQRMKCSSMQKFGERAFKAWAVARLSQTFPNADFAEITKLATDLTKVNKECCHGDLLECADDRAELAKYMCENQATISSKLQTCCDKPLLKKAHCLSEVEHDTMPADLPAIAADFVEDQEVCKNYAEAKDVFLGTFLYEYSRRHPDYSVSLLLRLAKKYEATLEKCCAEANPPACYGTVLAEFQPLVEEPKNLVKTNCDLYEKLGEYGFQNAILVRYTQKAPQVSTPTLVEAARNLGRVGTKCCTLPEDQRLPCVEDYLSAILNRVCLLHEKTPVSEHVTKCCSGSLVERRPCFSALTVDETYVPKEFKAETFTFHSDICTLPEKEKQIKKQTALAELVKHKPKATAEQLKTVMDDFAQFLDTCCKAADKDTCFSTEGPNLVTRCKDALA

SEQ ID NO: 105 - protein, 607 aa, Sus scrofa
MKWVTFISLLFLFSSAYSRGVFRRDTYKSEIAHRFKDLGEQYFKGLVLIAFSQHLQQCPYEEHVKLVREVTEFAKTCVADESAENCDKSIHTLFGDKLCAIPSLREHYGDLADCCEKEEPERNECFLQHKNDNPDIPKLKPDPVALCADFQEDEQKFWGKYLYEIARRHPYFYAPELLYYAIIYKDVFSECCQAADKAACLLPKIEHLREKVLTSAAKQRLKCASIQKFGERAFKAWSLARLSQRFPKADFTEISKIVTDLAKVHKECCHGDLLECADDRADLAKYICENQDTISTKLKECCDKPLLEKSHCIAEAKRDELPADLNPLEHDFVEDKEVCKNYKEAKHVFLGTFLYEYSRRHPDYSVSLLLRIAKIYEATLEDCCAKEDPPACYATVFDKFQPLVDEPKNLIKQNCELFEKLGEYGFQNALIVRYTKKVPQVSTPTLVEVARKLGLVGSRCCKRPEEERLSCAEDYLSLVLNRLCVLHEKTPVSEKVTKCCTESLVNRRPCFSALTPDETYKPKEFVEGTFTFHADLCTLPEDEKQIKKQTALVELLKHKPHATEEQLRTVLGNFAAFVQKCCAAPDHEACFAVEGPKFVIEIRGILA

SEQ ID NO: 106 - protein, 608 aa, Oryctolagus cuniculus
MKWVTFISLLFLFSSAYSRGVFRREAHKSEIAHRFNDVGEEHFIGLVLITFSQYLQKCPYEEHAKLVKEVTDLAKACVADESAANCDKSLHDIFGDKICALPSLRDTYGDVADCCEKKEPERNECFLHHKDDKPDLPPFARPEADVLCKAFHDDEKAFFGHYLYEVARRHPYFYAPELLYYAQKYKAILTECCEAADKGACLTPKLDALEGKSLISAAQERLRCASIQKFGDRAYKAWALVRLSQRFPKADFTDISKIVTDLTKVHKECCHGDLLECADDRADLAKYMCEHQETISSHLKECCDKPILEKAHCIYGLHNDETPAGLPAVAEEFVEDKDVCKNYEEAKDLFLGKFLYEYSRRHPDYSVVLLLRLGKAYEATLKKCCATDDPHACYAKVLDEFQPLVDEPKNLVKQNCELYEQLGDYNFQNALLVRYTKKVPQVSTPTLVEISRSLGKVGSKCCKHPEAERLPCVEDYLSVVLNRLCVLHEKTPVSEKVTKCCSESLVDRRPCFSALGPDETYVPKEFNAETFTFHADICTLPETERKIKKQTALVELVKHKPHATNDQLKTVVGEFTALLDKCCSAEDKEACFAVEGPKLVESSKATLG

SEQ ID NO: 107 - protein, 608 aa, Rattus norvegicus
MKWVTFLLLLFISGSAFSRGVFRREAHKSEIAHRFKDLGEQHFKGLVLIAFSQYLQKCPYEEHIKLVQEVTDFAKTCVADENAENCDKSIHTLFGDKLCAIPKLRDNYGELADCCAKQEPERNECFLQHKDDNPNLPPFQRPEAEAMCTSFQENPTSFLGHYLHEVARRHPYFYAPELLYYAEKYNEVLTQCCTESDKAACLTPKLDAVKEKALVAAVRQRMKCSSMQRFGERAFKAWAVARMSQRFPNAEFAEITKLATDVTKINKECCHGDLLECADDRAELAKYMCENQATISSKLQACCDKPVLQKSQCLAEIEHDNIPADLPSIAADFVEDKEVCKNYAEAKDVFLGTFLYEYSRRHPDYSVSLLLRLAKKYEATLEKCCAEGDPPACYGTVLAEFQPLVEEPKNLVKTNCELYEKLGEYGFQNAVLVRYTQKAPQVSTPTLVEAARNLGRVGTKCCTLPEAQRLPCVEDYLSAILNRLCVLHEKTPVSEKVTKCCSGSLVERRPCFSALTVDETYVPKEFKAETFTFHSDICTLPDKEKQIKKQTALAELVKHKPKATEDQLKTVMGDFAQFVDKCCKAADKDNCFATEGPNLVARSKEALA

SEQ ID NO: 108 - protein, 607 aa, Ovis aries
MKWVTFISLLLLFSSAYSRGVFRRDTHKSEIAHRFNDLGEENFQGLVLIAFSQYLQQCPFDEHVKLVKELTEFAKTCVADESHAGCDKSLHTLFGDELCKVATLRETYGDMADCCEKQEPERNECFLNHKDDSPDLPKLKPEPDTLCAEFKADEKKFWGKYLYEVARRHPYFYAPELLYYANKYNGVFQECCQAEDKGACLLPKIDAMREKVLASSARQRLRCASIQKFGERALKAWSVARLSQKFPKADFTDVTKIVTDLTKVHKECCHGDLLECADDRADLAKYICDHQDALSSKLKECCDKPVLEKSHCIAEVDKDAVPENLPPLTADFAEDKEVCKNYQEAKDVFLGSFLYEYSRRHPEYAVSVLLRLAKEYEATLEDCCAKEDPHACYATVFDKLKHLVDEPQNLIKKNCELFEKHGEYGFQNALIVRYTRKAPQVSTPTLVEISRSLGKVGTKCCAKPESERMPCTEDYLSLILNRLCVLHEKTPVSEKVTKCCTESLVNRRPCFSDLTLDETYVPKPFDEKFFTFHADICTLPDTEKQIKKQTALVELLKHKPKATDEQLKTVMENFVAFVDKCCAADDKEGCFVLEGPKLVASTQAALA